European Patent Application EP 4 790 065 A1, published August 12, 2026. Title: Coronavirus spike protein mutants. Applicant: SHIONOGI & CO., LTD. Application JP. The sequence listing filed with the application follows.

SEQUENCE LISTING (122 sequences)

SEQ ID NO: 1 - protein, 203 aa, synthetic construct
  SITE 3: note = X can be Q or N.
  SITE 132: note = X can be N or K.
  SITE 149: note = X can be S or Y.
  SITE 173: note = X can be N or Y.
FPXITNLCPFGEVFNATKFPSVYAWERKKISNCVADYSVLYNSTFFSTFKCYGVSATKLNDLCFSNVYADSFVVKGDDVRQIAPGQTGVIADYNYKLPDDFMGCVIAWNSNNLDSKVGGNYNYRYRLFRKSXLKPFERDISTEIYQAGXKPCNGVEGFNCYFPLQSYGFQPTXGVGYQPYRVVVLSFELLHAPATVCGPKKST

SEQ ID NO: 2 - protein, 203 aa, synthetic construct
FPQITNLCPFGEVFNATKFPSVYAWERKKISNCVADYSVLYNSTFFSTFKCYGVSATKLNDLCFSNVYADSFVVKGDDVRQIAPGQTGVIADYNYKLPDDFMGCVIAWNSNNLDSKVGGNYNYRYRLFRKSNLKPFERDISTEIYQAGSKPCNGVEGFNCYFPLQSYGFQPTNGVGYQPYRVVVLSFELLHAPATVCGPKKST

SEQ ID NO: 3 - protein, 203 aa, synthetic construct
FPNITNLCPFGEVFNATKFPSVYAWERKKISNCVADYSVLYNSTFFSTFKCYGVSATKLNDLCFSNVYADSFVVKGDDVRQIAPGQTGVIADYNYKLPDDFMGCVIAWNSNNLDSKVGGNYNYRYRLFRKSNLKPFERDISTEIYQAGSKPCNGVEGFNCYFPLQSYGFQPTNGVGYQPYRVVVLSFELLHAPATVCGPKKST

SEQ ID NO: 4 - protein, 203 aa, synthetic construct
FPQITNLCPFGEVFNATKFPSVYAWERKKISNCVADYSVLYNSTFFSTFKCYGVSATKLNDLCFSNVYADSFVVKGDDVRQIAPGQTGVIADYNYKLPDDFMGCVIAWNSNNLDSKVGGNYNYRYRLFRKSKLKPFERDISTEIYQAGSKPCNGVEGFNCYFPLQSYGFQPTYGVGYQPYRVVVLSFELLHAPATVCGPKKST

SEQ ID NO: 5 - protein, 203 aa, synthetic construct
FPQITNLCPFGEVFNATKFPSVYAWERKKISNCVADYSVLYNSTFFSTFKCYGVSATKLNDLCFSNVYADSFVVKGDDVRQIAPGQTGVIADYNYKLPDDFMGCVIAWNSNNLDSKVGGNYNYRYRLFRKSKLKPFERDISTEIYQAGNKPCNGVEGFNCYFPLQSYGFQPTYGVGYQPYRVVVLSFELLHAPATVCGPKKST

SEQ ID NO: 6 - protein, 1252 aa, synthetic construct
MFVFLVLLPLVSSQCVNLRTRTQLPPAYTNSFTRGVYYPDKVFRSSVLHSTQDLFLPFFSNVTWFHAIHVSGTNGTKRFDNPVLPFNDGVYFASTEKSNIIRGWIFGTTLDSKTQSLLIVNNATNVVIKVCEFQFCNDPFLDVYYHKNNKSWMESGVYSSANNCTFEYVSQPFLMDLEGKQGNFKNLREFVFKNIDGYFKIYSKHTPINLVRDLPQGFSALEPLVDLPIGINITRFQTLLALHRSYLTPGDSSSGWTAGAAAYYVGYLQPRTFLLKYNENGTITDAVDCALDPLSETKCTLKSFTVEKGIYQTSNFRVQPTESIVRFPNITNLCPFGEVFNATRFASVYAWNRKRISNCVADYSVLYNSASFSTFKCYGVSPTKLNDLCFTNVYADSFVIRGDEVRQIAPGQTGKIADYNYKLPDDFTGCVIAWNSNNLDSKVGGNYNYRYRLFRKSNLKPFERDISTEIYQAGSKPCNGVEGFNCYFPLQSYGFQPTNGVGYQPYRVVVLSFELLHAPATVCGPKKSTNLVKNKCVNFNFNGLTGTGVLTESNKKFLPFQQFGRDIADTTDAVRDPQTLEILDITPCSFGGVSVITPGTNTSNQVAVLYQGVNCTEVPVAIHADQLTPTWRVYSTGSNVFQTRAGCLIGAEHVNNSYECDIPIGAGICASYQTQTNSRRRARSVASQSIIAYTMSLGAENSVAYSNNSIAIPTNFTISVTTEILPVSMTKTSVDCTMYICGDSTECSNLLLQYGSFCTQLNRALTGIAVEQDKNTQEVFAQVKQIYKTPPIKDFGGFNFSQILPDPSKPSKRSFIEDLLFNKVTLADAGFIKQYGDCLGDIAARDLICAQKFNGLTVLPPLLTDEMIAQYTSALLAGTITSGWTFGAGAALQIPFAMQMAYRFNGIGVTQNVLYENQKLIANQFNSAIGKIQDSLSSTASALGKLQNVVNQNAQALNTLVKQLSSNFGAISSVLNDILSRLDKVEAEVQIDRLITGRLQSLQTYVTQQLIRAAEIRASANLAATKMSECVLGQSKRVDFCGKGYHLMSFPQSAPHGVVFLHVTYVPAQEKNFTTAPAICHDGKAHFPREGVFVSNGTHWFVTQRNFYEPQIITTDNTFVSGNCDVVIGIVNNTVYDPLQPELDSFKEELDKYFKNHTSPDVDLGDISGINASVVNIQKEIDRLNEVAKNLNESLIDLQELGKYEQYIKWPWYIWLGFIAGLIAIVMVTIMLCCMTSCCSCLKGCCSCGSCC

SEQ ID NO: 7 - protein, 288 aa, synthetic construct
  SITE 150: note = X can be T or L
QCVNLITRTQSYTNSFTRGVYYPDKVFRSSVLHSTQDLFLPFFSNVTWFHAIHVSGTNGTKRFDNPALPFNDGVYFASTEKSNIIRGWIFGTTLDSKTQSLLIVNNATNVVIKVCEFQFCNDPFLDVYQKNNKSWMESEFRVYSSANNCXFEYVSQPFLMDLEGKEGNFKNLREFVFKNIDGYFKIYSKHTPINLERDLPQGFSALEPLVDLPIGINITRFQTLLALHRSYLTPVDSSSGWTAGAAAYYVGYLQPRTFLLKYNENGTITDAVDCALDPLSETKCTLKS

SEQ ID NO: 8 - protein, 288 aa, synthetic construct
QCVNLITRTQSYTNSFTRGVYYPDKVFRSSVLHSTQDLFLPFFSNVTWFHAIHVSGTNGTKRFDNPALPFNDGVYFASTEKSNIIRGWIFGTTLDSKTQSLLIVNNATNVVIKVCEFQFCNDPFLDVYQKNNKSWMESEFRVYSSANNCTFEYVSQPFLMDLEGKEGNFKNLREFVFKNIDGYFKIYSKHTPINLERDLPQGFSALEPLVDLPIGINITRFQTLLALHRSYLTPVDSSSGWTAGAAAYYVGYLQPRTFLLKYNENGTITDAVDCALDPLSETKCTLKS

SEQ ID NO: 9 - protein, 288 aa, synthetic construct
QCVNLITRTQSYTNSFTRGVYYPDKVFRSSVLHSTQDLFLPFFSNVTWFHAIHVSGTNGTKRFDNPALPFNDGVYFASTEKSNIIRGWIFGTTLDSKTQSLLIVNNATNVVIKVCEFQFCNDPFLDVYQKNNKSWMESEFRVYSSANNCLFEYVSQPFLMDLEGKEGNFKNLREFVFKNIDGYFKIYSKHTPINLERDLPQGFSALEPLVDLPIGINITRFQTLLALHRSYLTPVDSSSGWTAGAAAYYVGYLQPRTFLLKYNENGTITDAVDCALDPLSETKCTLKS

SEQ ID NO: 10 - protein, 682 aa, synthetic construct
  SITE 264: note = X can be K or P.
  SITE 434: note = X can be Q or C.
  SITE 455: note = X can be P ro K.
  SITE 472: note = X can be S or C.
  SITE 543: note = X can be N or Q.
  SITE 567: note = X can be N or T.
  SITE 642: note = X can be N or L.
NLVKNKCVNFNFNGLTGTGVLTESNKKFLPFQQFGRDIADTTDAVRDPQTLEILDITPCSFGGVSVITPGTNTSNQVAVLYQGVNCTEVPVAIHADQLTPTWRVYSTGSNVFQTRAGCLIGAEHVNNSYECDIPIGAGICASYQTQTNSRGSASSVASQSIIAYTMSLGAENSVAYSNNSIAIPTNFTISVTTEILPVSMPKTSVDCTMYICGDSTECSNLLLQYGSFCTQLNRALTGIAVEQDKNTQEVFAQVKQIYKTPPIXDFGGFNFSQILPDPSKPSKRSPIEDLLFNKVTLADAGFIKQYGDCLGDIAARDLICAQKFNGLTVLPPLLTDEMIAQYTSALLAGTITSGWTFGAGPALQIPFPMQMAYRFNGIGVTQNVLYENQKLIANQFNSAIGKIQDSLSSTPSALGKLQNVVNQNAQALNTLVKXLSSNFGAISSVLNDILSRLDXPEAEVQIDRLITGRLQXLQTYVTQQLIRAAEIRASANLAATKMSECVLGQSKRVDFCGKGYHLMSFPQSAPHGVVFLHVTYVPAQEKXFTTAPAICHDGKAHFPREGVFVSXGTHWFVTQRNFYEPQIITTDNTFVSGNCDVVIGIVNNTVYDPLQPELDSFKEELDKYFKNHTSPDVDLGDISGIXASVVNIQKEIDRLNEVAKNLNESLIDLQELGKYEQYIKWP

SEQ ID NO: 11 - protein, 682 aa, synthetic construct
NLVKNKCVNFNFNGLTGTGVLTESNKKFLPFQQFGRDIADTTDAVRDPQTLEILDITPCSFGGVSVITPGTNTSNQVAVLYQGVNCTEVPVAIHADQLTPTWRVYSTGSNVFQTRAGCLIGAEHVNNSYECDIPIGAGICASYQTQTNSRGSASSVASQSIIAYTMSLGAENSVAYSNNSIAIPTNFTISVTTEILPVSMPKTSVDCTMYICGDSTECSNLLLQYGSFCTQLNRALTGIAVEQDKNTQEVFAQVKQIYKTPPIKDFGGFNFSQILPDPSKPSKRSPIEDLLFNKVTLADAGFIKQYGDCLGDIAARDLICAQKFNGLTVLPPLLTDEMIAQYTSALLAGTITSGWTFGAGPALQIPFPMQMAYRFNGIGVTQNVLYENQKLIANQFNSAIGKIQDSLSSTPSALGKLQNVVNQNAQALNTLVKQLSSNFGAISSVLNDILSRLDPPEAEVQIDRLITGRLQSLQTYVTQQLIRAAEIRASANLAATKMSECVLGQSKRVDFCGKGYHLMSFPQSAPHGVVFLHVTYVPAQEKNFTTAPAICHDGKAHFPREGVFVSNGTHWFVTQRNFYEPQIITTDNTFVSGNCDVVIGIVNNTVYDPLQPELDSFKEELDKYFKNHTSPDVDLGDISGINASVVNIQKEIDRLNEVAKNLNESLIDLQELGKYEQYIKWP

SEQ ID NO: 12 - protein, 682 aa, synthetic construct
NLVKNKCVNFNFNGLTGTGVLTESNKKFLPFQQFGRDIADTTDAVRDPQTLEILDITPCSFGGVSVITPGTNTSNQVAVLYQGVNCTEVPVAIHADQLTPTWRVYSTGSNVFQTRAGCLIGAEHVNNSYECDIPIGAGICASYQTQTNSRGSASSVASQSIIAYTMSLGAENSVAYSNNSIAIPTNFTISVTTEILPVSMPKTSVDCTMYICGDSTECSNLLLQYGSFCTQLNRALTGIAVEQDKNTQEVFAQVKQIYKTPPIKDFGGFNFSQILPDPSKPSKRSPIEDLLFNKVTLADAGFIKQYGDCLGDIAARDLICAQKFNGLTVLPPLLTDEMIAQYTSALLAGTITSGWTFGAGPALQIPFPMQMAYRFNGIGVTQNVLYENQKLIANQFNSAIGKIQDSLSSTPSALGKLQNVVNQNAQALNTLVKQLSSNFGAISSVLNDILSRLDPPEAEVQIDRLITGRLQSLQTYVTQQLIRAAEIRASANLAATKMSECVLGQSKRVDFCGKGYHLMSFPQSAPHGVVFLHVTYVPAQEKNFTTAPAICHDGKAHFPREGVFVSNGTHWFVTQRNFYEPQIITTDNTFVSGNCDVVIGIVNNTVYDPLQPELDSFKEELDKYFKNHTSPDVDLGDISGILASVVNIQKEIDRLNEVAKNLNESLIDLQELGKYEQYIKWP

SEQ ID NO: 13 - protein, 682 aa, synthetic construct
NLVKNKCVNFNFNGLTGTGVLTESNKKFLPFQQFGRDIADTTDAVRDPQTLEILDITPCSFGGVSVITPGTNTSNQVAVLYQGVNCTEVPVAIHADQLTPTWRVYSTGSNVFQTRAGCLIGAEHVNNSYECDIPIGAGICASYQTQTNSRGSASSVASQSIIAYTMSLGAENSVAYSNNSIAIPTNFTISVTTEILPVSMPKTSVDCTMYICGDSTECSNLLLQYGSFCTQLNRALTGIAVEQDKNTQEVFAQVKQIYKTPPIKDFGGFNFSQILPDPSKPSKRSPIEDLLFNKVTLADAGFIKQYGDCLGDIAARDLICAQKFNGLTVLPPLLTDEMIAQYTSALLAGTITSGWTFGAGPALQIPFPMQMAYRFNGIGVTQNVLYENQKLIANQFNSAIGKIQDSLSSTPSALGKLQNVVNQNAQALNTLVKQLSSNFGAISSVLNDILSRLDKPEAEVQIDRLITGRLQSLQTYVTQQLIRAAEIRASANLAATKMSECVLGQSKRVDFCGKGYHLMSFPQSAPHGVVFLHVTYVPAQEKNFTTAPAICHDGKAHFPREGVFVSNGTHWFVTQRNFYEPQIITTDNTFVSGNCDVVIGIVNNTVYDPLQPELDSFKEELDKYFKNHTSPDVDLGDISGINASVVNIQKEIDRLNEVAKNLNESLIDLQELGKYEQYIKWP

SEQ ID NO: 14 - protein, 682 aa, synthetic construct
NLVKNKCVNFNFNGLTGTGVLTESNKKFLPFQQFGRDIADTTDAVRDPQTLEILDITPCSFGGVSVITPGTNTSNQVAVLYQGVNCTEVPVAIHADQLTPTWRVYSTGSNVFQTRAGCLIGAEHVNNSYECDIPIGAGICASYQTQTNSRGSASSVASQSIIAYTMSLGAENSVAYSNNSIAIPTNFTISVTTEILPVSMPKTSVDCTMYICGDSTECSNLLLQYGSFCTQLNRALTGIAVEQDKNTQEVFAQVKQIYKTPPIPDFGGFNFSQILPDPSKPSKRSPIEDLLFNKVTLADAGFIKQYGDCLGDIAARDLICAQKFNGLTVLPPLLTDEMIAQYTSALLAGTITSGWTFGAGPALQIPFPMQMAYRFNGIGVTQNVLYENQKLIANQFNSAIGKIQDSLSSTPSALGKLQNVVNQNAQALNTLVKCLSSNFGAISSVLNDILSRLDPPEAEVQIDRLITGRLQCLQTYVTQQLIRAAEIRASANLAATKMSECVLGQSKRVDFCGKGYHLMSFPQSAPHGVVFLHVTYVPAQEKNFTTAPAICHDGKAHFPREGVFVSNGTHWFVTQRNFYEPQIITTDNTFVSGNCDVVIGIVNNTVYDPLQPELDSFKEELDKYFKNHTSPDVDLGDISGILASVVNIQKEIDRLNEVAKNLNESLIDLQELGKYEQYIKWP

SEQ ID NO: 15 - protein, 682 aa, synthetic construct
NLVKNKCVNFNFNGLTGTGVLTESNKKFLPFQQFGRDIADTTDAVRDPQTLEILDITPCSFGGVSVITPGTNTSNQVAVLYQGVNCTEVPVAIHADQLTPTWRVYSTGSNVFQTRAGCLIGAEHVNNSYECDIPIGAGICASYQTQTNSRGSASSVASQSIIAYTMSLGAENSVAYSNNSIAIPTNFTISVTTEILPVSMPKTSVDCTMYICGDSTECSNLLLQYGSFCTQLNRALTGIAVEQDKNTQEVFAQVKQIYKTPPIPDFGGFNFSQILPDPSKPSKRSPIEDLLFNKVTLADAGFIKQYGDCLGDIAARDLICAQKFNGLTVLPPLLTDEMIAQYTSALLAGTITSGWTFGAGPALQIPFPMQMAYRFNGIGVTQNVLYENQKLIANQFNSAIGKIQDSLSSTPSALGKLQNVVNQNAQALNTLVKCLSSNFGAISSVLNDILSRLDPPEAEVQIDRLITGRLQCLQTYVTQQLIRAAEIRASANLAATKMSECVLGQSKRVDFCGKGYHLMSFPQSAPHGVVFLHVTYVPAQEKQFTTAPAICHDGKAHFPREGVFVSTGTHWFVTQRNFYEPQIITTDNTFVSGNCDVVIGIVNNTVYDPLQPELDSFKEELDKYFKNHTSPDVDLGDISGILASVVNIQKEIDRLNEVAKNLNESLIDLQELGKYEQYIKWP

SEQ ID NO: 16 - protein, 682 aa, synthetic construct
NLVKNKCVNFNFNGLTGTGVLTESNKKFLPFQQFGRDIADTTDAVRDPQTLEILDITPCSFGGVSVITPGTNTSNQVAVLYQGVNCTEVPVAIHADQLTPTWRVYSTGSNVFQTRAGCLIGAEHVNNSYECDIPIGAGICASYQTQTNSRRRARSVASQSIIAYTMSLGAENSVAYSNNSIAIPTNFTISVTTEILPVSMTKTSVDCTMYICGDSTECSNLLLQYGSFCTQLNRALTGIAVEQDKNTQEVFAQVKQIYKTPPIKDFGGFNFSQILPDPSKPSKRSFIEDLLFNKVTLADAGFIKQYGDCLGDIAARDLICAQKFNGLTVLPPLLTDEMIAQYTSALLAGTITSGWTFGAGAALQIPFAMQMAYRFNGIGVTQNVLYENQKLIANQFNSAIGKIQDSLSSTASALGKLQNVVNQNAQALNTLVKQLSSNFGAISSVLNDILSRLDKVEAEVQIDRLITGRLQSLQTYVTQQLIRAAEIRASANLAATKMSECVLGQSKRVDFCGKGYHLMSFPQSAPHGVVFLHVTYVPAQEKNFTTAPAICHDGKAHFPREGVFVSNGTHWFVTQRNFYEPQIITTDNTFVSGNCDVVIGIVNNTVYDPLQPELDSFKEELDKYFKNHTSPDVDLGDISGINASVVNIQKEIDRLNEVAKNLNESLIDLQELGKYEQYIKWP

SEQ ID NO: 17 - protein, 4 aa, synthetic construct
RRAR

SEQ ID NO: 18 - protein, 4 aa, synthetic construct
GSAS

SEQ ID NO: 19 - protein, 27 aa, synthetic construct
GYIPEAPRDGQAYVRKDGEWVLLSTFL

SEQ ID NO: 20 - protein, 6 aa, synthetic construct
HHHHHH

SEQ ID NO: 21 - protein, 1242 aa, synthetic construct
MFVFLVLLPLVSSQCVNLITRTQSYTNSFTRGVYYPDKVFRSSVLHSTQDLFLPFFSNVTWFHAIHVSGTNGTKRFDNPALPFNDGVYFASTEKSNIIRGWIFGTTLDSKTQSLLIVNNATNVVIKVCEFQFCNDPFLDVYQKNNKSWMESEFRVYSSANNCTFEYVSQPFLMDLEGKEGNFKNLREFVFKNIDGYFKIYSKHTPINLERDLPQGFSALEPLVDLPIGINITRFQTLLALHRSYLTPVDSSSGWTAGAAAYYVGYLQPRTFLLKYNENGTITDAVDCALDPLSETKCTLKSFTVEKGIYQTSNFRVQPTESIVRFPQITNLCPFGEVFNATKFPSVYAWERKKISNCVADYSVLYNSTFFSTFKCYGVSATKLNDLCFSNVYADSFVVKGDDVRQIAPGQTGVIADYNYKLPDDFMGCVIAWNSNNLDSKVGGNYNYRYRLFRKSNLKPFERDISTEIYQAGSKPCNGVEGFNCYFPLQSYGFQPTNGVGYQPYRVVVLSFELLHAPATVCGPKKSTNLVKNKCVNFNFNGLTGTGVLTESNKKFLPFQQFGRDIADTTDAVRDPQTLEILDITPCSFGGVSVITPGTNTSNQVAVLYQGVNCTEVPVAIHADQLTPTWRVYSTGSNVFQTRAGCLIGAEHVNNSYECDIPIGAGICASYQTQTNSRGSASSVASQSIIAYTMSLGAENSVAYSNNSIAIPTNFTISVTTEILPVSMPKTSVDCTMYICGDSTECSNLLLQYGSFCTQLNRALTGIAVEQDKNTQEVFAQVKQIYKTPPIKDFGGFNFSQILPDPSKPSKRSPIEDLLFNKVTLADAGFIKQYGDCLGDIAARDLICAQKFNGLTVLPPLLTDEMIAQYTSALLAGTITSGWTFGAGPALQIPFPMQMAYRFNGIGVTQNVLYENQKLIANQFNSAIGKIQDSLSSTPSALGKLQNVVNQNAQALNTLVKQLSSNFGAISSVLNDILSRLDPPEAEVQIDRLITGRLQSLQTYVTQQLIRAAEIRASANLAATKMSECVLGQSKRVDFCGKGYHLMSFPQSAPHGVVFLHVTYVPAQEKNFTTAPAICHDGKAHFPREGVFVSNGTHWFVTQRNFYEPQIITTDNTFVSGNCDVVIGIVNNTVYDPLQPELDSFKEELDKYFKNHTSPDVDLGDISGINASVVNIQKEIDRLNEVAKNLNESLIDLQELGKYEQYIKWPGYIPEAPRDGQAYVRKDGEWVLLSTFLHHHHHH

SEQ ID NO: 22 - protein, 1242 aa, synthetic construct
MFVFLVLLPLVSSQCVNLITRTQSYTNSFTRGVYYPDKVFRSSVLHSTQDLFLPFFSNVTWFHAIHVSGTNGTKRFDNPALPFNDGVYFASTEKSNIIRGWIFGTTLDSKTQSLLIVNNATNVVIKVCEFQFCNDPFLDVYQKNNKSWMESEFRVYSSANNCTFEYVSQPFLMDLEGKEGNFKNLREFVFKNIDGYFKIYSKHTPINLERDLPQGFSALEPLVDLPIGINITRFQTLLALHRSYLTPVDSSSGWTAGAAAYYVGYLQPRTFLLKYNENGTITDAVDCALDPLSETKCTLKSFTVEKGIYQTSNFRVQPTESIVRFPNITNLCPFGEVFNATKFPSVYAWERKKISNCVADYSVLYNSTFFSTFKCYGVSATKLNDLCFSNVYADSFVVKGDDVRQIAPGQTGVIADYNYKLPDDFMGCVIAWNSNNLDSKVGGNYNYRYRLFRKSNLKPFERDISTEIYQAGSKPCNGVEGFNCYFPLQSYGFQPTNGVGYQPYRVVVLSFELLHAPATVCGPKKSTNLVKNKCVNFNFNGLTGTGVLTESNKKFLPFQQFGRDIADTTDAVRDPQTLEILDITPCSFGGVSVITPGTNTSNQVAVLYQGVNCTEVPVAIHADQLTPTWRVYSTGSNVFQTRAGCLIGAEHVNNSYECDIPIGAGICASYQTQTNSRGSASSVASQSIIAYTMSLGAENSVAYSNNSIAIPTNFTISVTTEILPVSMPKTSVDCTMYICGDSTECSNLLLQYGSFCTQLNRALTGIAVEQDKNTQEVFAQVKQIYKTPPIKDFGGFNFSQILPDPSKPSKRSPIEDLLFNKVTLADAGFIKQYGDCLGDIAARDLICAQKFNGLTVLPPLLTDEMIAQYTSALLAGTITSGWTFGAGPALQIPFPMQMAYRFNGIGVTQNVLYENQKLIANQFNSAIGKIQDSLSSTPSALGKLQNVVNQNAQALNTLVKQLSSNFGAISSVLNDILSRLDPPEAEVQIDRLITGRLQSLQTYVTQQLIRAAEIRASANLAATKMSECVLGQSKRVDFCGKGYHLMSFPQSAPHGVVFLHVTYVPAQEKNFTTAPAICHDGKAHFPREGVFVSNGTHWFVTQRNFYEPQIITTDNTFVSGNCDVVIGIVNNTVYDPLQPELDSFKEELDKYFKNHTSPDVDLGDISGILASVVNIQKEIDRLNEVAKNLNESLIDLQELGKYEQYIKWPGYIPEAPRDGQAYVRKDGEWVLLSTFLHHHHHH

SEQ ID NO: 23 - protein, 1242 aa, synthetic construct
MFVFLVLLPLVSSQCVNLITRTQSYTNSFTRGVYYPDKVFRSSVLHSTQDLFLPFFSNVTWFHAIHVSGTNGTKRFDNPALPFNDGVYFASTEKSNIIRGWIFGTTLDSKTQSLLIVNNATNVVIKVCEFQFCNDPFLDVYQKNNKSWMESEFRVYSSANNCTFEYVSQPFLMDLEGKEGNFKNLREFVFKNIDGYFKIYSKHTPINLERDLPQGFSALEPLVDLPIGINITRFQTLLALHRSYLTPVDSSSGWTAGAAAYYVGYLQPRTFLLKYNENGTITDAVDCALDPLSETKCTLKSFTVEKGIYQTSNFRVQPTESIVRFPQITNLCPFGEVFNATKFPSVYAWERKKISNCVADYSVLYNSTFFSTFKCYGVSATKLNDLCFSNVYADSFVVKGDDVRQIAPGQTGVIADYNYKLPDDFMGCVIAWNSNNLDSKVGGNYNYRYRLFRKSNLKPFERDISTEIYQAGSKPCNGVEGFNCYFPLQSYGFQPTNGVGYQPYRVVVLSFELLHAPATVCGPKKSTNLVKNKCVNFNFNGLTGTGVLTESNKKFLPFQQFGRDIADTTDAVRDPQTLEILDITPCSFGGVSVITPGTNTSNQVAVLYQGVNCTEVPVAIHADQLTPTWRVYSTGSNVFQTRAGCLIGAEHVNNSYECDIPIGAGICASYQTQTNSRGSASSVASQSIIAYTMSLGAENSVAYSNNSIAIPTNFTISVTTEILPVSMPKTSVDCTMYICGDSTECSNLLLQYGSFCTQLNRALTGIAVEQDKNTQEVFAQVKQIYKTPPIKDFGGFNFSQILPDPSKPSKRSPIEDLLFNKVTLADAGFIKQYGDCLGDIAARDLICAQKFNGLTVLPPLLTDEMIAQYTSALLAGTITSGWTFGAGPALQIPFPMQMAYRFNGIGVTQNVLYENQKLIANQFNSAIGKIQDSLSSTPSALGKLQNVVNQNAQALNTLVKQLSSNFGAISSVLNDILSRLDKPEAEVQIDRLITGRLQSLQTYVTQQLIRAAEIRASANLAATKMSECVLGQSKRVDFCGKGYHLMSFPQSAPHGVVFLHVTYVPAQEKNFTTAPAICHDGKAHFPREGVFVSNGTHWFVTQRNFYEPQIITTDNTFVSGNCDVVIGIVNNTVYDPLQPELDSFKEELDKYFKNHTSPDVDLGDISGINASVVNIQKEIDRLNEVAKNLNESLIDLQELGKYEQYIKWPGYIPEAPRDGQAYVRKDGEWVLLSTFLHHHHHH

SEQ ID NO: 24 - protein, 1242 aa, synthetic construct
MFVFLVLLPLVSSQCVNLITRTQSYTNSFTRGVYYPDKVFRSSVLHSTQDLFLPFFSNVTWFHAIHVSGTNGTKRFDNPALPFNDGVYFASTEKSNIIRGWIFGTTLDSKTQSLLIVNNATNVVIKVCEFQFCNDPFLDVYQKNNKSWMESEFRVYSSANNCTFEYVSQPFLMDLEGKEGNFKNLREFVFKNIDGYFKIYSKHTPINLERDLPQGFSALEPLVDLPIGINITRFQTLLALHRSYLTPVDSSSGWTAGAAAYYVGYLQPRTFLLKYNENGTITDAVDCALDPLSETKCTLKSFTVEKGIYQTSNFRVQPTESIVRFPQITNLCPFGEVFNATKFPSVYAWERKKISNCVADYSVLYNSTFFSTFKCYGVSATKLNDLCFSNVYADSFVVKGDDVRQIAPGQTGVIADYNYKLPDDFMGCVIAWNSNNLDSKVGGNYNYRYRLFRKSNLKPFERDISTEIYQAGSKPCNGVEGFNCYFPLQSYGFQPTNGVGYQPYRVVVLSFELLHAPATVCGPKKSTNLVKNKCVNFNFNGLTGTGVLTESNKKFLPFQQFGRDIADTTDAVRDPQTLEILDITPCSFGGVSVITPGTNTSNQVAVLYQGVNCTEVPVAIHADQLTPTWRVYSTGSNVFQTRAGCLIGAEHVNNSYECDIPIGAGICASYQTQTNSRGSASSVASQSIIAYTMSLGAENSVAYSNNSIAIPTNFTISVTTEILPVSMPKTSVDCTMYICGDSTECSNLLLQYGSFCTQLNRALTGIAVEQDKNTQEVFAQVKQIYKTPPIPDFGGFNFSQILPDPSKPSKRSPIEDLLFNKVTLADAGFIKQYGDCLGDIAARDLICAQKFNGLTVLPPLLTDEMIAQYTSALLAGTITSGWTFGAGPALQIPFPMQMAYRFNGIGVTQNVLYENQKLIANQFNSAIGKIQDSLSSTPSALGKLQNVVNQNAQALNTLVKCLSSNFGAISSVLNDILSRLDPPEAEVQIDRLITGRLQCLQTYVTQQLIRAAEIRASANLAATKMSECVLGQSKRVDFCGKGYHLMSFPQSAPHGVVFLHVTYVPAQEKNFTTAPAICHDGKAHFPREGVFVSNGTHWFVTQRNFYEPQIITTDNTFVSGNCDVVIGIVNNTVYDPLQPELDSFKEELDKYFKNHTSPDVDLGDISGILASVVNIQKEIDRLNEVAKNLNESLIDLQELGKYEQYIKWPGYIPEAPRDGQAYVRKDGEWVLLSTFLHHHHHH

SEQ ID NO: 25 - protein, 1242 aa, synthetic construct
MFVFLVLLPLVSSQCVNLITRTQSYTNSFTRGVYYPDKVFRSSVLHSTQDLFLPFFSNVTWFHAIHVSGTNGTKRFDNPALPFNDGVYFASTEKSNIIRGWIFGTTLDSKTQSLLIVNNATNVVIKVCEFQFCNDPFLDVYQKNNKSWMESEFRVYSSANNCLFEYVSQPFLMDLEGKEGNFKNLREFVFKNIDGYFKIYSKHTPINLERDLPQGFSALEPLVDLPIGINITRFQTLLALHRSYLTPVDSSSGWTAGAAAYYVGYLQPRTFLLKYNENGTITDAVDCALDPLSETKCTLKSFTVEKGIYQTSNFRVQPTESIVRFPQITNLCPFGEVFNATKFPSVYAWERKKISNCVADYSVLYNSTFFSTFKCYGVSATKLNDLCFSNVYADSFVVKGDDVRQIAPGQTGVIADYNYKLPDDFMGCVIAWNSNNLDSKVGGNYNYRYRLFRKSNLKPFERDISTEIYQAGSKPCNGVEGFNCYFPLQSYGFQPTNGVGYQPYRVVVLSFELLHAPATVCGPKKSTNLVKNKCVNFNFNGLTGTGVLTESNKKFLPFQQFGRDIADTTDAVRDPQTLEILDITPCSFGGVSVITPGTNTSNQVAVLYQGVNCTEVPVAIHADQLTPTWRVYSTGSNVFQTRAGCLIGAEHVNNSYECDIPIGAGICASYQTQTNSRGSASSVASQSIIAYTMSLGAENSVAYSNNSIAIPTNFTISVTTEILPVSMPKTSVDCTMYICGDSTECSNLLLQYGSFCTQLNRALTGIAVEQDKNTQEVFAQVKQIYKTPPIPDFGGFNFSQILPDPSKPSKRSPIEDLLFNKVTLADAGFIKQYGDCLGDIAARDLICAQKFNGLTVLPPLLTDEMIAQYTSALLAGTITSGWTFGAGPALQIPFPMQMAYRFNGIGVTQNVLYENQKLIANQFNSAIGKIQDSLSSTPSALGKLQNVVNQNAQALNTLVKCLSSNFGAISSVLNDILSRLDPPEAEVQIDRLITGRLQCLQTYVTQQLIRAAEIRASANLAATKMSECVLGQSKRVDFCGKGYHLMSFPQSAPHGVVFLHVTYVPAQEKQFTTAPAICHDGKAHFPREGVFVSTGTHWFVTQRNFYEPQIITTDNTFVSGNCDVVIGIVNNTVYDPLQPELDSFKEELDKYFKNHTSPDVDLGDISGILASVVNIQKEIDRLNEVAKNLNESLIDLQELGKYEQYIKWPGYIPEAPRDGQAYVRKDGEWVLLSTFLHHHHHH

SEQ ID NO: 26 - protein, 1242 aa, synthetic construct
MFVFLVLLPLVSSQCVNLITRTQSYTNSFTRGVYYPDKVFRSSVLHSTQDLFLPFFSNVTWFHAIHVSGTNGTKRFDNPALPFNDGVYFASTEKSNIIRGWIFGTTLDSKTQSLLIVNNATNVVIKVCEFQFCNDPFLDVYQKNNKSWMESEFRVYSSANNCTFEYVSQPFLMDLEGKEGNFKNLREFVFKNIDGYFKIYSKHTPINLERDLPQGFSALEPLVDLPIGINITRFQTLLALHRSYLTPVDSSSGWTAGAAAYYVGYLQPRTFLLKYNENGTITDAVDCALDPLSETKCTLKSFTVEKGIYQTSNFRVQPTESIVRFPQITNLCPFGEVFNATKFPSVYAWERKKISNCVADYSVLYNSTFFSTFKCYGVSATKLNDLCFSNVYADSFVVKGDDVRQIAPGQTGVIADYNYKLPDDFMGCVIAWNSNNLDSKVGGNYNYRYRLFRKSKLKPFERDISTEIYQAGSKPCNGVEGFNCYFPLQSYGFQPTYGVGYQPYRVVVLSFELLHAPATVCGPKKSTNLVKNKCVNFNFNGLTGTGVLTESNKKFLPFQQFGRDIADTTDAVRDPQTLEILDITPCSFGGVSVITPGTNTSNQVAVLYQGVNCTEVPVAIHADQLTPTWRVYSTGSNVFQTRAGCLIGAEHVNNSYECDIPIGAGICASYQTQTNSRGSASSVASQSIIAYTMSLGAENSVAYSNNSIAIPTNFTISVTTEILPVSMPKTSVDCTMYICGDSTECSNLLLQYGSFCTQLNRALTGIAVEQDKNTQEVFAQVKQIYKTPPIPDFGGFNFSQILPDPSKPSKRSPIEDLLFNKVTLADAGFIKQYGDCLGDIAARDLICAQKFNGLTVLPPLLTDEMIAQYTSALLAGTITSGWTFGAGPALQIPFPMQMAYRFNGIGVTQNVLYENQKLIANQFNSAIGKIQDSLSSTPSALGKLQNVVNQNAQALNTLVKCLSSNFGAISSVLNDILSRLDPPEAEVQIDRLITGRLQCLQTYVTQQLIRAAEIRASANLAATKMSECVLGQSKRVDFCGKGYHLMSFPQSAPHGVVFLHVTYVPAQEKNFTTAPAICHDGKAHFPREGVFVSNGTHWFVTQRNFYEPQIITTDNTFVSGNCDVVIGIVNNTVYDPLQPELDSFKEELDKYFKNHTSPDVDLGDISGILASVVNIQKEIDRLNEVAKNLNESLIDLQELGKYEQYIKWPGYIPEAPRDGQAYVRKDGEWVLLSTFLHHHHHH

SEQ ID NO: 27 - protein, 1242 aa, synthetic construct
MFVFLVLLPLVSSQCVNLITRTQSYTNSFTRGVYYPDKVFRSSVLHSTQDLFLPFFSNVTWFHAIHVSGTNGTKRFDNPALPFNDGVYFASTEKSNIIRGWIFGTTLDSKTQSLLIVNNATNVVIKVCEFQFCNDPFLDVYQKNNKSWMESEFRVYSSANNCTFEYVSQPFLMDLEGKEGNFKNLREFVFKNIDGYFKIYSKHTPINLERDLPQGFSALEPLVDLPIGINITRFQTLLALHRSYLTPVDSSSGWTAGAAAYYVGYLQPRTFLLKYNENGTITDAVDCALDPLSETKCTLKSFTVEKGIYQTSNFRVQPTESIVRFPQITNLCPFGEVFNATKFPSVYAWERKKISNCVADYSVLYNSTFFSTFKCYGVSATKLNDLCFSNVYADSFVVKGDDVRQIAPGQTGVIADYNYKLPDDFMGCVIAWNSNNLDSKVGGNYNYRYRLFRKSKLKPFERDISTEIYQAGNKPCNGVEGFNCYFPLQSYGFQPTYGVGYQPYRVVVLSFELLHAPATVCGPKKSTNLVKNKCVNFNFNGLTGTGVLTESNKKFLPFQQFGRDIADTTDAVRDPQTLEILDITPCSFGGVSVITPGTNTSNQVAVLYQGVNCTEVPVAIHADQLTPTWRVYSTGSNVFQTRAGCLIGAEHVNNSYECDIPIGAGICASYQTQTNSRGSASSVASQSIIAYTMSLGAENSVAYSNNSIAIPTNFTISVTTEILPVSMPKTSVDCTMYICGDSTECSNLLLQYGSFCTQLNRALTGIAVEQDKNTQEVFAQVKQIYKTPPIPDFGGFNFSQILPDPSKPSKRSPIEDLLFNKVTLADAGFIKQYGDCLGDIAARDLICAQKFNGLTVLPPLLTDEMIAQYTSALLAGTITSGWTFGAGPALQIPFPMQMAYRFNGIGVTQNVLYENQKLIANQFNSAIGKIQDSLSSTPSALGKLQNVVNQNAQALNTLVKCLSSNFGAISSVLNDILSRLDPPEAEVQIDRLITGRLQCLQTYVTQQLIRAAEIRASANLAATKMSECVLGQSKRVDFCGKGYHLMSFPQSAPHGVVFLHVTYVPAQEKNFTTAPAICHDGKAHFPREGVFVSNGTHWFVTQRNFYEPQIITTDNTFVSGNCDVVIGIVNNTVYDPLQPELDSFKEELDKYFKNHTSPDVDLGDISGILASVVNIQKEIDRLNEVAKNLNESLIDLQELGKYEQYIKWPGYIPEAPRDGQAYVRKDGEWVLLSTFLHHHHHH

SEQ ID NO: 28 - protein, 203 aa, synthetic construct
FPNITNLCPFGEVFNATRFASVYAWNRKRISNCVADYSVLYNSASFSTFKCYGVSPTKLNDLCFTNVYADSFVIRGDEVRQIAPGQTGKIADYNYKLPDDFTGCVIAWNSNNLDSKVGGNYNYRYRLFRKSNLKPFERDISTEIYQAGSKPCNGVEGFNCYFPLQSYGFQPTNGVGYQPYRVVVLSFELLHAPATVCGPKKST

SEQ ID NO: 29 - protein, 203 aa, synthetic construct
FPNITNLCPFGEVFNATRFASVYAWNRKRISNCVADYSVLYNSTFFSTFKCYGVSATKLNDLCFSNVYADSFVVKGDDVRQIAPGQTGKIADYNYKLPDDFTGCVIAWNSNNLDSKVGGNYNYRYRLFRKSNLKPFERDISTEIYQAGSKPCNGVEGFNCYFPLQSYGFYTTTGIGYQPYRVVVLSFELLNAPATVCGPKLST

SEQ ID NO: 30 - protein, 203 aa, synthetic construct
FPNITNLCPFGEVFNATRFASVYAWNRKRISNCVADYSVLYNSTFFSTFKCYGVSATKLNDLCFSNVYADSFVVKGDDVRQIAPGQTGVIADYNYKLPDDFMGCVIAWNSNNLDSKVGGNYNYRYRLFRKSNLKPFERDISTEIYQAGSKPCNGVEGFNCYFPLQSYGFQPTNGVGYQPYRVVVLSFELLHAPATVCGPKKST

SEQ ID NO: 31 - protein, 203 aa, synthetic construct
FPNITNLCPFGEVFNATRFASVYAWNRKRISNCVADYSVLYNSTFFSTFKCYGVSATKLNDLCFSNVYADSFVVKGDDVRQIAPGQTGVIADYNYKLPDDFMGCVLAWNTRNIDATSTGNYNYKYRLFRKSNLKPFERDISTEIYQAGSKPCNGVEGFNCYFPLQSYGFQPTNGVGYQPYRVVVLSFELLHAPATVCGPKKST

SEQ ID NO: 32 - protein, 203 aa, synthetic construct
FPNITNLCPFGEVFNATRFASVYAWNRKRISNCVADYSVLYNSTFFSTFKCYGVSATKLNDLCFSNVYADSFVVKGDDVRQIAPGQTGVIADYNYKLPDDFMGCVLAWNTRNIDATSTGNYNYKYRLFRKSNLKPFERDISTEIYQAGSKPCNGVEGFNCYFPLQSYGFYTTTGIGYQPYRVVVLSFELLNAPATVCGPKLST

SEQ ID NO: 33 - protein, 1244 aa, synthetic construct
MFVFLVLLPLVSSQCVNLRTRTQLPPAYTNSFTRGVYYPDKVFRSSVLHSTQDLFLPFFSNVTWFHAIHVSGTNGTKRFDNPVLPFNDGVYFASTEKSNIIRGWIFGTTLDSKTQSLLIVNNATNVVIKVCEFQFCNDPFLDVYYHKNNKSWMESGVYSSANNCTFEYVSQPFLMDLEGKQGNFKNLREFVFKNIDGYFKIYSKHTPINLVRDLPQGFSALEPLVDLPIGINITRFQTLLALHRSYLTPGDSSSGWTAGAAAYYVGYLQPRTFLLKYNENGTITDAVDCALDPLSETKCTLKSFTVEKGIYQTSNFRVQPTESIVRFPNITNLCPFGEVFNATRFASVYAWNRKRISNCVADYSVLYNSASFSTFKCYGVSPTKLNDLCFTNVYADSFVIRGDEVRQIAPGQTGKIADYNYKLPDDFTGCVIAWNSNNLDSKVGGNYNYRYRLFRKSNLKPFERDISTEIYQAGSKPCNGVEGFNCYFPLQSYGFQPTNGVGYQPYRVVVLSFELLHAPATVCGPKKSTNLVKNKCVNFNFNGLTGTGVLTESNKKFLPFQQFGRDIADTTDAVRDPQTLEILDITPCSFGGVSVITPGTNTSNQVAVLYQGVNCTEVPVAIHADQLTPTWRVYSTGSNVFQTRAGCLIGAEHVNNSYECDIPIGAGICASYQTQTNSRGSASSVASQSIIAYTMSLGAENSVAYSNNSIAIPTNFTISVTTEILPVSMTKTSVDCTMYICGDSTECSNLLLQYGSFCTQLNRALTGIAVEQDKNTQEVFAQVKQIYKTPPIKDFGGFNFSQILPDPSKPSKRSPIEDLLFNKVTLADAGFIKQYGDCLGDIAARDLICAQKFNGLTVLPPLLTDEMIAQYTSALLAGTITSGWTFGAGPALQIPFPMQMAYRFNGIGVTQNVLYENQKLIANQFNSAIGKIQDSLSSTPSALGKLQNVVNQNAQALNTLVKQLSSNFGAISSVLNDILSRLDPPEAEVQIDRLITGRLQSLQTYVTQQLIRAAEIRASANLAATKMSECVLGQSKRVDFCGKGYHLMSFPQSAPHGVVFLHVTYVPAQEKNFTTAPAICHDGKAHFPREGVFVSNGTHWFVTQRNFYEPQIITTDNTFVSGNCDVVIGIVNNTVYDPLQPELDSFKEELDKYFKNHTSPDVDLGDISGINASVVNIQKEIDRLNEVAKNLNESLIDLQELGKYEQYIKWPGYIPEAPRDGQAYVRKDGEWVLLSTFLHHHHHH

SEQ ID NO: 34 - protein, 1244 aa, synthetic construct
MFVFLVLLPLVSSQCVNLRTRTQLPPAYTNSFTRGVYYPDKVFRSSVLHSTQDLFLPFFSNVTWFHAIHVSGTNGTKRFDNPVLPFNDGVYFASTEKSNIIRGWIFGTTLDSKTQSLLIVNNATNVVIKVCEFQFCNDPFLDVYYHKNNKSWMESGVYSSANNCTFEYVSQPFLMDLEGKQGNFKNLREFVFKNIDGYFKIYSKHTPINLVRDLPQGFSALEPLVDLPIGINITRFQTLLALHRSYLTPGDSSSGWTAGAAAYYVGYLQPRTFLLKYNENGTITDAVDCALDPLSETKCTLKSFTVEKGIYQTSNFRVQPTESIVRFPNITNLCPFGEVFNATRFASVYAWNRKRISNCVADYSVLYNSTFFSTFKCYGVSATKLNDLCFSNVYADSFVVKGDDVRQIAPGQTGKIADYNYKLPDDFTGCVIAWNSNNLDSKVGGNYNYRYRLFRKSNLKPFERDISTEIYQAGSKPCNGVEGFNCYFPLQSYGFYTTTGIGYQPYRVVVLSFELLNAPATVCGPKLSTNLVKNKCVNFNFNGLTGTGVLTESNKKFLPFQQFGRDIADTTDAVRDPQTLEILDITPCSFGGVSVITPGTNTSNQVAVLYQGVNCTEVPVAIHADQLTPTWRVYSTGSNVFQTRAGCLIGAEHVNNSYECDIPIGAGICASYQTQTNSRGSASSVASQSIIAYTMSLGAENSVAYSNNSIAIPTNFTISVTTEILPVSMTKTSVDCTMYICGDSTECSNLLLQYGSFCTQLNRALTGIAVEQDKNTQEVFAQVKQIYKTPPIKDFGGFNFSQILPDPSKPSKRSPIEDLLFNKVTLADAGFIKQYGDCLGDIAARDLICAQKFNGLTVLPPLLTDEMIAQYTSALLAGTITSGWTFGAGPALQIPFPMQMAYRFNGIGVTQNVLYENQKLIANQFNSAIGKIQDSLSSTPSALGKLQNVVNQNAQALNTLVKQLSSNFGAISSVLNDILSRLDPPEAEVQIDRLITGRLQSLQTYVTQQLIRAAEIRASANLAATKMSECVLGQSKRVDFCGKGYHLMSFPQSAPHGVVFLHVTYVPAQEKNFTTAPAICHDGKAHFPREGVFVSNGTHWFVTQRNFYEPQIITTDNTFVSGNCDVVIGIVNNTVYDPLQPELDSFKEELDKYFKNHTSPDVDLGDISGINASVVNIQKEIDRLNEVAKNLNESLIDLQELGKYEQYIKWPGYIPEAPRDGQAYVRKDGEWVLLSTFLHHHHHH

SEQ ID NO: 35 - protein, 1244 aa, synthetic construct
MFVFLVLLPLVSSQCVNLRTRTQLPPAYTNSFTRGVYYPDKVFRSSVLHSTQDLFLPFFSNVTWFHAIHVSGTNGTKRFDNPVLPFNDGVYFASTEKSNIIRGWIFGTTLDSKTQSLLIVNNATNVVIKVCEFQFCNDPFLDVYYHKNNKSWMESGVYSSANNCTFEYVSQPFLMDLEGKQGNFKNLREFVFKNIDGYFKIYSKHTPINLVRDLPQGFSALEPLVDLPIGINITRFQTLLALHRSYLTPGDSSSGWTAGAAAYYVGYLQPRTFLLKYNENGTITDAVDCALDPLSETKCTLKSFTVEKGIYQTSNFRVQPTESIVRFPNITNLCPFGEVFNATRFASVYAWNRKRISNCVADYSVLYNSTFFSTFKCYGVSATKLNDLCFSNVYADSFVVKGDDVRQIAPGQTGVIADYNYKLPDDFMGCVIAWNSNNLDSKVGGNYNYRYRLFRKSNLKPFERDISTEIYQAGSKPCNGVEGFNCYFPLQSYGFQPTNGVGYQPYRVVVLSFELLHAPATVCGPKKSTNLVKNKCVNFNFNGLTGTGVLTESNKKFLPFQQFGRDIADTTDAVRDPQTLEILDITPCSFGGVSVITPGTNTSNQVAVLYQGVNCTEVPVAIHADQLTPTWRVYSTGSNVFQTRAGCLIGAEHVNNSYECDIPIGAGICASYQTQTNSRGSASSVASQSIIAYTMSLGAENSVAYSNNSIAIPTNFTISVTTEILPVSMTKTSVDCTMYICGDSTECSNLLLQYGSFCTQLNRALTGIAVEQDKNTQEVFAQVKQIYKTPPIKDFGGFNFSQILPDPSKPSKRSPIEDLLFNKVTLADAGFIKQYGDCLGDIAARDLICAQKFNGLTVLPPLLTDEMIAQYTSALLAGTITSGWTFGAGPALQIPFPMQMAYRFNGIGVTQNVLYENQKLIANQFNSAIGKIQDSLSSTPSALGKLQNVVNQNAQALNTLVKQLSSNFGAISSVLNDILSRLDPPEAEVQIDRLITGRLQSLQTYVTQQLIRAAEIRASANLAATKMSECVLGQSKRVDFCGKGYHLMSFPQSAPHGVVFLHVTYVPAQEKNFTTAPAICHDGKAHFPREGVFVSNGTHWFVTQRNFYEPQIITTDNTFVSGNCDVVIGIVNNTVYDPLQPELDSFKEELDKYFKNHTSPDVDLGDISGINASVVNIQKEIDRLNEVAKNLNESLIDLQELGKYEQYIKWPGYIPEAPRDGQAYVRKDGEWVLLSTFLHHHHHH

SEQ ID NO: 36 - protein, 1244 aa, synthetic construct
MFVFLVLLPLVSSQCVNLRTRTQLPPAYTNSFTRGVYYPDKVFRSSVLHSTQDLFLPFFSNVTWFHAIHVSGTNGTKRFDNPVLPFNDGVYFASTEKSNIIRGWIFGTTLDSKTQSLLIVNNATNVVIKVCEFQFCNDPFLDVYYHKNNKSWMESGVYSSANNCTFEYVSQPFLMDLEGKQGNFKNLREFVFKNIDGYFKIYSKHTPINLVRDLPQGFSALEPLVDLPIGINITRFQTLLALHRSYLTPGDSSSGWTAGAAAYYVGYLQPRTFLLKYNENGTITDAVDCALDPLSETKCTLKSFTVEKGIYQTSNFRVQPTESIVRFPNITNLCPFGEVFNATRFASVYAWNRKRISNCVADYSVLYNSTFFSTFKCYGVSATKLNDLCFSNVYADSFVVKGDDVRQIAPGQTGVIADYNYKLPDDFMGCVLAWNTRNIDATSTGNYNYKYRLFRKSNLKPFERDISTEIYQAGSKPCNGVEGFNCYFPLQSYGFQPTNGVGYQPYRVVVLSFELLHAPATVCGPKKSTNLVKNKCVNFNFNGLTGTGVLTESNKKFLPFQQFGRDIADTTDAVRDPQTLEILDITPCSFGGVSVITPGTNTSNQVAVLYQGVNCTEVPVAIHADQLTPTWRVYSTGSNVFQTRAGCLIGAEHVNNSYECDIPIGAGICASYQTQTNSRGSASSVASQSIIAYTMSLGAENSVAYSNNSIAIPTNFTISVTTEILPVSMTKTSVDCTMYICGDSTECSNLLLQYGSFCTQLNRALTGIAVEQDKNTQEVFAQVKQIYKTPPIKDFGGFNFSQILPDPSKPSKRSPIEDLLFNKVTLADAGFIKQYGDCLGDIAARDLICAQKFNGLTVLPPLLTDEMIAQYTSALLAGTITSGWTFGAGPALQIPFPMQMAYRFNGIGVTQNVLYENQKLIANQFNSAIGKIQDSLSSTPSALGKLQNVVNQNAQALNTLVKQLSSNFGAISSVLNDILSRLDPPEAEVQIDRLITGRLQSLQTYVTQQLIRAAEIRASANLAATKMSECVLGQSKRVDFCGKGYHLMSFPQSAPHGVVFLHVTYVPAQEKNFTTAPAICHDGKAHFPREGVFVSNGTHWFVTQRNFYEPQIITTDNTFVSGNCDVVIGIVNNTVYDPLQPELDSFKEELDKYFKNHTSPDVDLGDISGINASVVNIQKEIDRLNEVAKNLNESLIDLQELGKYEQYIKWPGYIPEAPRDGQAYVRKDGEWVLLSTFLHHHHHH

SEQ ID NO: 37 - protein, 1244 aa, synthetic construct
MFVFLVLLPLVSSQCVNLRTRTQLPPAYTNSFTRGVYYPDKVFRSSVLHSTQDLFLPFFSNVTWFHAIHVSGTNGTKRFDNPVLPFNDGVYFASTEKSNIIRGWIFGTTLDSKTQSLLIVNNATNVVIKVCEFQFCNDPFLDVYYHKNNKSWMESGVYSSANNCTFEYVSQPFLMDLEGKQGNFKNLREFVFKNIDGYFKIYSKHTPINLVRDLPQGFSALEPLVDLPIGINITRFQTLLALHRSYLTPGDSSSGWTAGAAAYYVGYLQPRTFLLKYNENGTITDAVDCALDPLSETKCTLKSFTVEKGIYQTSNFRVQPTESIVRFPNITNLCPFGEVFNATRFASVYAWNRKRISNCVADYSVLYNSTFFSTFKCYGVSATKLNDLCFSNVYADSFVVKGDDVRQIAPGQTGVIADYNYKLPDDFMGCVLAWNTRNIDATSTGNYNYKYRLFRKSNLKPFERDISTEIYQAGSKPCNGVEGFNCYFPLQSYGFYTTTGIGYQPYRVVVLSFELLNAPATVCGPKLSTNLVKNKCVNFNFNGLTGTGVLTESNKKFLPFQQFGRDIADTTDAVRDPQTLEILDITPCSFGGVSVITPGTNTSNQVAVLYQGVNCTEVPVAIHADQLTPTWRVYSTGSNVFQTRAGCLIGAEHVNNSYECDIPIGAGICASYQTQTNSRGSASSVASQSIIAYTMSLGAENSVAYSNNSIAIPTNFTISVTTEILPVSMTKTSVDCTMYICGDSTECSNLLLQYGSFCTQLNRALTGIAVEQDKNTQEVFAQVKQIYKTPPIKDFGGFNFSQILPDPSKPSKRSPIEDLLFNKVTLADAGFIKQYGDCLGDIAARDLICAQKFNGLTVLPPLLTDEMIAQYTSALLAGTITSGWTFGAGPALQIPFPMQMAYRFNGIGVTQNVLYENQKLIANQFNSAIGKIQDSLSSTPSALGKLQNVVNQNAQALNTLVKQLSSNFGAISSVLNDILSRLDPPEAEVQIDRLITGRLQSLQTYVTQQLIRAAEIRASANLAATKMSECVLGQSKRVDFCGKGYHLMSFPQSAPHGVVFLHVTYVPAQEKNFTTAPAICHDGKAHFPREGVFVSNGTHWFVTQRNFYEPQIITTDNTFVSGNCDVVIGIVNNTVYDPLQPELDSFKEELDKYFKNHTSPDVDLGDISGINASVVNIQKEIDRLNEVAKNLNESLIDLQELGKYEQYIKWPGYIPEAPRDGQAYVRKDGEWVLLSTFLHHHHHH

SEQ ID NO: 38 - protein, 1244 aa, synthetic construct
MFVFLVLLPLVSSQCVNLRTRTQLPPAYTNSFTRGVYYPDKVFRSSVLHSTQDLFLPFFSNVTWFHAIHVSGTNGTKRFDNPVLPFNDGVYFASTEKSNIIRGWIFGTTLDSKTQSLLIVNNATNVVIKVCEFQFCNDPFLDVYYHKNNKSWMESGVYSSANNCTFEYVSQPFLMDLEGKQGNFKNLREFVFKNIDGYFKIYSKHTPINLVRDLPQGFSALEPLVDLPIGINITRFQTLLALHRSYLTPGDSSSGWTAGAAAYYVGYLQPRTFLLKYNENGTITDAVDCALDPLSETKCTLKSFTVEKGIYQTSNFRVQPTESIVRFPNITNLCPFGEVFNATKFPSVYAWERKKISNCVADYSVLYNSTFFSTFKCYGVSATKLNDLCFSNVYADSFVVKGDDVRQIAPGQTGVIADYNYKLPDDFMGCVIAWNSNNLDSKVGGNYNYRYRLFRKSNLKPFERDISTEIYQAGSKPCNGVEGFNCYFPLQSYGFQPTNGVGYQPYRVVVLSFELLHAPATVCGPKKSTNLVKNKCVNFNFNGLTGTGVLTESNKKFLPFQQFGRDIADTTDAVRDPQTLEILDITPCSFGGVSVITPGTNTSNQVAVLYQGVNCTEVPVAIHADQLTPTWRVYSTGSNVFQTRAGCLIGAEHVNNSYECDIPIGAGICASYQTQTNSRGSASSVASQSIIAYTMSLGAENSVAYSNNSIAIPTNFTISVTTEILPVSMTKTSVDCTMYICGDSTECSNLLLQYGSFCTQLNRALTGIAVEQDKNTQEVFAQVKQIYKTPPIKDFGGFNFSQILPDPSKPSKRSPIEDLLFNKVTLADAGFIKQYGDCLGDIAARDLICAQKFNGLTVLPPLLTDEMIAQYTSALLAGTITSGWTFGAGPALQIPFPMQMAYRFNGIGVTQNVLYENQKLIANQFNSAIGKIQDSLSSTPSALGKLQNVVNQNAQALNTLVKQLSSNFGAISSVLNDILSRLDPPEAEVQIDRLITGRLQSLQTYVTQQLIRAAEIRASANLAATKMSECVLGQSKRVDFCGKGYHLMSFPQSAPHGVVFLHVTYVPAQEKNFTTAPAICHDGKAHFPREGVFVSNGTHWFVTQRNFYEPQIITTDNTFVSGNCDVVIGIVNNTVYDPLQPELDSFKEELDKYFKNHTSPDVDLGDISGINASVVNIQKEIDRLNEVAKNLNESLIDLQELGKYEQYIKWPGYIPEAPRDGQAYVRKDGEWVLLSTFLHHHHHH

SEQ ID NO: 39 - protein, 4 aa, synthetic construct
QQAQ

SEQ ID NO: 40 - protein, 245 aa, synthetic construct
MIHSVFLLMFLLTPTESYVDITNLCPFGEVFNATRFASVYAWNRKRISNCVADYSVLYNSASFSTFKCYGVSPTKLNDLCFTNVYADSFVIRGDEVRQIAPGQTGKIADYNYKLPDDFTGCVIAWNSNNLDSKVGGNYNYRYRLFRKSNLKPFERDISTEIYQAGSKPCNGVEGFNCYFPLQSYGFQPTNGVGYQPYRVVVLSFELLHAPATVCGPKKSTHHHHHHGSGSGLNDIFEAQKIEWHE

SEQ ID NO: 41 - protein, 247 aa, synthetic construct
MIHSVFLLMFLLTPTESYVDFPNITNLCPFGEVFNATKFPSVYAWERKKISNCVADYSVLYNSTFFSTFKCYGVSATKLNDLCFSNVYADSFVVKGDDVRQIAPGQTGVIADYNYKLPDDFMGCVLAWNTRNIDATSTGNYNYKYRYLRHGKLRPFERDISNVPFSPDGKPCTPPALNCYWPLNDYGFYTTTGIGYQPYRVVVLSFELLNAPATVCGPKLSTHHHHHHGSGSGLNDIFEAQKIEWHE

SEQ ID NO: 42 - protein, 248 aa, synthetic construct
MIHSVFLLMFLLTPTESYVDFPNITNLCPFGEVFNATRFASVYAWNRKRISNCVADYSVLYNSTFFSTFKCYGVSATKLNDLCFSNVYADSFVVKGDDVRQIAPGQTGKIADYNYKLPDDFTGCVIAWNSNNLDSKVGGNYNYRYRLFRKSNLKPFERDISTEIYQAGSKPCNGVEGFNCYFPLQSYGFYTTTGIGYQPYRVVVLSFELLNAPATVCGPKLSTHHHHHHGSGSGLNDIFEAQKIEWHE

SEQ ID NO: 43 - protein, 248 aa, synthetic construct
MIHSVFLLMFLLTPTESYVDFPNITNLCPFGEVFNATRFASVYAWNRKRISNCVADYSVLYNSTFFSTFKCYGVSATKLNDLCFSNVYADSFVVKGDDVRQIAPGQTGVIADYNYKLPDDFMGCVIAWNSNNLDSKVGGNYNYRYRLFRKSNLKPFERDISTEIYQAGSKPCNGVEGFNCYFPLQSYGFQPTNGVGYQPYRVVVLSFELLHAPATVCGPKKSTHHHHHHGSGSGLNDIFEAQKIEWHE

SEQ ID NO: 44 - protein, 248 aa, synthetic construct
MIHSVFLLMFLLTPTESYVDFPNITNLCPFGEVFNATRFASVYAWNRKRISNCVADYSVLYNSTFFSTFKCYGVSATKLNDLCFSNVYADSFVVKGDDVRQIAPGQTGVIADYNYKLPDDFMGCVLAWNTRNIDATSTGNYNYKYRLFRKSNLKPFERDISTEIYQAGSKPCNGVEGFNCYFPLQSYGFYTTTGIGYQPYRVVVLSFELLNAPATVCGPKLSTHHHHHHGSGSGLNDIFEAQKIEWHE

SEQ ID NO: 45 - protein, 248 aa, synthetic construct
MIHSVFLLMFLLTPTESYVDFPNITNLCPFGEVFNATKFPSVYAWERKKISNCVADYSVLYNSTFFSTFKCYGVSATKLNDLCFSNVYADSFVVKGDDVRQIAPGQTGVIADYNYKLPDDFMGCVIAWNSNNLDSKVGGNYNYRYRLFRKSNLKPFERDISTEIYQAGSKPCNGVEGFNCYFPLQSYGFQPTNGVGYQPYRVVVLSFELLHAPATVCGPKKSTHHHHHHGSGSGLNDIFEAQKIEWHE

SEQ ID NO: 46 - protein, 1241 aa, synthetic construct
MFVFLVLLPLVSSQCVNLITRTQSYTNSFTRGVYYPDKVFRSSVLHSTQDLFLPFFSNVTWFHAISGTNGTKRFDNPVLPFNDGVYFASTEKSNIIRGWIFGTTLDSKTQSLLIVNNATNVVIKVCEFQFCNDPFLDVYYHKNNKSWMESEFRVYSSANNCTFEYVSQPFLMDLEGKQGNFKNLREFVFKNIDGYFKIYSKHTPINLGRDLPQGFSALEPLVDLPIGINITRFQTLLALHRSYLTPGDSSSGWTAGAAAYYVGYLQPRTFLLKYNENGTITDAVDCALDPLSETKCTLKSFTVEKGIYQTSNFRVQPTESIVRFPNITNLCPFGEVFNATRFASVYAWNRKRISNCVADYSVLYNSASFSTFKCYGVSPTKLNDLCFTNVYADSFVIRGDEVRQIAPGQTGKIADYNYKLPDDFTGCVIAWNSNNLDSKVGGNYNYRYRLFRKSNLKPFERDISTEIYQAGSKPCNGVEGFNCYFPLQSYGFQPTNGVGYQPYRVVVLSFELLHAPATVCGPKKSTNLVKNKCVNFNFNGLTGTGVLTESNKKFLPFQQFGRDIADTTDAVRDPQTLEILDITPCSFGGVSVITPGTNTSNQVAVLYQGVNCTEVPVAIHADQLTPTWRVYSTGSNVFQTRAGCLIGAEHVNNSYECDIPIGAGICASYQTQTNSRGSASSVASQSIIAYTMSLGAENSVAYSNNSIAIPTNFTISVTTEILPVSMTKTSVDCTMYICGDSTECSNLLLQYGSFCTQLNRALTGIAVEQDKNTQEVFAQVKQIYKTPPIKDFGGFNFSQILPDPSKPSKRSPIEDLLFNKVTLADAGFIKQYGDCLGDIAARDLICAQKFNGLTVLPPLLTDEMIAQYTSALLAGTITSGWTFGAGPALQIPFPMQMAYRFNGIGVTQNVLYENQKLIANQFNSAIGKIQDSLSSTPSALGKLQNVVNQNAQALNTLVKQLSSNFGAISSVLNDILSRLDPPEAEVQIDRLITGRLQSLQTYVTQQLIRAAEIRASANLAATKMSECVLGQSKRVDFCGKGYHLMSFPQSAPHGVVFLHVTYVPAQEKNFTTAPAICHDGKAHFPREGVFVSNGTHWFVTQRNFYEPQIITTDNTFVSGNCDVVIGIVNNTVYDPLQPELDSFKEELDKYFKNHTSPDVDLGDISGINASVVNIQKEIDRLNEVAKNLNESLIDLQELGKYEQYIKWPGYIPEAPRDGQAYVRKDGEWVLLSTFLHHHHHH

SEQ ID NO: 47 - protein, 1233 aa, synthetic construct
MFIFLLFLTLTSGSDLDRCTTFDDVQAPNYTQHTSSMRGVYYPDEIFRSDTLYLTQDLFLPFYSNVTGFHTINHTFGNPVIPFKDGIYFAATEKSNVVRGWVFGSTMNNKSQSVIIINNSTNVVIRACNFELCDNPFFAVSKPMGTQTHTMIFDNAFNCTFEYISDAFSLDVSEKSGNFKHLREFVFKNKDGFLYVYKGYQPIDVVRDLPSGFNTLKPIFKLPLGINITNFRAILTAFSPAQDIWGTSAAAYFVGYLKPTTFMLKYDENGTITDAVDCSQNPLAELKCSVKSFEIDKGIYQTSNFRVVPSGDVVRFPNITNLCPFGEVFNATRFASVYAWNRKRISNCVADYSVLYNSASFSTFKCYGVSPTKLNDLCFTNVYADSFVIRGDEVRQIAPGQTGKIADYNYKLPDDFTGCVIAWNSNNLDSKVGGNYNYRYRLFRKSNLKPFERDISTEIYQAGSKPCNGVEGFNCYFPLQSYGFQPTNGVGYQPYRVVVLSFELLHAPATVCGPKKSTNLVKNKCVNFNFNGLTGTGVLTESNKKFLPFQQFGRDIADTTDAVRDPQTLEILDITPCSFGGVSVITPGTNTSNQVAVLYQGVNCTEVPVAIHADQLTPTWRVYSTGSNVFQTRAGCLIGAEHVNNSYECDIPIGAGICASYQTQTNSRGSASSVASQSIIAYTMSLGAENSVAYSNNSIAIPTNFTISVTTEILPVSMTKTSVDCTMYICGDSTECSNLLLQYGSFCTQLNRALTGIAVEQDKNTQEVFAQVKQIYKTPPIKDFGGFNFSQILPDPSKPSKRSPIEDLLFNKVTLADAGFIKQYGDCLGDIAARDLICAQKFNGLTVLPPLLTDEMIAQYTSALLAGTITSGWTFGAGPALQIPFPMQMAYRFNGIGVTQNVLYENQKLIANQFNSAIGKIQDSLSSTPSALGKLQNVVNQNAQALNTLVKQLSSNFGAISSVLNDILSRLDPPEAEVQIDRLITGRLQSLQTYVTQQLIRAAEIRASANLAATKMSECVLGQSKRVDFCGKGYHLMSFPQSAPHGVVFLHVTYVPAQEKNFTTAPAICHDGKAHFPREGVFVSNGTHWFVTQRNFYEPQIITTDNTFVSGNCDVVIGIVNNTVYDPLQPELDSFKEELDKYFKNHTSPDVDLGDISGINASVVNIQKEIDRLNEVAKNLNESLIDLQELGKYEQYIKWPGYIPEAPRDGQAYVRKDGEWVLLSTFLHHHHHH

SEQ ID NO: 48 - protein, 1241 aa, synthetic construct
MFVFLVLLPLVSSQCVNLITRTQSYTNSFTRGVYYPDKVFRSSVLHSTQDLFLPFFSNVTWFHAISGTNGTKRFDNPVLPFNDGVYFASTEKSNIIRGWIFGTTLDSKTQSLLIVNNATNVVIKVCEFQFCNDPFLDVYYHKNNKSWMESEFRVYSSANNCTFEYVSQPFLMDLEGKQGNFKNLREFVFKNIDGYFKIYSKHTPINLGRDLPQGFSALEPLVDLPIGINITRFQTLLALHRSYLTPGDSSSGWTAGAAAYYVGYLQPRTFLLKYNENGTITDAVDCALDPLSETKCTLKSFTVEKGIYQTSNFRVQPTESIVRFPNITNLCPFGEVFNATRFASVYAWNRKRISNCVADYSVLYNSASFSTFKCYGVSPTKLNDLCFTNVYADSFVIRGDEVRQIAPGQTGKIADYNYKLPDDFTGCVIAWNSNNLDSKVGGNYNYRYRLFRKSNLKPFERDISTEIYQAGSKPCNGVEGFNCYFPLQSYGFQPTNGVGYQPYRVVVLSFELLHAPATVCGPKKSTNLVKNKCVNFNFNGLTGTGVLTESNKKFLPFQQFGRDIADTTDAVRDPQTLEILDITPCSFGGVSVITPGTNTSNQVAVLYQGVNCTEVPVAIHADQLTPTWRVYSTGSNVFQTRAGCLIGAEYVNNSYECDIPIGAGICASYQTQTKSHGSASSVASQSIIAYTMSLGAENSVAYSNNSIAIPTNFTISVTTEILPVSMTKTSVDCTMYICGDSTECSNLLLQYGSFCTQLKRALTGIAVEQDKNTQEVFAQVKQIYKTPPIKYFGGFNFSQILPDPSKPSKRSPIEDLLFNKVTLADAGFIKQYGDCLGDIAARDLICAQKFNGLTVLPPLLTDEMIAQYTSALLAGTITSGWTFGAGPALQIPFPMQMAYRFNGIGVTQNVLYENQKLIANQFNSAIGKIQDSLSSTPSALGKLQDVVNHNAQALNTLVKQLSSKFGAISSVLNDILSRLDPPEAEVQIDRLITGRLQSLQTYVTQQLIRAAEIRASANLAATKMSECVLGQSKRVDFCGKGYHLMSFPQSAPHGVVFLHVTYVPAQEKNFTTAPAICHDGKAHFPREGVFVSNGTHWFVTQRNFYEPQIITTDNTFVSGNCDVVIGIVNNTVYDPLQPELDSFKEELDKYFKNHTSPDVDLGDISGINASVVNIQKEIDRLNEVAKNLNESLIDLQELGKYEQYIKWPGYIPEAPRDGQAYVRKDGEWVLLSTFLHHHHHH

SEQ ID NO: 49 - protein, 1241 aa, synthetic construct
MFVFLVLLPLVSSQCVNLITRTQSYTNSFTRGVYYPDKVFRSSVLHSTQDLFLPFFSNVTWFHAISGTNGTKRFDNPVLPFNDGVYFASTEKSNIIRGWIFGTTLDSKTQSLLIVNNATNVVIKVCEFQFCNDPFLDVYYHKNNKSWMESEFRVYSSANNCTFEYVSQPFLMDLEGKQGNFKNLREFVFKNIDGYFKIYSKHTPINLGRDLPQGFSALEPLVDLPIGINITRFQTLLALHRSYLTPGDSSSGWTAGAAAYYVGYLQPRTFLLKYNENGTITDAVDCALDPLSETKCTLKSFTVEKGIYQTSNFRVQPTESIVRFPNITNLCPFGEVFNATKFPSVYAWERKKISNCVADYSVLYNSTFFSTFKCYGVSATKLNDLCFSNVYADSFVVKGDDVRQIAPGQTGVIADYNYKLPDDFMGCVIAWNSNNLDSKVGGNYNYRYRLFRKSNLKPFERDISTEIYQAGSKPCNGVEGFNCYFPLQSYGFQPTNGVGYQPYRVVVLSFELLHAPATVCGPKKSTNLVKNKCVNFNFNGLTGTGVLTESNKKFLPFQQFGRDIADTTDAVRDPQTLEILDITPCSFGGVSVITPGTNTSNQVAVLYQGVNCTEVPVAIHADQLTPTWRVYSTGSNVFQTRAGCLIGAEYVNNSYECDIPIGAGICASYQTQTKSHGSASSVASQSIIAYTMSLGAENSVAYSNNSIAIPTNFTISVTTEILPVSMTKTSVDCTMYICGDSTECSNLLLQYGSFCTQLKRALTGIAVEQDKNTQEVFAQVKQIYKTPPIKYFGGFNFSQILPDPSKPSKRSPIEDLLFNKVTLADAGFIKQYGDCLGDIAARDLICAQKFNGLTVLPPLLTDEMIAQYTSALLAGTITSGWTFGAGPALQIPFPMQMAYRFNGIGVTQNVLYENQKLIANQFNSAIGKIQDSLSSTPSALGKLQDVVNHNAQALNTLVKQLSSKFGAISSVLNDILSRLDPPEAEVQIDRLITGRLQSLQTYVTQQLIRAAEIRASANLAATKMSECVLGQSKRVDFCGKGYHLMSFPQSAPHGVVFLHVTYVPAQEKNFTTAPAICHDGKAHFPREGVFVSNGTHWFVTQRNFYEPQIITTDNTFVSGNCDVVIGIVNNTVYDPLQPELDSFKEELDKYFKNHTSPDVDLGDISGINASVVNIQKEIDRLNEVAKNLNESLIDLQELGKYEQYIKWPGYIPEAPRDGQAYVRKDGEWVLLSTFLHHHHHH

SEQ ID NO: 50 - protein, 1241 aa, synthetic construct
MFVFLVLLPLVSSQCVNLITRTQSYTNSFTRGVYYPDKVFRSSVLHSTQDLFLPFFSNVTWFHAISGTNGTKRFDNPVLPFNDGVYFASTEKSNIIRGWIFGTTLDSKTQSLLIVNNATNVVIKVCEFQFCNDPFLDVYYHKNNKSWMESEFRVYSSANNCTFEYVSQPFLMDLEGKQGNFKNLREFVFKNIDGYFKIYSKHTPINLGRDLPQGFSALEPLVDLPIGINITRFQTLLALHRSYLTPGDSSSGWTAGAAAYYVGYLQPRTFLLKYNENGTITDAVDCALDPLSETKCTLKSFTVEKGIYQTSNFRVQPTESIVRFPNITNLCPFGEVFNATRFASVYAWNRKRISNCVADYSVLYNSTFFSTFKCYGVSATKLNDLCFSNVYADSFVVKGDDVRQIAPGQTGVIADYNYKLPDDFMGCVLAWNTRNIDATSTGNYNYKYRLFRKSNLKPFERDISTEIYQAGSKPCNGVEGFNCYFPLQSYGFYTTTGIGYQPYRVVVLSFELLNAPATVCGPKLSTNLVKNKCVNFNFNGLTGTGVLTESNKKFLPFQQFGRDIADTTDAVRDPQTLEILDITPCSFGGVSVITPGTNTSNQVAVLYQGVNCTEVPVAIHADQLTPTWRVYSTGSNVFQTRAGCLIGAEYVNNSYECDIPIGAGICASYQTQTKSHGSASSVASQSIIAYTMSLGAENSVAYSNNSIAIPTNFTISVTTEILPVSMTKTSVDCTMYICGDSTECSNLLLQYGSFCTQLKRALTGIAVEQDKNTQEVFAQVKQIYKTPPIKYFGGFNFSQILPDPSKPSKRSPIEDLLFNKVTLADAGFIKQYGDCLGDIAARDLICAQKFNGLTVLPPLLTDEMIAQYTSALLAGTITSGWTFGAGPALQIPFPMQMAYRFNGIGVTQNVLYENQKLIANQFNSAIGKIQDSLSSTPSALGKLQDVVNHNAQALNTLVKQLSSKFGAISSVLNDILSRLDPPEAEVQIDRLITGRLQSLQTYVTQQLIRAAEIRASANLAATKMSECVLGQSKRVDFCGKGYHLMSFPQSAPHGVVFLHVTYVPAQEKNFTTAPAICHDGKAHFPREGVFVSNGTHWFVTQRNFYEPQIITTDNTFVSGNCDVVIGIVNNTVYDPLQPELDSFKEELDKYFKNHTSPDVDLGDISGINASVVNIQKEIDRLNEVAKNLNESLIDLQELGKYEQYIKWPGYIPEAPRDGQAYVRKDGEWVLLSTFLHHHHHH

SEQ ID NO: 51 - protein, 1244 aa, synthetic construct
MFVFLVLLPLVSSQCVNLRTRTQLPPAYTNSFTRGVYYPDKVFRSSVLHSTQDLFLPFFSNVTWFHAIHVSGTNGTKRFDNPVLPFNDGVYFASTEKSNIIRGWIFGTTLDSKTQSLLIVNNATNVVIKVCEFQFCNDPFLDVYYHKNNKSWMESGVYSSANNCLFEYVSQPFLMDLEGKQGNFKNLREFVFKNIDGYFKIYSKHTPINLVRDLPQGFSALEPLVDLPIGINITRFQTLLALHRSYLTPGDSSSGWTAGAAAYYVGYLQPRTFLLKYNENGTITDAVDCALDPLSETKCTLKSFTVEKGIYQTSNFRVQPTESIVRFPNITNLCPFGEVFNATRFASVYAWNRKRISNCVADYSVLYNSASFSTFKCYGVSPTKLNDLCFTNVYADSFVIRGDEVRQIAPGQTGKIADYNYKLPDDFTGCVIAWNSNNLDSKVGGNYNYRYRLFRKSNLKPFERDISTEIYQAGSKPCNGVEGFNCYFPLQSYGFQPTNGVGYQPYRVVVLSFELLHAPATVCGPKKSTNLVKNKCVNFNFNGLTGTGVLTESNKKFLPFQQFGRDIADTTDAVRDPQTLEILDITPCSFGGVSVITPGTNTSNQVAVLYQGVNCTEVPVAIHADQLTPTWRVYSTGSNVFQTRAGCLIGAEHVNNSYECDIPIGAGICASYQTQTNSRGSASSVASQSIIAYTMSLGAENSVAYSNNSIAIPTNFTISVTTEILPVSMTKTSVDCTMYICGDSTECSNLLLQYGSFCTQLNRALTGIAVEQDKNTQEVFAQVKQIYKTPPIKDFGGFNFSQILPDPSKPSKRSPIEDLLFNKVTLADAGFIKQYGDCLGDIAARDLICAQKFNGLTVLPPLLTDEMIAQYTSALLAGTITSGWTFGAGPALQIPFPMQMAYRFNGIGVTQNVLYENQKLIANQFNSAIGKIQDSLSSTPSALGKLQNVVNQNAQALNTLVKQLSSNFGAISSVLNDILSRLDPPEAEVQIDRLITGRLQSLQTYVTQQLIRAAEIRASANLAATKMSECVLGQSKRVDFCGKGYHLMSFPQSAPHGVVFLHVTYVPAQEKNFTTAPAICHDGKAHFPREGVFVSNGTHWFVTQRNFYEPQIITTDNTFVSGNCDVVIGIVNNTVYDPLQPELDSFKEELDKYFKNHTSPDVDLGDISGINASVVNIQKEIDRLNEVAKNLNESLIDLQELGKYEQYIKWPGYIPEAPRDGQAYVRKDGEWVLLSTFLHHHHHH

SEQ ID NO: 52 - protein, 1244 aa, synthetic construct
MFVFLVLLPLVSSQCVNLRTRTQLPPAYTNSFTRGVYYPDKVFRSSVLHSTQDLFLPFFSNVTWFHAIHVSGTNGTKRFDNPVLPFNDGVYFASTEKSNIIRGWIFGTTLDSKTQSLLIVNNATNVVIKVCEFQFCNDPFLDVYYHKNNKSWMESGVYSSANNCTFEYVSQPFLMDLEGKQGNFKNLREFVFKNIDGYFKIYSKHTPINLVRDLPQGFSALEPLVDLPIGINITRFQTLLALHRSYLTPGDSSSGWTAGAAAYYVGYLQPRTFLLKYNENGTITDAVDCALDPLSETKCTLKSFTVEKGIYQTSNFRVQPTESIVRFPQITNLCPFGEVFNATRFASVYAWNRKRISNCVADYSVLYNSASFSTFKCYGVSPTKLNDLCFTNVYADSFVIRGDEVRQIAPGQTGKIADYNYKLPDDFTGCVIAWNSNNLDSKVGGNYNYRYRLFRKSNLKPFERDISTEIYQAGSKPCNGVEGFNCYFPLQSYGFQPTNGVGYQPYRVVVLSFELLHAPATVCGPKKSTNLVKNKCVNFNFNGLTGTGVLTESNKKFLPFQQFGRDIADTTDAVRDPQTLEILDITPCSFGGVSVITPGTNTSNQVAVLYQGVNCTEVPVAIHADQLTPTWRVYSTGSNVFQTRAGCLIGAEHVNNSYECDIPIGAGICASYQTQTNSRGSASSVASQSIIAYTMSLGAENSVAYSNNSIAIPTNFTISVTTEILPVSMTKTSVDCTMYICGDSTECSNLLLQYGSFCTQLNRALTGIAVEQDKNTQEVFAQVKQIYKTPPIKDFGGFNFSQILPDPSKPSKRSPIEDLLFNKVTLADAGFIKQYGDCLGDIAARDLICAQKFNGLTVLPPLLTDEMIAQYTSALLAGTITSGWTFGAGPALQIPFPMQMAYRFNGIGVTQNVLYENQKLIANQFNSAIGKIQDSLSSTPSALGKLQNVVNQNAQALNTLVKQLSSNFGAISSVLNDILSRLDPPEAEVQIDRLITGRLQSLQTYVTQQLIRAAEIRASANLAATKMSECVLGQSKRVDFCGKGYHLMSFPQSAPHGVVFLHVTYVPAQEKNFTTAPAICHDGKAHFPREGVFVSNGTHWFVTQRNFYEPQIITTDNTFVSGNCDVVIGIVNNTVYDPLQPELDSFKEELDKYFKNHTSPDVDLGDISGINASVVNIQKEIDRLNEVAKNLNESLIDLQELGKYEQYIKWPGYIPEAPRDGQAYVRKDGEWVLLSTFLHHHHHH

SEQ ID NO: 53 - protein, 1244 aa, synthetic construct
MFVFLVLLPLVSSQCVNLRTRTQLPPAYTNSFTRGVYYPDKVFRSSVLHSTQDLFLPFFSNVTWFHAIHVSGTNGTKRFDNPVLPFNDGVYFASTEKSNIIRGWIFGTTLDSKTQSLLIVNNATNVVIKVCEFQFCNDPFLDVYYHKNNKSWMESGVYSSANNCTFEYVSQPFLMDLEGKQGNFKNLREFVFKNIDGYFKIYSKHTPINLVRDLPQGFSALEPLVDLPIGINITRFQTLLALHRSYLTPGDSSSGWTAGAAAYYVGYLQPRTFLLKYNENGTITDAVDCALDPLSETKCTLKSFTVEKGIYQTSNFRVQPTESIVRFPNITNLCPFGEVFNATRFASVYAWNRKRISNCVADYSVLYNSASFSTFKCYGVSPTKLNDLCFTNVYADSFVIRGDEVRQIAPGQTGKIADYNYKLPDDFTGCVIAWNSNNLDSKVGGNYNYRYRLFRKSNLKPFERDISTEIYQAGSKPCNGVEGFNCYFPLQSYGFQPTNGVGYQPYRVVVLSFELLHAPATVCGPKKSTNLVKNKCVNFNFNGLTGTGVLTESNKKFLPFQQFGRDIADTTDAVRDPQTLEILDITPCSFGGVSVITPGTNTSNQVAVLYQGVNCTEVPVAIHADQLTPTWRVYSTGSNVFQTRAGCLIGAEHVNNSYECDIPIGAGICASYQTQTNSRGSASSVASQSIIAYTMSLGAENSVAYSNNSIAIPTNFTISVTTEILPVSMTKTSVDCTMYICGDSTECSNLLLQYGSFCTQLNRALTGIAVEQDKNTQEVFAQVKQIYKTPPIKDFGGFNFSQILPDPSKPSKRSPIEDLLFNKVTLADAGFIKQYGDCLGDIAARDLICAQKFNGLTVLPPLLTDEMIAQYTSALLAGTITSGWTFGAGPALQIPFPMQMAYRFNGIGVTQNVLYENQKLIANQFNSAIGKIQDSLSSTPSALGKLQNVVNQNAQALNTLVKQLSSNFGAISSVLNDILSRLDPPEAEVQIDRLITGRLQSLQTYVTQQLIRAAEIRASANLAATKMSECVLGQSKRVDFCGKGYHLMSFPQSAPHGVVFLHVTYVPAQEKNFTTAPAICHDGKAHFPREGVFVSNGTHWFVTQRNFYEPQIITTDNTFVSGNCDVVIGIVNNTVYDPLQPELDSFKEELDKYFKNHTSPDVDLGDISGILASVVNIQKEIDRLNEVAKNLNESLIDLQELGKYEQYIKWPGYIPEAPRDGQAYVRKDGEWVLLSTFLHHHHHH

SEQ ID NO: 54 - protein, 1244 aa, synthetic construct
MFVFLVLLPLVSSQCVNLRTRTQLPPAYTNSFTRGVYYPDKVFRSSVLHSTQDLFLPFFSNVTWFHAIHVSGTNGTKRFDNPVLPFNDGVYFASTEKSNIIRGWIFGTTLDSKTQSLLIVNNATNVVIKVCEFQFCNDPFLDVYYHKNNKSWMESGVYSSANNCTFEYVSQPFLMDLEGKQGNFKNLREFVFKNIDGYFKIYSKHTPINLVRDLPQGFSALEPLVDLPIGINITRFQTLLALHRSYLTPGDSSSGWTAGAAAYYVGYLQPRTFLLKYNENGTITDAVDCALDPLSETKCTLKSFTVEKGIYQTSNFRVQPTESIVRFPNITNLCPFGEVFNATRFASVYAWNRKRISNCVADYSVLYNSASFSTFKCYGVSPTKLNDLCFTNVYADSFVIRGDEVRQIAPGQTGKIADYNYKLPDDFTGCVIAWNSNNLDSKVGGNYNYRYRLFRKSNLKPFERDISTEIYQAGSKPCNGVEGFNCYFPLQSYGFQPTNGVGYQPYRVVVLSFELLHAPATVCGPKKSTNLVKNKCVNFNFNGLTGTGVLTESNKKFLPFQQFGRDIADTTDAVRDPQTLEILDITPCSFGGVSVITPGTNTSNQVAVLYQGVNCTEVPVAIHADQLTPTWRVYSTGSNVFQTRAGCLIGAEHVNNSYECDIPIGAGICASYQTQTNSRGSASSVASQSIIAYTMSLGAENSVAYSNNSIAIPTNFTISVTTEILPVSMTKTSVDCTMYICGDSTECSNLLLQYGSFCTQLNRALTGIAVEQDKNTQEVFAQVKQIYKTPPIKDFGGFNFSQILPDPSKPSKRSPIEDLLFNKVTLADAGFIKQYGDCLGDIAARDLICAQKFNGLTVLPPLLTDEMIAQYTSALLAGTITSGWTFGAGPALQIPFPMQMAYRFNGIGVTQNVLYENQKLIANQFNSAIGKIQDSLSSTPSALGKLQNVVNQNAQALNTLVKQLSSNFGAISSVLNDILSRLDPPEAEVQIDRLITGRLQSLQTYVTQQLIRAAEIRASANLAATKMSECVLGQSKRVDFCGKGYHLMSFPQSAPHGVVFLHVTYVPAQEKQFTTAPAICHDGKAHFPREGVFVSTGTHWFVTQRNFYEPQIITTDNTFVSGNCDVVIGIVNNTVYDPLQPELDSFKEELDKYFKNHTSPDVDLGDISGINASVVNIQKEIDRLNEVAKNLNESLIDLQELGKYEQYIKWPGYIPEAPRDGQAYVRKDGEWVLLSTFLHHHHHH

SEQ ID NO: 55 - protein, 1244 aa, synthetic construct
MFVFLVLLPLVSSQCVNLRTRTQLPPAYTNSFTRGVYYPDKVFRSSVLHSTQDLFLPFFSNVTWFHAIHVSGTNGTKRFDNPVLPFNDGVYFASTEKSNIIRGWIFGTTLDSKTQSLLIVNNATNVVIKVCEFQFCNDPFLDVYYHKNNKSWMESGVYSSANNCTFEYVSQPFLMDLEGKQGNFKNLREFVFKNIDGYFKIYSKHTPINLVRDLPQGFSALEPLVDLPIGINITRFQTLLALHRSYLTPGDSSSGWTAGAAAYYVGYLQPRTFLLKYNENGTITDAVDCALDPLSETKCTLKSFTVEKGIYQTSNFRVQPTESIVRFPNITNLCPFGEVFNATRFASVYAWNRKRISNCVADYSVLYNSASFSTFKCYGVSPTKLNDLCFTNVYADSFVIRGDEVRQIAPGQTGKIADYNYKLPDDFTGCVIAWNSNNLDSKVGGNYNYRYRLFRKSNLKPFERDISTEIYQAGSKPCNGVEGFNCYFPLQSYGFQPTNGVGYQPYRVVVLSFELLHAPATVCGPKKSTNLVKNKCVNFNFNGLTGTGVLTESNKKFLPFQQFGRDIADTTDAVRDPQTLEILDITPCSFGGVSVITPGTNTSNQVAVLYQGVNCTEVPVAIHADQLTPTWRVYSTGSNVFQTRAGCLIGAEHVNNSYECDIPIGAGICASYQTQTNSRGSASSVASQSIIAYTMSLGAENSVAYSNNSIAIPTNFTISVTTEILPVSMTKTSVDCTMYICGDSTECSNLLLQYGSFCTQLNRALTGIAVEQDKNTQEVFAQVKQIYKTPPIKDFGGFNFSQILPDPSKPSKRSPIEDLLFNKVTLADAGFIKQYGDCLGDIAARDLICAQKFNGLTVLPPLLTDEMIAQYTSALLAGTITSGWTFGAGPALQIPFPMQMAYRFNGIGVTQNVLYENQKLIANQFNSAIGKIQDSLSSTPSALGKLQNVVNQNAQALNTLVKCLSSNFGAISSVLNDILSRLDPPEAEVQIDRLITGRLQCLQTYVTQQLIRAAEIRASANLAATKMSECVLGQSKRVDFCGKGYHLMSFPQSAPHGVVFLHVTYVPAQEKNFTTAPAICHDGKAHFPREGVFVSNGTHWFVTQRNFYEPQIITTDNTFVSGNCDVVIGIVNNTVYDPLQPELDSFKEELDKYFKNHTSPDVDLGDISGINASVVNIQKEIDRLNEVAKNLNESLIDLQELGKYEQYIKWPGYIPEAPRDGQAYVRKDGEWVLLSTFLHHHHHH

SEQ ID NO: 56 - protein, 1244 aa, synthetic construct
MFVFLVLLPLVSSQCVNLRTRTQLPPAYTNSFTRGVYYPDKVFRSSVLHSTQDLFLPFFSNVTWFHAIHVSGTNGTKRFDNPVLPFNDGVYFASTEKSNIIRGWIFGTTLDSKTQSLLIVNNATNVVIKVCEFQFCNDPFLDVYYHKNNKSWMESGVYSSANNCTFEYVSQPFLMDLEGKQGNFKNLREFVFKNIDGYFKIYSKHTPINLVRDLPQGFSALEPLVDLPIGINITRFQTLLALHRSYLTPGDSSSGWTAGAAAYYVGYLQPRTFLLKYNENGTITDAVDCALDPLSETKCTLKSFTVEKGIYQTSNFRVQPTESIVRFPNITNLCPFGEVFNATRFASVYAWNRKRISNCVADYSVLYNSASFSTFKCYGVSPTKLNDLCFTNVYADSFVIRGDEVRQIAPGQTGKIADYNYKLPDDFTGCVIAWNSNNLDSKVGGNYNYRYRLFRKSNLKPFERDISTEIYQAGSKPCNGVEGFNCYFPLQSYGFQPTNGVGYQPYRVVVLSFELLHAPATVCGPKKSTNLVKNKCVNFNFNGLTGTGVLTESNKKFLPFQQFGRDIADTTDAVRDPQTLEILDITPCSFGGVSVITPGTNTSNQVAVLYQGVNCTEVPVAIHADQLTPTWRVYSTGSNVFQTRAGCLIGAEHVNNSYECDIPIGAGICASYQTQTNSRGSASSVASQSIIAYTMSLGAENSVAYSNNSIAIPTNFTISVTTEILPVSMTKTSVDCTMYICGDSTECSNLLLQYGSFCTQLNRALTGIAVEQDKNTQEVFAQVKQIYKTPPIPDFGGFNFSQILPDPSKPSKRSPIEDLLFNKVTLADAGFIKQYGDCLGDIAARDLICAQKFNGLTVLPPLLTDEMIAQYTSALLAGTITSGWTFGAGPALQIPFPMQMAYRFNGIGVTQNVLYENQKLIANQFNSAIGKIQDSLSSTPSALGKLQNVVNQNAQALNTLVKQLSSNFGAISSVLNDILSRLDPPEAEVQIDRLITGRLQSLQTYVTQQLIRAAEIRASANLAATKMSECVLGQSKRVDFCGKGYHLMSFPQSAPHGVVFLHVTYVPAQEKNFTTAPAICHDGKAHFPREGVFVSNGTHWFVTQRNFYEPQIITTDNTFVSGNCDVVIGIVNNTVYDPLQPELDSFKEELDKYFKNHTSPDVDLGDISGINASVVNIQKEIDRLNEVAKNLNESLIDLQELGKYEQYIKWPGYIPEAPRDGQAYVRKDGEWVLLSTFLHHHHHH

SEQ ID NO: 57 - protein, 1244 aa, synthetic construct
MFVFLVLLPLVSSQCVNLRTRTQLPPAYTNSFTRGVYYPDKVFRSSVLHSTQDLFLPFFSNVTWFHAIHVSGTNGTKRFDNPVLPFNDGVYFASTEKSNIIRGWIFGTTLDSKTQSLLIVNNATNVVIKVCEFQFCNDPFLDVYYHKNNKSWMESGVYSSANNCTFEYVSQPFLMDLEGKQGNFKNLREFVFKNIDGYFKIYSKHTPINLVRDLPQGFSALEPLVDLPIGINITRFQTLLALHRSYLTPGDSSSGWTAGAAAYYVGYLQPRTFLLKYNENGTITDAVDCALDPLSETKCTLKSFTVPKGIYQTSNFRVQPTESIVRFPNITNLCPFGEVFNATRFASVYAWNRKRISNCVADYSVLYNSASFSTFKCYGVSPTKLNDLCFTNVYADSFVIRGDEVRQIAPGQTGKIADYNYKLPDDFTGCVIAWNSNNLDSKVGGNYNYRYRLFRKSNLKPFERDISTEIYQAGSKPCNGVEGFNCYFPLQSYGFQPTNGVGYQPYRVVVLSFELLHAPATVCGPKKSTNLVKNKCVNFNFNGLTGTGVLTESNKKFLPFQQFGRDIADTTDAVRDPQTLEILDITPCSFGGVSVITPGTNTSNQVAVLYQGVNCTEVPVAIHADQLTPTWRVYSTGSNVFQTRAGCLIGAEHVNNSYECDIPIGAGICASYQTQTNSRGSASSVASQSIIAYTMSLGAENSVAYSNNSIAIPTNFTISVTTEILPVSMTKTSVDCTMYICGDSTECSNLLLQYGSFCTQLNRALTGIAVEQDKNTQEVFAQVKQIYKTPPIKDFGGFNFSQILPDPSKPSKRSPIEDLLFNKVTLADAGFIKQYGDCLGDIAARDLICAQKFNGLTVLPPLLTDEMIAQYTSALLAGTITSGWTFGAGPALQIPFPMQMAYRFNGIGVTQNVLYENQKLIANQFNSAIGKIQDSLSSTPSALGKLQNVVNQNAQALNTLVKQLSSNFGAISSVLNDILSRLDPPEAEVQIDRLITGRLQSLQTYVTQQLIRAAEIRASANLAATKMSECVLGQSKRVDFCGKGYHLMSFPQSAPHGVVFLHVTYVPAQEKNFTTAPAICHDGKAHFPREGVFVSNGTHWFVTQRNFYEPQIITTDNTFVSGNCDVVIGIVNNTVYDPLQPELDSFKEELDKYFKNHTSPDVDLGDISGINASVVNIQKEIDRLNEVAKNLNESLIDLQELGKYEQYIKWPGYIPEAPRDGQAYVRKDGEWVLLSTFLHHHHHH

SEQ ID NO: 58 - protein, 247 aa, synthetic construct; identical to SEQ ID NO: 41

SEQ ID NO: 59 - RNA, 4063 nt, synthetic construct
  source 1..4063: mol_type = other RNA
  modified_base 1..4063: mod_base = OTHER; note = Every A,C G and T = AMP, CMP, GMP and N1-psi-UMP, respectively
  misc_feature 1: note = 7MeGpppG2'OMe at 5' end
gggaaataagagagaaaagaagagtaagaagaaatataagaccccggcgccgccaccatgttcgtgttcctggtgctgctgcccctggtgagcagccagtgcgtgaatctgatcaccagaacccagagctataccaatagcttcaccaggggcgtgtactaccccgataaggtgttcaggtccagcgtgctgcacagcacccaggacctgttcctgccattcttcagcaatgtgacctggtttcacgccatccacgtgagcggcaccaacggcaccaagcggttcgacaaccctgccctgccattcaatgacggcgtgtacttcgcctccaccgagaagtccaacatcatcaggggctggatcttcggcaccaccctggacagcaagacccagtctctgctgatcgtgaataacgccaccaacgtggtgatcaaggtgtgcgagttccagttctgcaacgatccattcctggacgtgtaccagaagaacaacaagtcctggatggagtctgagttcagagtgtacagctctgccaacaactgtacctttgagtacgtgagccagcctttcctgatggacctggagggcaaggagggcaacttcaagaatctgagggagttcgtgttcaagaacatcgacggctacttcaagatctacagcaagcacacccccatcaatctggagcgcgacctgcctcagggcttcagcgccctggagcctctggtggacctgcccatcggcatcaacatcaccaggttccagaccctgctggccctgcacaggagctacctgacccccgtggatagcagcagcggctggaccgccggcgccgccgcctactacgtggggtacctgcagcccaggaccttcctgctgaagtacaacgagaacggcaccatcaccgacgccgtggactgcgccctggatccactgtctgagaccaagtgcaccctgaagtccttcaccgtggagaagggcatctaccagacctccaacttcagggtgcagcctaccgagagcatcgtgcggtttccccagatcaccaatctgtgtccttttggcgaggtgttcaacgccaccaagttccccagcgtgtacgcctgggagcggaagaagatcagcaactgcgtggccgactacagcgtgctgtacaattccaccttcttcagcaccttcaagtgctacggcgtgagcgccaccaagctgaacgatctgtgcttcagcaacgtgtacgccgacagcttcgtggtgaagggcgacgacgtgcggcagatcgcccccggccagaccggcgtgatcgccgactacaactacaagctgcctgacgacttcatgggctgcgtgatcgcctggaactccaacaacctggattccaaggtgggcggcaactataattacaggtacaggctgttcagaaagagcaacctgaagcctttcgagagagacatctctaccgagatctatcaggccggctccaagccctgcaatggcgtggagggcttcaactgctacttccccctgcagagctacggcttccagcctaccaacggcgtgggctaccagccctacagggtggtggtgctgtccttcgagctgctgcacgcccctgccaccgtgtgcggccctaagaagtccaccaacctggtgaagaacaagtgcgtgaacttcaacttcaacggcctgaccggcaccggggtgctgaccgagagcaacaagaagtttctgcctttccagcagttcggcagggacatcgccgacaccaccgatgccgtgcgggatccacagaccctggagatcctggacatcaccccctgcagcttcggcggcgtgtctgtgatcacccctggcaccaacacctccaaccaggtggccgtgctgtaccagggcgtgaattgcaccgaggtgcctgtggccatccacgccgaccagctgacccccacctggcgggtgtacagcaccggctctaacgtgttccagaccagggccggctgcctgatcggcgccgagcacgtgaacaacagctacgagtgcgacatccctatcggggccggcatctgcgcctcttaccagacccagaccaacagcaggggctccgcctccagcgtggccagccagtccatcatcgcctacaccatgagcctgggcgccgagaactccgtggcctacagcaacaacagcatcgccatccccaccaacttcaccatcagcgtgaccaccgagatcctgcccgtgagcatgcccaagacctctgtggactgtaccatgtacatctgcggcgactccaccgagtgcagcaacctgctgctgcagtacggcagcttctgcacccagctgaatagggccctgaccggcatcgccgtggagcaggacaagaacacccaggaggtgtttgcccaggtgaagcagatctacaagacccctcctatccctgacttcggcggcttcaatttcagccagatcctgcccgaccccagcaagcctagcaagaggtcccccatcgaggacctgctgttcaataaggtgaccctggccgacgccgggttcatcaagcagtacggcgattgcctgggcgacatcgccgccagggacctgatctgcgcccagaagttcaatggcctgaccgtgctgcccccactgctgaccgacgagatgattgcccagtacacctctgccctgctggccggcaccatcaccagcggctggaccttcggggccggcccagccctgcagatccctttccccatgcagatggcctaccggttcaatggcatcggcgtgacccagaacgtgctgtacgagaaccagaagctgatcgccaatcagtttaactccgccatcggcaagatccaggacagcctgagcagcacccctagcgccctgggcaagctgcagaacgtggtgaatcagaacgcccaggccctgaataccctggtgaagtgcctgagctctaatttcggcgccatcagctctgtgctgaacgacatcctgtctcggctggacccccccgaggccgaggtgcagatcgacaggctgatcaccggccggctgcagtgcctgcagacctacgtgacccagcagctgatcagagccgccgagattagagccagcgccaatctggccgccaccaagatgagcgagtgtgtgctgggccagagcaagagggtggacttctgcggcaagggataccacctgatgagcttcccccagagcgcccctcacggcgtggtgttcctgcacgtgacctacgtgcccgcccaggagaagaatttcaccaccgccccagccatctgccacgacggcaaggcccactttcctcgggagggcgtgttcgtgagcaacggcacccactggttcgtgacccagagaaacttctacgagccccagatcatcaccaccgacaacaccttcgtgagcggcaactgcgacgtggtgatcgggatcgtgaataataccgtgtacgatcccctgcagcccgagctggacagcttcaaggaggagctggacaagtacttcaagaaccacacctcccccgatgtggatctgggcgacatttccggcatcctggcctctgtggtgaacatccagaaggagatcgacaggctgaacgaggtggccaagaacctgaacgagtctctgatcgacctgcaggagctgggcaagtacgagcagtacatcaagtggccttggtacatctggctgggcttcatcgccggcctgatcgccatcgtgatggtgaccatcatgctgtgctgcatgacctcctgctgcagctgtctgaagggctgttgcagctgcggcagctgctgcaagttcgacgaggacgacagcgagcccgtgctgaagggcgtgaagctgcattatacatgataataggctggagcctcggtggcctagcttcttgccccttgggcctccccccagcccctcctccccttcctgcacccgtacccccgtggtctttgaataaagtctgagtgggcggcaaaaaaaaaaaaaaaaaaaaaaaaaaaaaaaaaaaaaaaaaaaaaaaaaaaaaaaaaaaaaaaaaaaaaaaaaaaaaaaa

SEQ ID NO: 60 - DNA, 31 bp, synthetic construct
  source 1..31: mol_type = other DNA
gcataagctttaatacgactcactataggga

SEQ ID NO: 61 - DNA, 129 bp, synthetic construct
  source 1..129: mol_type = other DNA
ttttttttttttttttttttttttttttttttttttttttttttttttttttttttttttttttttttttttttttttttttttttttttttttttttttgctagcgccgcccactcagactttattca

SEQ ID NO: 62 - protein, 1269 aa, synthetic construct
MFVFLVLLPLVSSQCVNLITRTQSYTNSFTRGVYYPDKVFRSSVLHSTQDLFLPFFSNVTWFHAIHVSGTNGTKRFDNPALPFNDGVYFASTEKSNIIRGWIFGTTLDSKTQSLLIVNNATNVVIKVCEFQFCNDPFLDVYQKNNKSWMESEFRVYSSANNCTFEYVSQPFLMDLEGKEGNFKNLREFVFKNIDGYFKIYSKHTPINLERDLPQGFSALEPLVDLPIGINITRFQTLLALHRSYLTPVDSSSGWTAGAAAYYVGYLQPRTFLLKYNENGTITDAVDCALDPLSETKCTLKSFTVEKGIYQTSNFRVQPTESIVRFPQITNLCPFGEVFNATKFPSVYAWERKKISNCVADYSVLYNSTFFSTFKCYGVSATKLNDLCFSNVYADSFVVKGDDVRQIAPGQTGVIADYNYKLPDDFMGCVIAWNSNNLDSKVGGNYNYRYRLFRKSNLKPFERDISTEIYQAGSKPCNGVEGFNCYFPLQSYGFQPTNGVGYQPYRVVVLSFELLHAPATVCGPKKSTNLVKNKCVNFNFNGLTGTGVLTESNKKFLPFQQFGRDIADTTDAVRDPQTLEILDITPCSFGGVSVITPGTNTSNQVAVLYQGVNCTEVPVAIHADQLTPTWRVYSTGSNVFQTRAGCLIGAEHVNNSYECDIPIGAGICASYQTQTNSRGSASSVASQSIIAYTMSLGAENSVAYSNNSIAIPTNFTISVTTEILPVSMPKTSVDCTMYICGDSTECSNLLLQYGSFCTQLNRALTGIAVEQDKNTQEVFAQVKQIYKTPPIPDFGGFNFSQILPDPSKPSKRSPIEDLLFNKVTLADAGFIKQYGDCLGDIAARDLICAQKFNGLTVLPPLLTDEMIAQYTSALLAGTITSGWTFGAGPALQIPFPMQMAYRFNGIGVTQNVLYENQKLIANQFNSAIGKIQDSLSSTPSALGKLQNVVNQNAQALNTLVKCLSSNFGAISSVLNDILSRLDPPEAEVQIDRLITGRLQCLQTYVTQQLIRAAEIRASANLAATKMSECVLGQSKRVDFCGKGYHLMSFPQSAPHGVVFLHVTYVPAQEKNFTTAPAICHDGKAHFPREGVFVSNGTHWFVTQRNFYEPQIITTDNTFVSGNCDVVIGIVNNTVYDPLQPELDSFKEELDKYFKNHTSPDVDLGDISGILASVVNIQKEIDRLNEVAKNLNESLIDLQELGKYEQYIKWPWYIWLGFIAGLIAIVMVTIMLCCMTSCCSCLKGCCSCGSCCKFDEDDSEPVLKGVKLHYT

SEQ ID NO: 63 - protein, 1261 aa, synthetic construct
QCVNLITRTQSYTNSFTRGVYYPDKVFRSSVLHSTQDLFLPFFSNVTWFHAISGTNGTKRFDNPVLPFNDGVYFASTEKSNIIRGWIFGTTLDSKTQSLLIVNNATNVVIKVCEFQFCNDPFLDVYYHKNNKSWMESEFRVYSSANNCTFEYVSQPFLMDLEGKQGNFKNLREFVFKNIDGYFKIYSKHTPINLGRDLPQGFSALEPLVDLPIGINITRFQTLLALHRSYLTPGDSSSGWTAGAAAYYVGYLQPRTFLLKYNENGTITDAVDCALDPLSETKCTLKSFTVEKGIYQTSNFRVQPTESIVRFPNITNLCPFDEVFNATRFASVYAWNRKRISNCVADYSVLYNFAPFFAFKCYGVSPTKLNDLCFTNVYADSFVIRGNEVSQIAPGQTGNIADYNYKLPDDFTGCVIAWNSNKLDSKVGGNYNYRYRLFRKSNLKPFERDISTEIYQAGNKPCNGVAGVNCYFPLQSYGFRPTYGVGHQPYRVVVLSFELLHAPATVCGPKKSTNLVKNKCVNFNFNGLTGTGVLTESNKKFLPFQQFGRDIADTTDAVRDPQTLEILDITPCSFGGVSVITPGTNTSNQVAVLYQGVNCTEVPVAIHADQLTPTWRVYSTGSNVFQTRAGCLIGAEYVNNSYECDIPIGAGICASYQTQTKSHGSASSVASQSIIAYTMSLGAENSVAYSNNSIAIPTNFTISVTTEILPVSMTKTSVDCTMYICGDSTECSNLLLQYGSFCTQLKRALTGIAVEQDKNTQEVFAQVKQIYKTPPIKYFGGFNFSQILPDPSKPSKRSFIEDLLFNKVTLADAGFIKQYGDCLGDIAARDLICAQKFNGLTVLPPLLTDEMIAQYTSALLAGTITSGWTFGAGAALQIPFAMQMAYRFNGIGVTQNVLYENQKLIANQFNSAIGKIQDSLSSTASALGKLQDVVNHNAQALNTLVKQLSSKFGAISSVLNDILSRLDPPEAEVQIDRLITGRLQSLQTYVTQQLIRAAEIRASANLAATKMSECVLGQSKRVDFCGKGYHLMSFPQSAPHGVVFLHVTYVPAQEKNFTTAPAICHDGKAHFPREGVFVSNGTHWFVTQRNFYEPQIITTDNTFVSGNCDVVIGIVNNTVYDPLQPELDSFKEELDKYFKNHTSPDVDLGDISGINASVVNIQKEIDRLNEVAKNLNESLIDLQELGKYEQYIKWPWYIWLGFIAGLIAIVMVTIMLCCMTSCCSCLKGCCSCGSCCKFDEDDSEPVLKGVKLHYTHHHHHH

SEQ ID NO: 64 - protein, 1264 aa, synthetic construct
VNLTTRTQLPPAYTNSFTRGVYYPDKVFRSSVLHSTQDLFLPFFSNVTWFHAIHVSGTNGTKRFDNPVLPFNDGVYFASTEKSNIIRGWIFGTTLDSKTQSLLIVNNATNVVIKVCEFQFCNDPFLGVYYHKNNKSWMESEFRVYSSANNCTFEYVSQPFLMDLEGKQGNFKNLREFVFKNIDGYFKIYSKHTPINLVRDLPQGFSALEPLVDLPIGINITRFQTLLALHRSYLTPGDSSSGWTAGAAAYYVGYLQPRTFLLKYNENGTITDAVDCALDPLSETKCTLKSFTVEKGIYQTSNFRVQPTESIVRFPNITNLCPFGEVFNATRFASVYAWNRKRISNCVADYSVLYNSASFSTFKCYGVSPTKLNDLCFTNVYADSFVIRGDEVRQIAPGQTGKIADYNYKLPDDFTGCVIAWNSNNLDSKVGGNYNYLYRLFRKSNLKPFERDISTEIYQAGSTPCNGVEGFNCYFPLQSYGFQPTNGVGYQPYRVVVLSFELLHAPATVCGPKKSTNLVKNKCVNFNFNGLTGTGVLTESNKKFLPFQQFGRDIADTTDAVRDPQTLEILDITPCSFGGVSVITPGTNTSNQVAVLYQDVNCTEVPVAIHADQLTPTWRVYSTGSNVFQTRAGCLIGAEHVNNSYECDIPIGAGICASYQTQTNSPGSASSVASQSIIAYTMSLGAENSVAYSNNSIAIPTNFTISVTTEILPVSMTKTSVDCTMYICGDSTECSNLLLQYGSFCTQLNRALTGIAVEQDKNTQEVFAQVKQIYKTPPIKDFGGFNFSQILPDPSKPSKRSFIEDLLFNKVTLADAGFIKQYGDCLGDIAARDLICAQKFNGLTVLPPLLTDEMIAQYTSALLAGTITSGWTFGAGAALQIPFAMQMAYRFNGIGVTQNVLYENQKLIANQFNSAIGKIQDSLSSTASALGKLQDVVNQNAQALNTLVKQLSSNFGAISSVLNDILSRLDPPEAEVQIDRLITGRLQSLQTYVTQQLIRAAEIRASANLAATKMSECVLGQSKRVDFCGKGYHLMSFPQSAPHGVVFLHVTYVPAQEKNFTTAPAICHDGKAHFPREGVFVSNGTHWFVTQRNFYEPQIITTDNTFVSGNCDVVIGIVNNTVYDPLQPELDSFKEELDKYFKNHTSPDVDLGDISGINASVVNIQKEIDRLNEVAKNLNESLIDLQELGKYEQYIKWPWYIWLGFIAGLIAIVMVTIMLCCMTSCCSCLKGCCSCGSCCKFDEDDSEPVLKGVKLHYTHHHHHH

SEQ ID NO: 65 - protein, 1242 aa, synthetic construct
MFVFLVLLPLVSSQCVNLITRTQSYTNSFTRGVYYPDKVFRSSVLHSTQDLFLPFFSNVTWFHAIHVSGTNGTKRFDNPALPFNDGVYFASTEKSNIIRGWIFGTTLDSKTQSLLIVNNATNVVIKVCEFQFCNDPFLDVYQKNNKSWMESEFRVYSSANNCTFEYVSQPFLMDLEGKEGNFKNLREFVFKNIDGYFKIYSKHTPINLERDLPQGFSALEPLVDLPIGINITRFQTLLALHRSYLTPVDSSSGWTAGAAAYYVGYLQPRTFLLKYNENGTITDAVDCALDPLSETKCTLKSFTVEKGIYQTSNFRVQPTESIVRFPQITNLCPFGEVFNATKFPSVYAWERKKISNCVADYSVLYNSTFFSTFKCYGVTATKLNDLCFSNVYADSFVVKGDDVRQIAPGQTGVIADYNYKLPDDFMGCVIAWNSNNLDSKVGGNYNYRYRLFRKSKLKPFERDISTEIYQAGSKPCNGVEGFNCYFPLQSYGFQPTYGVGYQPYRVVVLSFELLHAPATVCGPKKSTNLVKNKCVNFNFNGLTGTGVLTESNKKFLPFQQFGRDIADTTDAVRDPQTLEILDITPCSFGGVSVITPGTNTSNQVAVLYQGVNCTEVPVAIHADQLTPTWRVYSTGSNVFQTRAGCLIGAEHVNNSYECDIPIGAGICASYQTQTNSRGSASSVASQSIIAYTMSLGAENSVAYSNNSIAIPTNFTISVTTEILPVSMPKTSVDCTMYICGDSTECSNLLLQYGSFCTQLNRALTGIAVEQDKNTQEVFAQVKQIYKTPPIPDFGGFNFSQILPDPSKPSKRSPIEDLLFNKVTLADAGFIKQYGDCLGDIAARDLICAQKFNGLTVLPPLLTDEMIAQYTSALLAGTITSGWTFGAGPALQIPFPMQMAYRFNGIGVTQNVLYENQKLIANQFNSAIGKIQDSLSSTPSALGKLQNVVNQNAQALNTLVKCLSSNFGAISSVLNDILSRLDPPEAEVQIDRLITGRLQCLQTYVTQQLIRAAEIRASANLAATKMSECVLGQSKRVDFCGKGYHLMSFPQSAPHGVVFLHVTYVPAQEKNFTTAPAICHDGKAHFPREGVFVSNGTHWFVTQRNFYEPQIITTDNTFVSGNCDVVIGIVNNTVYDPLQPELDSFKEELDKYFKNHTSPDVDLGDISGILASVVNIQKEIDRLNEVAKNLNESLIDLQELGKYEQYIKWPGYIPEAPRDGQAYVRKDGEWVLLSTFLHHHHHH

SEQ ID NO: 66 - protein, 1242 aa, synthetic construct
MFVFLVLLPLVSSQCVNLITRTQSYTNSFTRGVYYPDKVFRSSVLHSTQDLFLPFFSNVTWFHAIHVSGTNGTKRFDNPALPFNDGVYFASTEKSNIIRGWIFGTTLDSKTQSLLIVNNATNVVIKVCEFQFCNDPFLDVYQKNNKSWMESEFRVYSSANNCTFEYVSQPFLMDLEGKEGNFKNLREFVFKNIDGYFKIYSKHTPINLNRTLPQGFSALEPLVDLPIGINITRFQTLLALHRSYLTPVDNSTGWTAGAANYTVGYLQPRTFLLKYNENGTITDAVDCALDPLSETKCTLKSFTVEKGIYQTSNFRVQPTESIVRFPQITNLCPFGEVFNATKFPSVYAWERKKISNCVADYSVLYNSTFFSTFKCYGVSATKLNDLCFSNVYADSFVVKGDDVRQIAPGQTGVIADYNYKLPDDFMGCVIAWNSNNLDSKVGGNYNYRYRLFRKSKLKPFERDISTEIYQAGSKPCNGVEGFNCYFPLQSYGFQPTYGVGYQPYRVVVLSFELLHAPATVCGPKKSTNLVKNKCVNFNFNGLTGTGVLTESNKKFLPFQQFGRDIADTTDAVRDPQTLEILDITPCSFGGVSVITPGTNTSNQVAVLYQGVNCTEVPVAIHADQLTPTWRVYSTGSNVFQTRAGCLIGAEHVNNSYECDIPIGAGICASYQTQTNSRGSASSVASQSIIAYTMSLGAENSVAYSNNSIAIPTNFTISVTTEILPVSMPKTSVDCTMYICGDSTECSNLLLQYGSFCTQLNRALTGIAVEQDKNTQEVFAQVKQIYKTPPIPDFGGFNFSQILPDPSKPSKRSPIEDLLFNKVTLADAGFIKQYGDCLGDIAARDLICAQKFNGLTVLPPLLTDEMIAQYTSALLAGTITSGWTFGAGPALQIPFPMQMAYRFNGIGVTQNVLYENQKLIANQFNSAIGKIQDSLSSTPSALGKLQNVVNQNAQALNTLVKCLSSNFGAISSVLNDILSRLDPPEAEVQIDRLITGRLQCLQTYVTQQLIRAAEIRASANLAATKMSECVLGQSKRVDFCGKGYHLMSFPQSAPHGVVFLHVTYVPAQEKNFTTAPAICHDGKAHFPREGVFVSNGTHWFVTQRNFYEPQIITTDNTFVSGNCDVVIGIVNNTVYDPLQPELDSFKEELDKYFKNHTSPDVDLGDISGILASVVNIQKEIDRLNEVAKNLNESLIDLQELGKYEQYIKWPGYIPEAPRDGQAYVRKDGEWVLLSTFLHHHHHH

SEQ ID NO: 67 - protein, 1242 aa, synthetic construct
MFVFLVLLPLVSSQCVNLITRTQSYTNSFTRGVYYPDKVFRSSVLHSTQDLFLPFFSNVTWFHAIHVSGTAGTKRFDNPALPFNDGVYFASTEKSNIIRGWIFGTTLDSKTQSLLIVNNATNVVIKVCEFQFCNDPFLDVYQKNNKSWMESEFRVYSSANNCTFEYVSQPFLMDLEGKEGNFKNLREFVFKNIDGYFKIYSKHTPINLERDLPQGFSALEPLVDLPIGINITRFQTLLALHRSYLTPVDSSSGWTAGAAAYYVGYLQPRTFLLKYNENGTITDAVDCALDPLSETKCTLKSFTVEKGIYQTSNFRVQPTESIVRFPQITNLCPFGEVFNATKFPSVYAWERKKISNCVADYSVLYNSTFFSTFKCYGVSATKLNDLCFSNVYADSFVVKGDDVRQIAPGQTGVIADYNYKLPDDFMGCVIAWNSNNLDSKVGGNYNYRYRLFRKSKLKPFERDISTEIYQAGSKPCNGVEGFNCYFPLQSYGFQPTYGVGYQPYRVVVLSFELLHAPATVCGPKKSTNLVKNKCVNFNFNGLTGTGVLTESNKKFLPFQQFGRDIADTTDAVRDPQTLEILDITPCSFGGVSVITPGTNTSNQVAVLYQGVNCTEVPVAIHADQLTPTWRVYSTGSNVFQTRAGCLIGAEHVNNSYECDIPIGAGICASYQTQTNSRGSASSVASQSIIAYTMSLGAENSVAYSNNSIAIPTNFTISVTTEILPVSMPKTSVDCTMYICGDSTECSNLLLQYGSFCTQLNRALTGIAVEQDKNTQEVFAQVKQIYKTPPIPDFGGFNFSQILPDPSKPSKRSPIEDLLFNKVTLADAGFIKQYGDCLGDIAARDLICAQKFNGLTVLPPLLTDEMIAQYTSALLAGTITSGWTFGAGPALQIPFPMQMAYRFNGIGVTQNVLYENQKLIANQFNSAIGKIQDSLSSTPSALGKLQNVVNQNAQALNTLVKCLSSNFGAISSVLNDILSRLDPPEAEVQIDRLITGRLQCLQTYVTQQLIRAAEIRASANLAATKMSECVLGQSKRVDFCGKGYHLMSFPQSAPHGVVFLHVTYVPAQEKNFTTAPAICHDGKAHFPREGVFVSNGTHWFVTQRNFYEPQIITTDNTFVSGNCDVVIGIVNNTVYDPLQPELDSFKEELDKYFKNHTSPDVDLGDISGILASVVNIQKEIDRLNEVAKNLNESLIDLQELGKYEQYIKWPGYIPEAPRDGQAYVRKDGEWVLLSTFLHHHHHH

SEQ ID NO: 68 - protein, 1242 aa, synthetic construct
MFVFLVLLPLVSSQCVNLITRTQSYTNSFTRGVYYPDKVFRSSVLHSTQDLFLPFFSNVTWFHAIHVSGTNGTKRFDNPALPFNDGVYFASTEKSNIIRGWIFGTTLDSKTQSLLIVNNATNVVIKVCEFQFCNDPFLDVYQKNNKSWMESEFRVYSSANNCTFEYVSQPFLMDLEGKEGNFKNLREFVFKNIDGYFKIYSKHTPINLERDLPQGFSALEPLVDLPIGINITRFQTLLALHRSYLTPVDSSSGWTAGAAAYYVGYLQPRTFLLKYNENGTITDAVDCALDPLSETKCTLKSFTVEKGIYQTSNFRVQPTESIVRFPQITNLCPFGEVFNATKFPSVYAWERKKISNCVADYSVLYNSTFFSTFKCYGVSATKLNDLCFSNVYADSFVVKGDDVRQIAPGQTGVIADYNYKLPDDFMGCVIAWNSNNTDSKVGGNYNYRYRLFRKSKLKPFERDISTEIYQAGSKPCNGVEGFNCYFPLQSYGFQPTYGVGYQPYRVVVLSFELLHAPATVCGPKKSTNLVKNKCVNFNFNGLTGTGVLTESNKKFLPFQQFGRDIADTTDAVRDPQTLEILDITPCSFGGVSVITPGTNTSNQVAVLYQGVNCTEVPVAIHADQLTPTWRVYSTGSNVFQTRAGCLIGAEHVNNSYECDIPIGAGICASYQTQTNSRGSASSVASQSIIAYTMSLGAENSVAYSNNSIAIPTNFTISVTTEILPVSMPKTSVDCTMYICGDSTECSNLLLQYGSFCTQLNRALTGIAVEQDKNTQEVFAQVKQIYKTPPIPDFGGFNFSQILPDPSKPSKRSPIEDLLFNKVTLADAGFIKQYGDCLGDIAARDLICAQKFNGLTVLPPLLTDEMIAQYTSALLAGTITSGWTFGAGPALQIPFPMQMAYRFNGIGVTQNVLYENQKLIANQFNSAIGKIQDSLSSTPSALGKLQNVVNQNAQALNTLVKCLSSNFGAISSVLNDILSRLDPPEAEVQIDRLITGRLQCLQTYVTQQLIRAAEIRASANLAATKMSECVLGQSKRVDFCGKGYHLMSFPQSAPHGVVFLHVTYVPAQEKNFTTAPAICHDGKAHFPREGVFVSNGTHWFVTQRNFYEPQIITTDNTFVSGNCDVVIGIVNNTVYDPLQPELDSFKEELDKYFKNHTSPDVDLGDISGILASVVNIQKEIDRLNEVAKNLNESLIDLQELGKYEQYIKWPGYIPEAPRDGQAYVRKDGEWVLLSTFLHHHHHH

SEQ ID NO: 69 - protein, 1242 aa, synthetic construct
MFVFLVLLPLVSSQCVNLITRTQSYTNSFTRGVYYPDKVFRSSVLHSTQDLFLPFFSNVTWFHAIHVSGTNGTKRFDNPALPFNDGVYFASTEKSNIIRGWIFGTTLDSKTQSLLIVNNATNVVIKVCEFQFCNDPFLDVYQKNNKSWMESEFRVYSSANNCTFEYVSQPFLMDLEGKEGNFKNLREFVFKNIDGYFKIYSKHTPINLERDLPQGFSALEPLVDLPIGINITRFQTLLALHRSYLTPVDSSSGWTAGAAAYYVGYLQPRTFLLKYNENGTITDAVDCALDPLSETKCTLKSFTVEKGIYQTSNFRVQPTESIVRFPQITNLCPFGEVFNATKFPSVYAWERKKISNCVADYSVLYNSTFFSTFKCYGVSATKLNDLCFSNVYADSFVVKGDDVRQIAPGQTGVIADYNYKLPDDFMGCVIAWNSNNLDSKVGGNYNYRYRLFRKSKLKPFERDISTEIYQAGSKPCNGVEGFNCYFPLQSYGFQPTYGVGYQPYRVVVLSFELLHAPATVCGPKKSTNLVKNKCVNFNFNGLTGTGVLTESNKKFLPFQQFGRDIADTTDAVRDPQTLEILDITPCSFGGVSVITPGTNTSNQVAVLYQGVNCTEVPVAIHADQLTPTWRVYSTGSNVFQTRAGCLIGAEHVNNSYECDIPIGAGICASYQTQTNSRGSASSNATQSIIAYTMSLGAENSVAYSNNSIAIPTNFTISVTTEILPVSMPKTSVDCTMYICGDSTECSNLLLQYGSFCTQLNRALTGIAVEQDKNTQEVFAQVKQIYKTPPIPDFGGFNFSQILPDPSKPSNRTPIEDLLFNKVTLADAGFIKQYGDCNGTIAARDLICAQKFNGLTVLPPLLTDEMIAQYTSALLAGTITSGWTFGAGPALQIPFPMQMAYRFNGIGVTQNVLYENQKLIANQFNSAIGKIQDSLSSTPSALGKLQNVVNQNAQALNTLVKCLSSNFGAISSVLNDILSRLDPPEAEVQIDRLITGRLQCLQTYVTQQLIRAAEIRASANLAATKMSECVLGQSKRVDFCGKGYHLMSFPQSAPHGVVFLHVTYVPAQEKNFTTAPAICHDGKAHFPREGVFVSNGTHWFVTQRNFYEPQIITTDNTFVSGNCDVVIGIVNNTVYDPLQPELNSTKEELDKYFKNHTSPDVDLGDISGILASVVNIQKEIDRLNEVAKNLNESLIDLQELGKYEQYIKWPGYIPEAPRDGQAYVRKDGEWVLLSTFLHHHHHH

SEQ ID NO: 70 - protein, 1242 aa, synthetic construct
MFVFLVLLPLVSSQCVNLITRTQSYTNSFTRGVYYPDKVFRSSVLHSTQDLFLPFFSNVTWFHAIHVSGTNGTKRFDNPALPFNDGVYFASTEKSNIIRGWIFGTTLDSKTQSLLIVNNATNVVIKVCEFQFCNDPFLDVYQKNNKSWMESEFRVYSSANNCTFEYVSQPFLMDLEGKNGTFKNLREFVFKNIDGYFKIYSKHTPINLERDLPQGFSALEPLVDLPIGINITRFQTLLALHRSYLTPVDSSSGWTAGAANYTVGYLQPRTFLLKYNENGTITDAVDCALDPLSETKCTLKSFTVEKGIYQTSNFRVQPTESIVRFPQITNLCPFGEVFNATKFPSVYAWERKKISNCVADYSVLYNSTFFSTFKCYGVSATKLNDLCFSNVYADSFVVKGDDVRQIAPGQTGVIADYNYKLPDDFMGCVIAWNSNNLDSKVGGNYNYRYRLFRKSKLKPFERDISTEIYQAGSKPCNGVEGFNCYFPLQSYGFQPTYGVGYQPYRVVVLSFELLHAPATVCGPKKSTNLVKNKCVNFNFNGLTGTGVLTESNKKFLPFQQFGRDIADTTDAVRDPQTLEILDITPCSFGGVSVITPGTNTSNQVAVLYQGVNCTEVPVAIHADQLTPTWRVYSTGSNVFQTRAGCLIGAEHVNNSYECDIPIGAGICASYQTQTNSRGSASSVASQSIIAYTMSLGAENSVAYSNNSIAIPTNFTISVTTEILPVSMPKTSVDCTMYICGDSTECSNLLLQYGSFCTQLNRALTGIAVEQDKNTQEVFAQVKQIYKTPPIPDFGGFNFSQILPDPSKPSKRSPIEDLLFNKVTLADAGFIKQYGDCLGDIAARDLICAQKFNGLTVLPPLLTDEMIAQYTSALLAGTITSGWTFGAGPALQIPFPMQMAYRFNGIGVTQNVLYENQKLIANQFNSAIGKIQDSLSSTPSALGKLQNVVNQNAQALNTLVKCLSSNFGAISSVLNDILSRLDPPEAEVQIDRLITGRLQCLQTYVTQQLIRAAEIRASANLAATKMSECVLGQSKRVDFCGKGYHLMSFPQSAPHGVVFLHVTYVPAQEKNFTTAPAICHDGKAHFPREGVFVSNGTHWFVTQRNFYEPQIITTDNTFVSGNCDVVIGIVNNTVYDPLQPELDSFKEELDKYFKNHTSPDVDLGDISGILASVVNIQKEIDRLNEVAKNLNESLIDLQELGKYEQYIKWPGYIPEAPRDGQAYVRKDGEWVLLSTFLHHHHHH

SEQ ID NO: 71 - protein, 1242 aa, synthetic construct
MFVFLVLLPLVSSQCVNLITRTQSYTNSFTRGVYYPDKVFRSSVLHSTQDLFLPFFSNVTWFHAIHVSGTNGTKRFDNPALPFNDGVYFASTEKSNIIRGWIFGTTLDSKTQSLLIVNNATNVVIKVCEFQFCNDPFLDVYQKNNKSWMESEFRVYSSANNCTFEYVSQPFLMDLEGKEGNFKNLREFVFKNIDGYFKIYSKHTPINLERDLPQGFSALEPLVDLPIGINITRFQTLLALHRSYLTPVDSSSGWTAGAAAYYVGYLQPRTFLLKYNENGTITDAVDCALDPLSETKCTLKSFTVEKGIYQTSNFRVQPTESIVRFPQITNLCPFGEVFNATKFPSVYAWERKKISNCVADYSVLYNSTFFSTFKCYGVSATKLNDLCFSNVYADSFVVKGDDVRQIAPGQTGVIADYNYKLPDDFMGCVIAWNSNKLDSKVGGNYNYLYRLFRKSKLKPFERDISTEIYQAGSKPCNGVAGFNCYFPLQSYGFQPTYGVGYQPYRVVVLSFELLHAPATVCGPKKSTNLVKNKCVNFNFNGLTGTGVLTESNKKFLPFQQFGRDIADTTDAVRDPQTLEILDITPCSFGGVSVITPGTNTSNQVAVLYQGVNCTEVPVAIHADQLTPTWRVYSTGSNVFQTRAGCLIGAEHVNNSYECDIPIGAGICASYQTQTNSRGSASSVASQSIIAYTMSLGAENSVAYSNNSIAIPTNFTISVTTEILPVSMPKTSVDCTMYICGDSTECSNLLLQYGSFCTQLNRALTGIAVEQDKNTQEVFAQVKQIYKTPPIPDFGGFNFSQILPDPSKPSKRSPIEDLLFNKVTLADAGFIKQYGDCLGDIAARDLICAQKFNGLTVLPPLLTDEMIAQYTSALLAGTITSGWTFGAGPALQIPFPMQMAYRFNGIGVTQNVLYENQKLIANQFNSAIGKIQDSLSSTPSALGKLQNVVNQNAQALNTLVKCLSSNFGAISSVLNDILSRLDPPEAEVQIDRLITGRLQCLQTYVTQQLIRAAEIRASANLAATKMSECVLGQSKRVDFCGKGYHLMSFPQSAPHGVVFLHVTYVPAQEKNFTTAPAICHDGKAHFPREGVFVSNGTHWFVTQRNFYEPQIITTDNTFVSGNCDVVIGIVNNTVYDPLQPELDSFKEELDKYFKNHTSPDVDLGDISGILASVVNIQKEIDRLNEVAKNLNESLIDLQELGKYEQYIKWPGYIPEAPRDGQAYVRKDGEWVLLSTFLHHHHHH

SEQ ID NO: 72 - protein, 1242 aa, synthetic construct
MFVFLVLLPLVSSQCVNLINRTQSYTNSFTRGVYYPDKVFRSSVLHSTQDLFLPFFSNVTWFHAIHNSTTNGTKRFDNPALPFNDGVYFASTEKSNIIRGWIFGTTLDSKTQSLLIVNNATNVVIKVCEFQFCNDPFLDVYQKNNKSWMESEFRVYSSANNCTFEYVSQPFLMDLEGKEGNFKNLREFVFKNIDGYFKIYSKHTPINLERDLPQGFSALEPLVDLPIGINITRFQTLLALHRSYLTPVDSSSGWTAGAAAYYVGYLQPRTFLLKYNENGTITDAVDCALDPLSETKCTLKSFTVEKGIYQTSNFRVQPTESIVRFPQITNLCPFGEVFNATKFPSVYAWERKKISNCVADYSVLYNSTFFSTFKCYGVSATKLNDLCFSNVYADSFVVKGDDVRQIAPGQTGVIADYNYKLPDDFMGCVIAWNSNNLDSKVGGNYNYRYRLFRKSKLKPFERDISTEIYQAGSKPCNGVEGFNCYFPLQSYGFQPTYGVGYQPYRVVVLSFELLHAPATVCGPKKSTNLVKNKCVNFNFNGLTGTGVLTESNKKFLPFQQFGRDIADTTDAVRDPQTLEILDITPCSFGGVSVITPGTNTSNQVAVLYQGVNCTEVPVAIHADQLTPTWRVYSTGSNVFQTRAGCLIGAEHVNNSYECDIPIGAGICASYQTQTNSRGSASSVASQSIIAYTMSLGAENSVAYSNNSIAIPTNFTISVTTEILPVSMPKTSVDCTMYICGDSTECSNLLLQYGSFCTQLNRALTGIAVEQDKNTQEVFAQVKQIYKTPPIPDFGGFNFSQILPDPSKPSKRSPIEDLLFNKVTLADAGFIKQYGDCLGDIAARDLICAQKFNGLTVLPPLLTDEMIAQYTSALLAGTITSGWTFGAGPALQIPFPMQMAYRFNGIGVTQNVLYENQKLIANQFNSAIGKIQDSLSSTPSALGKLQNVVNQNAQALNTLVKCLSSNFGAISSVLNDILSRLDPPEAEVQIDRLITGRLQCLQTYVTQQLIRAAEIRASANLAATKMSECVLGQSKRVDFCGKGYHLMSFPQSAPHGVVFLHVTYVPAQEKNFTTAPAICHDGKAHFPREGVFVSNGTHWFVTQRNFYEPQIITTDNTFVSGNCDVVIGIVNNTVYDPLQPELDSFKEELDKYFKNHTSPDVDLGDISGILASVVNIQKEIDRLNEVAKNLNESLIDLQELGKYEQYIKWPGYIPEAPRDGQAYVRKDGEWVLLSTFLHHHHHH

SEQ ID NO: 73 - protein, 1242 aa, synthetic construct
MFVFLVLLPLVSSQCVNLITRTQSYTNSFTRGVYYPDKVFRSSVLHSTQDLFLPFFSNVTWFHAIHVSGTNGTKRFDNPALPFNDGVYFASTEKSNIIRGWIFGTTLDSKTQSLLIVNNATNVVIKVCEFQFCNDPFLDVYQKNNKSWMESEFRVYSSANNCTFEYVSQPFLMDLEGKEGNFKNLREFVFKNIDGYFKIYSKHTPINLERDLPQGFSALEPLVDLPIGINITRFQTLLALHRSYLTPVDSSSGWTAGAAAYYVGYLQPRTFLLKYNENGTITDAVDCALDPLSETKCTLKSFTVEKGIYQTSNFRVQPTESIVRFPQITNLCPFGEVFNATKFPSVYAWERKKISNCVADYSVLYNSTFFSTFKCYGVSATKLNDLCFSNVYADSFVVKGDDVRQIAPGQTGVIADYNYKLPDDFMGCVIAWNSNNLDSKVGGNYNYRYRLFRKSKLKPFERDISTEIYQAGSKPCNGVEGFNCYFPLQSYGFQPTYGVGYQPYRVVVLSFELLHAPATVCGPKKSTNLVKNKCVNFNFNGLTGTGVLTESNKKFLPFQQFGRDIADTTDAVRDPQTLEILDITPCSFGGVSVITPGTNTSNQVAVLYQGVNCTEVPVAIHADQLTPNWTVYSTGSNVFQTRAGCLIGAEHVNNSYECDIPIGAGICASYQTQTNSRGSASSNATQSIIAYTMSLGAENSVAYSNNSIAIPTNFTISVTTEILPVSMPKTSVDCTMYICGDSTECSNLLLQYGSFCTQLNRALTGIAVEQDKNTQEVFAQVKQIYKTPPIPDFGGFNFSQILPDPSKPSNRTPIEDLLFNKVTLADAGFIKQYGDCNGTIAARDLICAQKFNGLTVLPPLLTDEMIAQYTSALLAGTITSGWTFGAGPALQIPFPMQMAYRFNGIGVTQNVLYENQKLIANQFNSAIGKIQDSLSSTPSALGKLQNVVNQNAQALNTLVKCLSSNFGAISSVLNDILSRLDPPEAEVQIDRLITGRLQCLQTYVTQQLIRAAEIRASANLAATKMSECVLGQSKRVDFCGKGYHLMSFPQSAPHGVVFLHVTYVPAQEKNFTTAPAICHDGKAHFPREGVFVSNGTHWFVTQRNFYEPQIITTDNTFVSGNCDVVIGIVNNTVYDPLQPELDSFKEELDKYFKNHTSPDVDLGDISGILASVVNIQKEIDRLNEVAKNLNESLIDLQELGKYEQYIKWPGYIPEAPRDGQAYVRKDGEWVLLSTFLHHHHHH

SEQ ID NO: 74 - protein, 1242 aa, synthetic construct
MFVFLVLLPLVSSQCVNLITRTQSYTNSFTRGVYYPDKVFRSSVLHSTQDLFLPFFSNVTWFHAIHVSGTNGTKRFDNPALPFNDGVYFASTEKSNIIRGWIFGTTLDSKTQSLLIVNNATNVVIKVCEFQFCNDPFLDVYQKNNKSWMESEFRVYSSANNCTFEYVSQPFLMDLEGKEGNFKNLREFVFKNIDGYFKIYSKHTPINLERDLPQGFSALEPLVDLPIGINITRFQTLLALHRSYLTPVDSSSGWTAGAAAYYVGYLQPRTFLLKYNENGTITDAVDCALDPLSETKCTLKSFTVEKGIYQTSNFRVQPTESIVRFPQITNLCPFGEVFNATKFPSVYAWERKKISNCVADYSVLYNSTFFSTFKCYGVSATKLNDLCFSNVYADSFVVKGDDVRQIAPGQTGVIADYNYKLPDDFMGCVIAWNSNNLDSKVGGNYNYRYRLFRKSNLTPFERDISTEIYQAGSKPCNGVEGFNCYFPLQSYGFQPTYGVGYQPYRVVVLSFELLHAPATVCGPKKSTNLVKNKCVNFNFNGLTGTGVLTESNKKFLPFQQFGRDIADTTDAVRDPQTLEILDITPCSFGGVSVITPGTNTSNQVAVLYQGVNCTEVPVAIHADQLTPTWRVYSTGSNVFQTRAGCLIGAEHVNNSYECDIPIGAGICASYQTQTNSRGSASSVASQSIIAYTMSLGAENSVAYSNNSIAIPTNFTISVTTEILPVSMPKTSVDCTMYICGDSTECSNLLLQYGSFCTQLNRALTGIAVEQDKNTQEVFAQVKQIYKTPPIPDFGGFNFSQILPDPSKPSKRSPIEDLLFNKVTLADAGFIKQYGDCLGDIAARDLICAQKFNGLTVLPPLLTDEMIAQYTSALLAGTITSGWTFGAGPALQIPFPMQMAYRFNGIGVTQNVLYENQKLIANQFNSAIGKIQDSLSSTPSALGKLQNVVNQNAQALNTLVKCLSSNFGAISSVLNDILSRLDPPEAEVQIDRLITGRLQCLQTYVTQQLIRAAEIRASANLAATKMSECVLGQSKRVDFCGKGYHLMSFPQSAPHGVVFLHVTYVPAQEKNFTTAPAICHDGKAHFPREGVFVSNGTHWFVTQRNFYEPQIITTDNTFVSGNCDVVIGIVNNTVYDPLQPELDSFKEELDKYFKNHTSPDVDLGDISGILASVVNIQKEIDRLNEVAKNLNESLIDLQELGKYEQYIKWPGYIPEAPRDGQAYVRKDGEWVLLSTFLHHHHHH

SEQ ID NO: 75 - protein, 1242 aa, synthetic construct
MFVFLVLLPLVSSQCVNLITRTQSYTNSFTRGVYYPDKVFRSSVLHSTQDLFLPFFSNVTWFHAIHVSGTNGTKRFDNPALPFNDGVYFASTEKSNIIRGWIFGTTLDSKTQSLLIVNNATNVVIKVCEFQFCNDPFLDVYQKNNKSWMESEFRVYSSANNCTFEYVSQPFLMDLEGKEGNFKNLREFVFKNIDGYFKIYSKHTPINLERDLPQGFSALEPLVDLPIGINITRFQTLLALHRSYLTPVDNSTGWTAGAANYTVGYLQPRTFLLKYNENGTITDAVDCALDPLSETKCTLKSFTVEKGIYQTSNFRVQPTESIVRFPQITNLCPFGEVFNATKFPSVYAWERKKISNCVADYSVLYNSTFFSTFKCYGVSATKLNDLCFSNVYADSFVVKGDDVRQIAPGQTGVIADYNYKLPDDFMGCVIAWNSNNLDSKVGGNYNYRYRLFRKSKLKPFERDISTEIYQAGSKPCNGVEGFNCYFPLQSYGFQPTYGVGYQPYRVVVLSFELLHAPATVCGPKKSTNLVKNKCVNFNFNGLTGTGVLTESNKKFLPFQQFGRDIADTTDAVRDPQTLEILDITPCSFGGVSVITPGTNTSNQVAVLYQGVNCTEVPVAIHADQLTPTWRVYSTGSNVFQTRAGCLIGAEHVNNSYECDIPIGAGICASYQTQTNSRGSASSVASQSIIAYTMSLGAENSVAYSNNSIAIPTNFTISVTTEILPVSMPKTSVDCTMYICGDSTECSNLLLQYGSFCTQLNRALTGIAVEQDKNTQEVFAQVKQIYKTPPIPDFGGFNFSQILPDPSKPSKRSPIEDLLFNKVTLADAGFIKQYGDCLGDIAARDLICAQKFNGLTVLPPLLTDEMIAQYTSALLAGTITSGWTFGAGPALQIPFPMQMAYRFNGIGVTQNVLYENQKLIANQFNSAIGKIQDSLSSTPSALGKLQNVVNQNAQALNTLVKCLSSNFGAISSVLNDILSRLDPPEAEVQIDRLITGRLQCLQTYVTQQLIRAAEIRASANLAATKMSECVLGQSKRVDFCGKGYHLMSFPQSAPHGVVFLHVTYVPAQEKNFTTAPAICHDGKAHFPREGVFVSNGTHWFVTQRNFYEPQIITTDNTFVSGNCDVVIGIVNNTVYDPLQPELDSFKEELDKYFKNHTSPDVDLGDISGILASVVNIQKEIDRLNEVAKNLNESLIDLQELGKYEQYIKWPGYIPEAPRDGQAYVRKDGEWVLLSTFLHHHHHH

SEQ ID NO: 76 - protein, 1242 aa, synthetic construct
MFVFLVLLPLVSSQCVNLITRTQSYTNSFTRGVYYPDKVFRSSVLHSTQDLFLPFFSNVTWFHAIHVSGTNGTKRFDNPALPFNDGVYFASTEKSNIIRGWIFGTTLDSKTQSLLIVNNATNVVIKVCEFQFCNDPFLDVYQKNNKSWMESEFRVYSSANNCTFEYVSQPFLMDLEGKEGNFKNLREFVFKNIDGYFKIYSKHTPINLERDLPQGFSALEPLVDLPIGINITRFQTLLALHRSYLTPVDSSSGWTAGAAAYYVGYLQPRTFLLKYNENGTITDAVDCALDPLSETKCTLKSFTVEKGIYQTSNFRVQPTESIVRFPQITNLCPFGEVFNATKFPSVYAWERKKISNCVADYSVLYNSTFFSTFKCYGVNATKLNDLCFSNVYADSFVVKGDDVRQIAPGQTGVIADYNYKLPDDFMGCVIAWNSNNLDSKVGGNYNYRYRLFRKSKLKPFERDISTEIYQAGSKPCNGVEGFNCYFPLQSYGFQPTYGVGYQPYRVVVLSFELLHAPATVCGPKKSTNLVKNKCVNFNFNGLTGTGVLTESNKKFLPFQQFGRDIADTTDAVRDPQTLEILDITPCSFGGVSVITPGTNTSNQVAVLYQGVNCTEVPVAIHADQLTPTWRVYSTGSNVFQTRAGCLIGAEHVNNSYECDIPIGAGICASYQTQTNSRGSASSVASQSIIAYTMSLGAENSVAYSNNSIAIPTNFTISVTTEILPVSMPKTSVDCTMYICGDSTECSNLLLQYGSFCTQLNRALTGIAVEQDKNTQEVFAQVKQIYKTPPIPDFGGFNFSQILPDPSKPSKRSPIEDLLFNKVTLADAGFIKQYGDCLGDIAARDLICAQKFNGLTVLPPLLTDEMIAQYTSALLAGTITSGWTFGAGPALQIPFPMQMAYRFNGIGVTQNVLYENQKLIANQFNSAIGKIQDSLSSTPSALGKLQNVVNQNAQALNTLVKCLSSNFGAISSVLNDILSRLDPPEAEVQIDRLITGRLQCLQTYVTQQLIRAAEIRASANLAATKMSECVLGQSKRVDFCGKGYHLMSFPQSAPHGVVFLHVTYVPAQEKNFTTAPAICHDGKAHFPREGVFVSNGTHWFVTQRNFYEPQIITTDNTFVSGNCDVVIGIVNNTVYDPLQPELDSFKEELDKYFKNHTSPDVDLGDISGILASVVNIQKEIDRLNEVAKNLNESLIDLQELGKYEQYIKWPGYIPEAPRDGQAYVRKDGEWVLLSTFLHHHHHH

SEQ ID NO: 77 - protein, 1242 aa, synthetic construct
MFVFLVLLPLVSSQCVNLITRTQSYTNSFTRGVYYPDKVFRSSVLHSTQDLFLPFFSNVTWFHAIHVSGTNGTKRFDNPALPFNDGVYFASTEKSNIIRGWIFGTTLDSKTQSLLIVNNATNVVIKVCEFQFCNDPFLDVYQKNNKSWMESEFRVYSSANNCTFEYVSQPFLMDLEGKNGTFKNLREFVFKNIDGYFKIYSKHTPINLNRTLPQGFSALEPLVDLPIGINITRFQTLLALHRSYLTPVDNSTGWTAGAAAYYVGYLQPRTFLLKYNENGTITDAVDCALDPLSETKCTLKSFTVEKGIYQTSNFRVQPTESIVRFPQITNLCPFGEVFNATKFPSVYAWERKKISNCVADYSVLYNSTFFSTFKCYGVSATKLNDLCFSNVYADSFVVKGDDVRQIAPGQTGVIADYNYKLPDDFMGCVIAWNSNNLDSKVGGNYNYRYRLFRKSKLKPFERDISTEIYQAGSKPCNGVEGFNCYFPLQSYGFQPTYGVGYQPYRVVVLSFELLHAPATVCGPKKSTNLVKNKCVNFNFNGLTGTGVLTESNKKFLPFQQFGRDIADTTDAVRDPQTLEILDITPCSFGGVSVITPGTNTSNQVAVLYQGVNCTEVPVAIHADQLTPTWRVYSTGSNVFQTRAGCLIGAEHVNNSYECDIPIGAGICASYQTQTNSRGSASSVASQSIIAYTMSLGAENSVAYSNNSIAIPTNFTISVTTEILPVSMPKTSVDCTMYICGDSTECSNLLLQYGSFCTQLNRALTGIAVEQDKNTQEVFAQVKQIYKTPPIPDFGGFNFSQILPDPSKPSKRSPIEDLLFNKVTLADAGFIKQYGDCLGDIAARDLICAQKFNGLTVLPPLLTDEMIAQYTSALLAGTITSGWTFGAGPALQIPFPMQMAYRFNGIGVTQNVLYENQKLIANQFNSAIGKIQDSLSSTPSALGKLQNVVNQNAQALNTLVKCLSSNFGAISSVLNDILSRLDPPEAEVQIDRLITGRLQCLQTYVTQQLIRAAEIRASANLAATKMSECVLGQSKRVDFCGKGYHLMSFPQSAPHGVVFLHVTYVPAQEKNFTTAPAICHDGKAHFPREGVFVSNGTHWFVTQRNFYEPQIITTDNTFVSGNCDVVIGIVNNTVYDPLQPELDSFKEELDKYFKNHTSPDVDLGDISGILASVVNIQKEIDRLNEVAKNLNESLIDLQELGKYEQYIKWPGYIPEAPRDGQAYVRKDGEWVLLSTFLHHHHHH

SEQ ID NO: 78 - protein, 1242 aa, synthetic construct
MFVFLVLLPLVSSQCVNLITRTQSYTNSFTRGVYYPDKVFRSSVLHSTQDLFLPFFSNVTWFHAIHVSGTNGTKRFDNPALPFNDGVYFASTEKSNIIRGWIFGTTLDSKTQSLLIVNNATNVVIKVCEFQFCNDPFLDVYQKNNKSWMESEFRVYSSANNCTFEYVSQPFLMDLEGKNGTFKNLREFVFKNIDGYFKIYSKHTPINLERDLPQGFSALEPLVDLPIGINITRFQTLLALHRSYLTPVDSSSGWTAGAAAYYVGYLQPRTFLLKYNENGTITDAVDCALDPLSETKCTLKSFTVEKGIYQTSNFRVQPTESIVRFPQITNLCPFGEVFNATKFPSVYAWERKKISNCVADYSVLYNSTFFSTFKCYGVSATKLNDLCFSNVYADSFVVKGDDVRQIAPGQTGVIADYNYKLPDDFMGCVIAWNSNNLDSKVGGNYNYRYRLFRKSKLKPFERDISTEIYQAGSKPCNGVEGFNCYFPLQSYGFQPTYGVGYQPYRVVVLSFELLHAPATVCGPKKSTNLVKNKCVNFNFNGLTGTGVLTESNKKFLPFQQFGRDIADTTDAVRDPQTLEILDITPCSFGGVSVITPGTNTSNQVAVLYQGVNCTEVPVAIHADQLTPTWRVYSTGSNVFQTRAGCLIGAEHVNNSYECDIPIGAGICASYQTQTNSRGSASSVASQSIIAYTMSLGAENSVAYSNNSIAIPTNFTISVTTEILPVSMPKTSVDCTMYICGDSTECSNLLLQYGSFCTQLNRALTGIAVEQDKNTQEVFAQVKQIYKTPPIPDFGGFNFSQILPDPSKPSKRSPIEDLLFNKVTLADAGFIKQYGDCLGDIAARDLICAQKFNGLTVLPPLLTDEMIAQYTSALLAGTITSGWTFGAGPALQIPFPMQMAYRFNGIGVTQNVLYENQKLIANQFNSAIGKIQDSLSSTPSALGKLQNVVNQNAQALNTLVKCLSSNFGAISSVLNDILSRLDPPEAEVQIDRLITGRLQCLQTYVTQQLIRAAEIRASANLAATKMSECVLGQSKRVDFCGKGYHLMSFPQSAPHGVVFLHVTYVPAQEKNFTTAPAICHDGKAHFPREGVFVSNGTHWFVTQRNFYEPQIITTDNTFVSGNCDVVIGIVNNTVYDPLQPELDSFKEELDKYFKNHTSPDVDLGDISGILASVVNIQKEIDRLNEVAKNLNESLIDLQELGKYEQYIKWPGYIPEAPRDGQAYVRKDGEWVLLSTFLHHHHHH

SEQ ID NO: 79 - protein, 1242 aa, synthetic construct
MFVFLVLLPLVSSQCVNLINRTQSYTNSFTRGVYYPDKVFRSSVLHSTQDLFLPFFSNVTWFHAIHVSGTNGTKRFDNPALPFNDGVYFASTEKSNIIRGWIFGTTLDSKTQSLLIVNNATNVVIKVCEFQFCNDPFLDVYQKNNKSWMESEFRVYSSANNCTFEYVSQPFLMDLEGKEGNFKNLREFVFKNIDGYFKIYSKHTPINLERDLPQGFSALEPLVDLPIGINITRFQTLLALHRSYLTPVDSSSGWTAGAAAYYVGYLQPRTFLLKYNENGTITDAVDCALDPLSETKCTLKSFTVEKGIYQTSNFRVQPTESIVRFPQITNLCPFGEVFNATKFPSVYAWERKKISNCVADYSVLYNSTFFSTFKCYGVSATKLNDLCFSNVYADSFVVKGDDVRQIAPGQTGVIADYNYKLPDDFMGCVIAWNSNNLDSKVGGNYNYRYRLFRKSKLKPFERDISTEIYQAGSKPCNGVEGFNCYFPLQSYGFQPTYGVGYQPYRVVVLSFELLHAPATVCGPKKSTNLVKNKCVNFNFNGLTGTGVLTESNKKFLPFQQFGRDIADTTDAVRDPQTLEILDITPCSFGGVSVITPGTNTSNQVAVLYQGVNCTEVPVAIHADQLTPTWRVYSTGSNVFQTRAGCLIGAEHVNNSYECDIPIGAGICASYQTQTNSRGSASSVASQSIIAYTMSLGAENSVAYSNNSIAIPTNFTISVTTEILPVSMPKTSVDCTMYICGDSTECSNLLLQYGSFCTQLNRALTGIAVEQDKNTQEVFAQVKQIYKTPPIPDFGGFNFSQILPDPSKPSKRSPIEDLLFNKVTLADAGFIKQYGDCLGDIAARDLICAQKFNGLTVLPPLLTDEMIAQYTSALLAGTITSGWTFGAGPALQIPFPMQMAYRFNGIGVTQNVLYENQKLIANQFNSAIGKIQDSLSSTPSALGKLQNVVNQNAQALNTLVKCLSSNFGAISSVLNDILSRLDPPEAEVQIDRLITGRLQCLQTYVTQQLIRAAEIRASANLAATKMSECVLGQSKRVDFCGKGYHLMSFPQSAPHGVVFLHVTYVPAQEKNFTTAPAICHDGKAHFPREGVFVSNGTHWFVTQRNFYEPQIITTDNTFVSGNCDVVIGIVNNTVYDPLQPELDSFKEELDKYFKNHTSPDVDLGDISGILASVVNIQKEIDRLNEVAKNLNESLIDLQELGKYEQYIKWPGYIPEAPRDGQAYVRKDGEWVLLSTFLHHHHHH

SEQ ID NO: 80 - protein, 1242 aa, synthetic construct
MFVFLVLLPLVSSQCVNLITRTQSYTNSFTRGVYYPDKVFRSSVLHSTQDLFLPFFSNVTWFHAIHVSGTNGTKRFDNPALPFNDGVYFASTEKSNIIRGWIFGTTLDSKTQSLLIVNNATNVVIKVCEFQFCNDPFLDVYQKNNKSWMESEFRVYSSANNCTFEYVSQPFLMDLEGKEGNFKNLREFVFKNIDGYFKIYSKHTPINLNRTLPQGFSALEPLVDLPIGINITRFQTLLALHRSYLTPVDSSSGWTAGAAAYYVGYLQPRTFLLKYNENGTITDAVDCALDPLSETKCTLKSFTVEKGIYQTSNFRVQPTESIVRFPQITNLCPFGEVFNATKFPSVYAWERKKISNCVADYSVLYNSTFFSTFKCYGVSATKLNDLCFSNVYADSFVVKGDDVRQIAPGQTGVIADYNYKLPDDFMGCVIAWNSNNLDSKVGGNYNYRYRLFRKSKLKPFERDISTEIYQAGSKPCNGVEGFNCYFPLQSYGFQPTYGVGYQPYRVVVLSFELLHAPATVCGPKKSTNLVKNKCVNFNFNGLTGTGVLTESNKKFLPFQQFGRDIADTTDAVRDPQTLEILDITPCSFGGVSVITPGTNTSNQVAVLYQGVNCTEVPVAIHADQLTPTWRVYSTGSNVFQTRAGCLIGAEHVNNSYECDIPIGAGICASYQTQTNSRGSASSVASQSIIAYTMSLGAENSVAYSNNSIAIPTNFTISVTTEILPVSMPKTSVDCTMYICGDSTECSNLLLQYGSFCTQLNRALTGIAVEQDKNTQEVFAQVKQIYKTPPIPDFGGFNFSQILPDPSKPSKRSPIEDLLFNKVTLADAGFIKQYGDCLGDIAARDLICAQKFNGLTVLPPLLTDEMIAQYTSALLAGTITSGWTFGAGPALQIPFPMQMAYRFNGIGVTQNVLYENQKLIANQFNSAIGKIQDSLSSTPSALGKLQNVVNQNAQALNTLVKCLSSNFGAISSVLNDILSRLDPPEAEVQIDRLITGRLQCLQTYVTQQLIRAAEIRASANLAATKMSECVLGQSKRVDFCGKGYHLMSFPQSAPHGVVFLHVTYVPAQEKNFTTAPAICHDGKAHFPREGVFVSNGTHWFVTQRNFYEPQIITTDNTFVSGNCDVVIGIVNNTVYDPLQPELDSFKEELDKYFKNHTSPDVDLGDISGILASVVNIQKEIDRLNEVAKNLNESLIDLQELGKYEQYIKWPGYIPEAPRDGQAYVRKDGEWVLLSTFLHHHHHH

SEQ ID NO: 81 - protein, 1242 aa, synthetic construct
MFVFLVLLPLVSSQCVNLITRTQSYTNSFTRGVYYPDKVFRSSVLHSTQDLFLPFFSSVTWFHAIHVSGTAGTKRFDNPALPFNDGVYFASTEKSNIIRGWIFGTTLDSKTQSLLIVNNATNVVIKVCEFQFCNDPFLDVYQKNNKSWMESEFRVYSSANNCTFEYVSQPFLMDLEGKEGNFKNLREFVFKNIDGYFKIYSKHTPINLERDLPQGFSALEPLVDLPIGINITRFQTLLALHRSYLTPVDSSSGWTAGAAAYYVGYLQPRTFLLKYNEQGTITDAVDCALDPLSETKCTLKSFTVEKGIYQTSNFRVQPTESIVRFPQITNLCPFGEVFNATKFPSVYAWERKKISNCVADYSVLYNSTFFSTFKCYGVSATKLNDLCFSNVYADSFVVKGDDVRQIAPGQTGVIADYNYKLPDDFMGCVIAWNSNNLDSKVGGNYNYRYRLFRKSKLKPFERDISTEIYQAGSKPCNGVEGFNCYFPLQSYGFQPTYGVGYQPYRVVVLSFELLHAPATVCGPKKSTNLVKNKCVNFNFNGLTGTGVLTESNKKFLPFQQFGRDIADTTDAVRDPQTLEILDITPCSFGGVSVITPGTNTSNQVAVLYQGVNCTEVPVAIHADQLTPTWRVYSTGSNVFQTRAGCLIGAEHVNNSYECDIPIGAGICASYQTQTNSRGSASSVASQSIIAYTMSLGAENSVAYSNNSIAIPTNFTISVTTEILPVSMPKTSVDCTMYICGDSTECSNLLLQYGSFCTQLNRALTGIAVEQDKNTQEVFAQVKQIYKTPPIPDFGGFNFSQILPDPSKPSKRSPIEDLLFNKVTLADAGFIKQYGDCLGDIAARDLICAQKFNGLTVLPPLLTDEMIAQYTSALLAGTITSGWTFGAGPALQIPFPMQMAYRFNGIGVTQNVLYENQKLIANQFNSAIGKIQDSLSSTPSALGKLQNVVNQNAQALNTLVKCLSSNFGAISSVLNDILSRLDPPEAEVQIDRLITGRLQCLQTYVTQQLIRAAEIRASANLAATKMSECVLGQSKRVDFCGKGYHLMSFPQSAPHGVVFLHVTYVPAQEKNFTTAPAICHDGKAHFPREGVFVSNGTHWFVTQRNFYEPQIITTDNTFVSGNCDVVIGIVNNTVYDPLQPELDSFKEELDKYFKNHTSPDVDLGDISGILASVVNIQKEIDRLNEVAKNLNESLIDLQELGKYEQYIKWPGYIPEAPRDGQAYVRKDGEWVLLSTFLHHHHHH

SEQ ID NO: 82 - protein, 1242 aa, synthetic construct
MFVFLVLLPLVSSQCVNLITRTQSYTNSFTRGVYYPDKVFRSSVLHSTQDLFLPFFSNVTWFHAIHVSGTNGTKRFDNPALPFNDGVYFASTEKSNIIRGWIFGTTLDSKTQSLLIVNNATNVVIKVCEFQFCNDPFLDVYQKNNKSWMESEFRVYSSANNCTFEYVSQPFLMDLEGKEGNFKNLREFVFKNIDGYFKIYSKHTPINLERDLPQGFSALEPLVDLPIGINITRFQTLLALHRSYLTPVDSSSGWTAGAAAYYVGYLQPRTFLLKYNENGTITDAVDCALDPLSETKCTLKSFTVEKGIYQTSNFRVQPTESIVRFPQITNLCPFGEVFNATKFPSVYAWERKKISNCVADYSVLYNSTFFSTFKCYGVNATKLNDLCFSNVYADSFVVKGDDVRQIAPGQTGVIADYNYKLPDDFMGCVIAWNSNNLDSKVGGNYNYRYRLFRKSNLTPFERDNSTEIYQAGSKPCNGVEGFNCYFPLQSYGFQPTYGVGYQPYRVVVLSFELLHAPATVCGPKKSTNLVKNKCVNFNFNGLTGTGVLTESNKKFLPFQQFGRDIADTTDAVRDPQTLEILDITPCSFGGVSVITPGTNTSNQVAVLYQGVNCTEVPVAIHADQLTPTWRVYSTGSNVFQTRAGCLIGAEHVNNSYECDIPIGAGICASYQTQTNSRGSASSVASQSIIAYTMSLGAENSVAYSNNSIAIPTNFTISVTTEILPVSMPKTSVDCTMYICGDSTECSNLLLQYGSFCTQLNRALTGIAVEQDKNTQEVFAQVKQIYKTPPIPDFGGFNFSQILPDPSKPSKRSPIEDLLFNKVTLADAGFIKQYGDCLGDIAARDLICAQKFNGLTVLPPLLTDEMIAQYTSALLAGTITSGWTFGAGPALQIPFPMQMAYRFNGIGVTQNVLYENQKLIANQFNSAIGKIQDSLSSTPSALGKLQNVVNQNAQALNTLVKCLSSNFGAISSVLNDILSRLDPPEAEVQIDRLITGRLQCLQTYVTQQLIRAAEIRASANLAATKMSECVLGQSKRVDFCGKGYHLMSFPQSAPHGVVFLHVTYVPAQEKNFTTAPAICHDGKAHFPREGVFVSNGTHWFVTQRNFYEPQIITTDNTFVSGNCDVVIGIVNNTVYDPLQPELDSFKEELDKYFKNHTSPDVDLGDISGILASVVNIQKEIDRLNEVAKNLNESLIDLQELGKYEQYIKWPGYIPEAPRDGQAYVRKDGEWVLLSTFLHHHHHH

SEQ ID NO: 83 - protein, 1242 aa, synthetic construct
MFVFLVLLPLVSSQCVNLITRTQSYTNSFTRGVYYPDKVFRSSVLHSTQDLFLPFFSNVTWFHAIHVSGTNGTKRFDNPALPFNDGVYFASTEKSNIIRGWIFGTTLDSKTQSLLIVNNATNVVIKVCEFQFCNDPFLDVYNKTNKSWMESEFRVYSSANNCTFEYVSQPFLMDLEGKEGNFKNLREFVFKNIDGYFKIYSKHTPINLERDLPQGFSALEPLVDLPIGINITRFQTLLALHRSYLTPVDSSSGWTAGAAAYYVGYLQPRTFLLKYNENGTITDAVDCALDPLSETKCTLKSFTVEKGIYQTSNFRVQPTESIVRFPQITNLCPFGEVFNATKFPSVYAWERKKISNCVADYSVLYNSTFFSTFKCYGVSATKLNDLCFSNVYADSFVVKGDDVRQIAPGQTGVIADYNYKLPDDFMGCVIAWNSNNLDSKVGGNYNYRYRLFRKSKLKPFERDISTEIYQAGSKPCNGVEGFNCYFPLQSYGFQPTYGVGYQPYRVVVLSFELLHAPATVCGPKKSTNLVKNKCVNFNFNGLTGTGVLTESNKKFLPFQQFGRDIADTTDAVRDPQTLEILDITPCSFGGVSVITPGTNTSNQVAVLYQGVNCTEVPVAIHADQLTPTWRVYSTGSNVFQTRAGCLIGAEHVNNSYECDIPIGAGICASYQTQTNSRGSASSVASQSIIAYTMSLGAENSVAYSNNSIAIPTNFTISVTTEILPVSMPKTSVDCTMYICGDSTECSNLLLQYGSFCTQLNRALTGIAVEQDKNTQEVFAQVKQIYKTPPIPDFGGFNFSQILPDPSKPSKRSPIEDLLFNKVTLADAGFIKQYGDCLGDIAARDLICAQKFNGLTVLPPLLTDEMIAQYTSALLAGTITSGWTFGAGPALQIPFPMQMAYRFNGIGVTQNVLYENQKLIANQFNSAIGKIQDSLSSTPSALGKLQNVVNQNAQALNTLVKCLSSNFGAISSVLNDILSRLDPPEAEVQIDRLITGRLQCLQTYVTQQLIRAAEIRASANLAATKMSECVLGQSKRVDFCGKGYHLMSFPQSAPHGVVFLHVTYVPAQEKNFTTAPAICHDGKAHFPREGVFVSNGTHWFVTQRNFYEPQIITTDNTFVSGNCDVVIGIVNNTVYDPLQPELDSFKEELDKYFKNHTSPDVDLGDISGILASVVNIQKEIDRLNEVAKNLNESLIDLQELGKYEQYIKWPGYIPEAPRDGQAYVRKDGEWVLLSTFLHHHHHH

SEQ ID NO: 84 - protein, 1242 aa, synthetic construct
MFVFLVLLPLVSSQCVNLITRTQSYTNSFTRGVYYPDKVFRSSVLHSTQDLFLPFFSNVTWFHAIHVSGTNGTKRFDNPALPFNDGVYFASTEKSNIIRGWIFGTTLDSKTQSLLIVNNATNVVIKVCEFQFCNDPFLDVYQKNNKSWMESEFRVYSSANNCTFEYVSQPFLMDLEGKEGNFKNLREFVFKNIDGYFKIYSKHTPINLERDLPQGFSALEPLVDLPIGINITRFQTLLALHRSYLTPVDSSSGWTAGAAAYYVGYLQPRTFLLKYNENGTITDAVDCALDPLSETKCTLKSFTVEKGIYQTSNFRVQPTESIVRFPQITNLCPFGEVFNATKFPSVYAWERKKISNCVADYSVLYNSTFFSTFKCYGVNATKLNDLCFSNVYADSFVVKGDDVRQIAPGQTGVIADYNYKLPDDFMGCVIAWNSNNLDSKVGGNYNYRYRLFRKSKLKPFERDNSTEIYQAGSKPCNGVEGFNCYFPLQSYGFQPTYGVGYQPYRVVVLSFELLHAPATVCGPKKSTNLVKNKCVNFNFNGLTGTGVLTESNKKFLPFQQFGRDIADTTDAVRDPQTLEILDITPCSFGGVSVITPGTNTSNQVAVLYQGVNCTEVPVAIHADQLTPTWRVYSTGSNVFQTRAGCLIGAEHVNNSYECDIPIGAGICASYQTQTNSRGSASSVASQSIIAYTMSLGAENSVAYSNNSIAIPTNFTISVTTEILPVSMPKTSVDCTMYICGDSTECSNLLLQYGSFCTQLNRALTGIAVEQDKNTQEVFAQVKQIYKTPPIPDFGGFNFSQILPDPSKPSKRSPIEDLLFNKVTLADAGFIKQYGDCLGDIAARDLICAQKFNGLTVLPPLLTDEMIAQYTSALLAGTITSGWTFGAGPALQIPFPMQMAYRFNGIGVTQNVLYENQKLIANQFNSAIGKIQDSLSSTPSALGKLQNVVNQNAQALNTLVKCLSSNFGAISSVLNDILSRLDPPEAEVQIDRLITGRLQCLQTYVTQQLIRAAEIRASANLAATKMSECVLGQSKRVDFCGKGYHLMSFPQSAPHGVVFLHVTYVPAQEKNFTTAPAICHDGKAHFPREGVFVSNGTHWFVTQRNFYEPQIITTDNTFVSGNCDVVIGIVNNTVYDPLQPELDSFKEELDKYFKNHTSPDVDLGDISGILASVVNIQKEIDRLNEVAKNLNESLIDLQELGKYEQYIKWPGYIPEAPRDGQAYVRKDGEWVLLSTFLHHHHHH

SEQ ID NO: 85 - protein, 1242 aa, synthetic construct
MFVFLVLLPLVSSQCVNLITRTQSYTNSFTRGVYYPDKVFRSSVLHSTQDLFLPFFSNVTWFHAIHVSGTNGTKRFDNPALPFNDGVYFASTEKSNIIRGWIFGTTLDSKTQSLLIVNNATNVVIKVCEFQFCNDPFLDVYQKNNKSWMESEFRVYSSANNCTFEYVSQPFLMDLEGKNGTFKNLREFVFKNIDGYFKIYSKHTPINLNRTLPQGFSALEPLVDLPIGINITRFQTLLALHRSYLTPVDSSSGWTAGAAAYYVGYLQPRTFLLKYNENGTITDAVDCALDPLSETKCTLKSFTVEKGIYQTSNFRVQPTESIVRFPQITNLCPFGEVFNATKFPSVYAWERKKISNCVADYSVLYNSTFFSTFKCYGVSATKLNDLCFSNVYADSFVVKGDDVRQIAPGQTGVIADYNYKLPDDFMGCVIAWNSNNLDSKVGGNYNYRYRLFRKSKLKPFERDISTEIYQAGSKPCNGVEGFNCYFPLQSYGFQPTYGVGYQPYRVVVLSFELLHAPATVCGPKKSTNLVKNKCVNFNFNGLTGTGVLTESNKKFLPFQQFGRDIADTTDAVRDPQTLEILDITPCSFGGVSVITPGTNTSNQVAVLYQGVNCTEVPVAIHADQLTPTWRVYSTGSNVFQTRAGCLIGAEHVNNSYECDIPIGAGICASYQTQTNSRGSASSVASQSIIAYTMSLGAENSVAYSNNSIAIPTNFTISVTTEILPVSMPKTSVDCTMYICGDSTECSNLLLQYGSFCTQLNRALTGIAVEQDKNTQEVFAQVKQIYKTPPIPDFGGFNFSQILPDPSKPSKRSPIEDLLFNKVTLADAGFIKQYGDCLGDIAARDLICAQKFNGLTVLPPLLTDEMIAQYTSALLAGTITSGWTFGAGPALQIPFPMQMAYRFNGIGVTQNVLYENQKLIANQFNSAIGKIQDSLSSTPSALGKLQNVVNQNAQALNTLVKCLSSNFGAISSVLNDILSRLDPPEAEVQIDRLITGRLQCLQTYVTQQLIRAAEIRASANLAATKMSECVLGQSKRVDFCGKGYHLMSFPQSAPHGVVFLHVTYVPAQEKNFTTAPAICHDGKAHFPREGVFVSNGTHWFVTQRNFYEPQIITTDNTFVSGNCDVVIGIVNNTVYDPLQPELDSFKEELDKYFKNHTSPDVDLGDISGILASVVNIQKEIDRLNEVAKNLNESLIDLQELGKYEQYIKWPGYIPEAPRDGQAYVRKDGEWVLLSTFLHHHHHH

SEQ ID NO: 86 - protein, 1242 aa, synthetic construct
MFVFLVLLPLVSSQCVNLITRTQSYTNSFTRGVYYPDKVFRSSVLHSTQDLFLPFFSNVTWFHAIHVSGTNGTKRFDNPALPFNDGVYFASTEKSNIIRGWIFGTTLDSKTQSLLIVNNATNVVIKVCEFQFCNDPFLDVYQKNNKSWMESEFRVYSSANNCTFEYVSQPFLMDLEGKEGNFKNLREFVFKNIDGYFKIYSKHTPINLERDLPQGFSALEPLVDLPIGINITRFQTLLALHRSYLTPVDSSSGWTAGAAAYYVGYLQPRTFLLKYNEQGTITDAVDCALDPLSETKCTLKSFTVEKGIYQTSNFRVQPTESIVRFPQITNLCPFGEVFNATKFPSVYAWERKKISNCVADYSVLYNSTFFSTFKCYGVSATKLNDLCFSNVYADSFVVKGDDVRQIAPGQTGVIADYNYKLPDDFMGCVIAWNSNNLDSKVGGNYNYRYRLFRKSKLKPFERDISTEIYQAGSKPCNGVEGFNCYFPLQSYGFQPTYGVGYQPYRVVVLSFELLHAPATVCGPKKSTNLVKNKCVNFNFNGLTGTGVLTESNKKFLPFQQFGRDIADTTDAVRDPQTLEILDITPCSFGGVSVITPGTNTSNQVAVLYQGVNCTEVPVAIHADQLTPTWRVYSTGSNVFQTRAGCLIGAEHVNNSYECDIPIGAGICASYQTQTNSRGSASSVASQSIIAYTMSLGAENSVAYSNNSIAIPTNFTISVTTEILPVSMPKTSVDCTMYICGDSTECSNLLLQYGSFCTQLNRALTGIAVEQDKNTQEVFAQVKQIYKTPPIPDFGGFNFSQILPDPSKPSKRSPIEDLLFNKVTLADAGFIKQYGDCLGDIAARDLICAQKFNGLTVLPPLLTDEMIAQYTSALLAGTITSGWTFGAGPALQIPFPMQMAYRFNGIGVTQNVLYENQKLIANQFNSAIGKIQDSLSSTPSALGKLQNVVNQNAQALNTLVKCLSSNFGAISSVLNDILSRLDPPEAEVQIDRLITGRLQCLQTYVTQQLIRAAEIRASANLAATKMSECVLGQSKRVDFCGKGYHLMSFPQSAPHGVVFLHVTYVPAQEKNFTTAPAICHDGKAHFPREGVFVSNGTHWFVTQRNFYEPQIITTDNTFVSGNCDVVIGIVNNTVYDPLQPELDSFKEELDKYFKNHTSPDVDLGDISGILASVVNIQKEIDRLNEVAKNLNESLIDLQELGKYEQYIKWPGYIPEAPRDGQAYVRKDGEWVLLSTFLHHHHHH

SEQ ID NO: 87 - protein, 1242 aa, synthetic construct
MFVFLVLLPLVSSQCVNLITRTQSYTNSFTRGVYYPDKVFRSSVLHSTQDLFLPFFSNVTWFHAIHVSGTNGTKRFDNPALPFNDGVYFASTEKSNIIRGWIFGTTLDSKTQSLLIVNNATNVVIKVCEFQFCNDPFLDVYQKNNKSWMESEFRVYSSANNCTFEYVSQPFLMDLEGKEGNFKNLREFVFKNIDGYFKIYSKHTPINLERDLPQGFSALEPLVDLPIGINITRFQTLLALHRSYLTPVDSSSGWTAGAAAYYVGYLQPRTFLLKYNENGTITDAVDCALDPLSETKCTLKSFTVEKGIYQTSNFRVQPTESIVRFPQITNLCPFGEVFNATKFPSVYAWERKKISNCVADYSVLYNSTFFSTFKCYGVNATKLNDLCFSNVYADSFVVKGDDVRQIAPGQTGVIADYNYKLPDDFMGCVIAWNSNNLDSKVGGNYNYRYRLFRKSKLKPFERDNSTEIYQAGSKPCNGVEGFNCYFPLQSYGFQPTYGVGYQPYRVVVLSFELNHTPATVCGPKKSTNLVKNKCVNFNFNGLTGTGVLTESNKKFLPFQQFGRDIADTTDAVRDPQTLEILDITPCSFGGVSVITPGTNTSNQVAVLYQGVNCTEVPVAIHADQLTPTWRVYSTGSNVFQTRAGCLIGAEHVNNSYECDIPIGAGICASYQTQTNSRGSASSVASQSIIAYTMSLGAENSVAYSNNSIAIPTNFTISVTTEILPVSMPKTSVDCTMYICGDSTECSNLLLQYGSFCTQLNRALTGIAVEQDKNTQEVFAQVKQIYKTPPIPDFGGFNFSQILPDPSKPSKRSPIEDLLFNKVTLADAGFIKQYGDCLGDIAARDLICAQKFNGLTVLPPLLTDEMIAQYTSALLAGTITSGWTFGAGPALQIPFPMQMAYRFNGIGVTQNVLYENQKLIANQFNSAIGKIQDSLSSTPSALGKLQNVVNQNAQALNTLVKCLSSNFGAISSVLNDILSRLDPPEAEVQIDRLITGRLQCLQTYVTQQLIRAAEIRASANLAATKMSECVLGQSKRVDFCGKGYHLMSFPQSAPHGVVFLHVTYVPAQEKNFTTAPAICHDGKAHFPREGVFVSNGTHWFVTQRNFYEPQIITTDNTFVSGNCDVVIGIVNNTVYDPLQPELDSFKEELDKYFKNHTSPDVDLGDISGILASVVNIQKEIDRLNEVAKNLNESLIDLQELGKYEQYIKWPGYIPEAPRDGQAYVRKDGEWVLLSTFLHHHHHH

SEQ ID NO: 88 - protein, 1242 aa, synthetic construct
MFVFLVLLPLVSSQCVNLINRTQSYTNSFTRGVYYPDKVFRSSVLHSTQDLFLPFFSNVTWFHAIHVSGTNGTKRFDNPALPFNDGVYFASTEKSNIIRGWIFGTTLDSKTQSLLIVNNATNVVIKVCEFQFCNDPFLDVYQKNNKSWMESEFRVYSSANNCTFEYVSQPFLMDLEGKEGNFKNLREFVFKNIDGYFKIYSKHTPINLNRTLPQGFSALEPLVDLPIGINITRFQTLLALHRSYLTPVDSSSGWTAGAAAYYVGYLQPRTFLLKYNENGTITDAVDCALDPLSETKCTLKSFTVEKGIYQTSNFRVQPTESIVRFPQITNLCPFGEVFNATKFPSVYAWERKKISNCVADYSVLYNSTFFSTFKCYGVSATKLNDLCFSNVYADSFVVKGDDVRQIAPGQTGVIADYNYKLPDDFMGCVIAWNSNNLDSKVGGNYNYRYRLFRKSKLKPFERDISTEIYQAGSKPCNGVEGFNCYFPLQSYGFQPTYGVGYQPYRVVVLSFELLHAPATVCGPKKSTNLVKNKCVNFNFNGLTGTGVLTESNKKFLPFQQFGRDIADTTDAVRDPQTLEILDITPCSFGGVSVITPGTNTSNQVAVLYQGVNCTEVPVAIHADQLTPTWRVYSTGSNVFQTRAGCLIGAEHVNNSYECDIPIGAGICASYQTQTNSRGSASSVASQSIIAYTMSLGAENSVAYSNNSIAIPTNFTISVTTEILPVSMPKTSVDCTMYICGDSTECSNLLLQYGSFCTQLNRALTGIAVEQDKNTQEVFAQVKQIYKTPPIPDFGGFNFSQILPDPSKPSKRSPIEDLLFNKVTLADAGFIKQYGDCLGDIAARDLICAQKFNGLTVLPPLLTDEMIAQYTSALLAGTITSGWTFGAGPALQIPFPMQMAYRFNGIGVTQNVLYENQKLIANQFNSAIGKIQDSLSSTPSALGKLQNVVNQNAQALNTLVKCLSSNFGAISSVLNDILSRLDPPEAEVQIDRLITGRLQCLQTYVTQQLIRAAEIRASANLAATKMSECVLGQSKRVDFCGKGYHLMSFPQSAPHGVVFLHVTYVPAQEKNFTTAPAICHDGKAHFPREGVFVSNGTHWFVTQRNFYEPQIITTDNTFVSGNCDVVIGIVNNTVYDPLQPELDSFKEELDKYFKNHTSPDVDLGDISGILASVVNIQKEIDRLNEVAKNLNESLIDLQELGKYEQYIKWPGYIPEAPRDGQAYVRKDGEWVLLSTFLHHHHHH

SEQ ID NO: 89 - protein, 1242 aa, synthetic construct
MFVFLVLLPLVSSQCVNLITRTQSYTNSFTRGVYYPDKVFRSSVLHSTQDLFLPFFSNVTWFHAIHVSGTNGTKRFDNPALPFNDGVYFASTEKSNIIRGWIFGTTLDSKTQSLLIVNNATNVVIKVCEFQFCNDPFLDVYQKNNKSWMESEFRVYSSANNCTFEYVSQPFLMDLEGKEGNFKNLREFVFKNIDGYFKIYSKHTPINLERDLPQGFSALEPLVDLPIGINITRFQTLLALHRSYLTPVDSSSGWTAGAAAYYVGYLQPRTFLLKYNENGTITDAVDCALDPLSETKCTLKSFTVEKGIYQTSNFRVQPTESIVRFPQITNLCPFGEVFNATKFPSVYAWERKKISNCVADYSVLYNSTFFSTFKCYGVNATKLNDLCFSNVYADSFVVKGDDVRQIAPGQTGVIADYNYKLPDDFMGCVIAWNSNNLDSKVGGNYNYRYRLFRKSKLKPFERDISTEIYQAGSKPCNGVEGFNCYFPLQSYGFQPTYGVGYQPYRVVVLSFELNHTPATVCGPKKSTNLVKNKCVNFNFNGLTGTGVLTESNKKFLPFQQFGRDIADTTDAVRDPQTLEILDITPCSFGGVSVITPGTNTSNQVAVLYQGVNCTEVPVAIHADQLTPTWRVYSTGSNVFQTRAGCLIGAEHVNNSYECDIPIGAGICASYQTQTNSRGSASSVASQSIIAYTMSLGAENSVAYSNNSIAIPTNFTISVTTEILPVSMPKTSVDCTMYICGDSTECSNLLLQYGSFCTQLNRALTGIAVEQDKNTQEVFAQVKQIYKTPPIPDFGGFNFSQILPDPSKPSKRSPIEDLLFNKVTLADAGFIKQYGDCLGDIAARDLICAQKFNGLTVLPPLLTDEMIAQYTSALLAGTITSGWTFGAGPALQIPFPMQMAYRFNGIGVTQNVLYENQKLIANQFNSAIGKIQDSLSSTPSALGKLQNVVNQNAQALNTLVKCLSSNFGAISSVLNDILSRLDPPEAEVQIDRLITGRLQCLQTYVTQQLIRAAEIRASANLAATKMSECVLGQSKRVDFCGKGYHLMSFPQSAPHGVVFLHVTYVPAQEKNFTTAPAICHDGKAHFPREGVFVSNGTHWFVTQRNFYEPQIITTDNTFVSGNCDVVIGIVNNTVYDPLQPELDSFKEELDKYFKNHTSPDVDLGDISGILASVVNIQKEIDRLNEVAKNLNESLIDLQELGKYEQYIKWPGYIPEAPRDGQAYVRKDGEWVLLSTFLHHHHHH

SEQ ID NO: 90 - protein, 1242 aa, synthetic construct
MFVFLVLLPLVSSQCVNLITRTQSYTNSFTRGVYYPDKVFRSSVLHSTQDLFLPFFSSVTWFHAIHVSGTNGTKRFDNPALPFNDGVYFASTEKSNIIRGWIFGTTLDSKTQSLLIVNNATNVVIKVCEFQFCNDPFLDVYQKNNKSWMESEFRVYSSANNCKFEYVSQPFLMDLEGKEGNFKNLREFVFKNIDGYFKIYSKHTPINLERDLPQGFSALEPLVDLPIGIVITRFQTLLALHRSYLTPVDSSSGWTAGAAAYYVGYLQPRTFLLKYNENGTITDAVDCALDPLSETKCTLKSFTVEKGIYQTSNFRVQPTESIVRFPQITNLCPFGEVFNATKFPSVYAWERKKISNCVADYSVLYNSTFFSTFKCYGVSATKLNDLCFSNVYADSFVVKGDDVRQIAPGQTGVIADYNYKLPDDFMGCVIAWNSNNLDSKVGGNYNYRYRLFRKSKLKPFERDISTEIYQAGSKPCNGVEGFNCYFPLQSYGFQPTYGVGYQPYRVVVLSFELLHAPATVCGPKKSTNLVKNKCVNFNFNGLTGTGVLTESNKKFLPFQQFGRDIADTTDAVRDPQTLEILDITPCSFGGVSVITPGTNTSNQVAVLYQGVNCTEVPVAIHADQLTPTWRVYSTGSNVFQTRAGCLIGAEHVNNSYECDIPIGAGICASYQTQTNSRGSASSVASQSIIAYTMSLGAENSVAYSNNSIAIPTNFTISVTTEILPVSMPKTSVDCTMYICGDSTECSNLLLQYGSFCTQLNRALTGIAVEQDKNTQEVFAQVKQIYKTPPIPDFGGFNFSQILPDPSKPSKRSPIEDLLFNKVTLADAGFIKQYGDCLGDIAARDLICAQKFNGLTVLPPLLTDEMIAQYTSALLAGTITSGWTFGAGPALQIPFPMQMAYRFNGIGVTQNVLYENQKLIANQFNSAIGKIQDSLSSTPSALGKLQNVVNQNAQALNTLVKCLSSNFGAISSVLNDILSRLDPPEAEVQIDRLITGRLQCLQTYVTQQLIRAAEIRASANLAATKMSECVLGQSKRVDFCGKGYHLMSFPQSAPHGVVFLHVTYVPAQEKNFTTAPAICHDGKAHFPREGVFVSNGTHWFVTQRNFYEPQIITTDNTFVSGNCDVVIGIVNNTVYDPLQPELDSFKEELDKYFKNHTSPDVDLGDISGILASVVNIQKEIDRLNEVAKNLNESLIDLQELGKYEQYIKWPGYIPEAPRDGQAYVRKDGEWVLLSTFLHHHHHH

SEQ ID NO: 91 - protein, 1242 aa, synthetic construct
MFVFLVLLPLVSSQCVNLITRTQSYTNSFTRGVYYPDKVFRSSVLHSTQDLFLPFFSNVTWFHAIHVNGTNGTKRFDNPALPFNDGVYFASTEKSNIIRGWIFGTTLDSKTQSLLIVNNATNVVIKVCEFQFCNDPFLDVYQKNNKSWMESEFRVYSSANNCTFEYVSQPFLMDLEGKEGNFKNLREFVFKNIDGYFKIYSKHTPINLERDLPQGFSALEPLVDLPIGINITRFQTLLALHRSYLTPVDSSSGWTAGAAAYYVGYLQPRTFLLKYNENGTITDAVDCALDPLSETKCTLKSFTVEKGIYQTSNFRVQPTESIVRFPQITNLCPFGEVFNATKFPSVYAWERKKISNCVADYSVLYNSTFFSTFKCYGVSATKLNDLCFSNVYADSFVVKGDDVRQIAPGQTGVIADYNYKLPDDFMGCVIAWNSNNLDSKVGGNYNYRYRLFRKSKLKPFERDISTEIYQAGSKPCNGVEGFNCYFPLQSYGFQPTYGVGYQPYRVVVLSFELLHAPATVCGPKKSTNLVKNKCVNFNFNGLTGTGVLTESNKKFLPFQQFGRDIADTTDAVRDPQTLEILDITPCSFGGVSVITPGTNTSNQVAVLYQGVNCTEVPVAIHADQLTPTWRVYSTGSNVFQTRAGCLIGAEHVNNSYECDIPIGAGICASYQTQTNSRGSASSVASQSIIAYTMSLGAENSVAYSNNSIAIPTNFTISVTTEILPVSMPKTSVDCTMYICGDSTECSNLLLQYGSFCTQLNRALTGIAVEQDKNTQEVFAQVKQIYKTPPIPDFGGFNFSQILPDPSKPSKRSPIEDLLFNKVTLADAGFIKQYGDCLGDIAARDLICAQKFNGLTVLPPLLTDEMIAQYTSALLAGTITSGWTFGAGPALQIPFPMQMAYRFNGIGVTQNVLYENQKLIANQFNSAIGKIQDSLSSTPSALGKLQNVVNQNAQALNTLVKCLSSNFGAISSVLNDILSRLDPPEAEVQIDRLITGRLQCLQTYVTQQLIRAAEIRASANLAATKMSECVLGQSKRVDFCGKGYHLMSFPQSAPHGVVFLHVTYVPAQEKNFTTAPAICHDGKAHFPREGVFVSNGTHWFVTQRNFYEPQIITTDNTFVSGNCDVVIGIVNNTVYDPLQPELDSFKEELDKYFKNHTSPDVDLGDISGILASVVNIQKEIDRLNEVAKNLNESLIDLQELGKYEQYIKWPGYIPEAPRDGQAYVRKDGEWVLLSTFLHHHHHH

SEQ ID NO: 92 - protein, 1242 aa, synthetic construct
MFVFLVLLPLVSSQCVNLITRTQSYTNSFTRGVYYPDKVFRSSVLHSTQDLFLPFFSNVTWFHAIHVSGTNGTKRFDNPALPFNDGVYFASTEKSNIIRGWIFGTTLDSKTQSLLIVNNATNVVIKVCEFQFCNDPFLDVYQKNNKSWMESEFRVYSSANNCTFEYVSQPFLMDLEGKEGNFKNLREFVFKNIDGYFKIYSKHTPINLERDLPQGFSALEPLVDLPIGINITRFQTLLALHRSYLTPVDSSSGWTAGAAAYYVGYLQPRTFLLKYNENGTITDAVDCALDPLSETKCTLKSFTVEKGIYQTSNFRVQPTESIVRFPQITNLCPFGEVFNATKFPSVYAWERKKISNCVADYSVLYNSTFFSTFKCYGVSATKLNDLCFSNVYADSFVVKGDDVRQIAPGQTGVIADYNYKLPDDFMGCVIAWNSNNLDSKNGTNYNYRYRLFRKSKLKPFERDISTEIYQAGSKPCNGVEGFNCYFPLQSYGFQPTYGVGYQPYRVVVLSFELLHAPATVCGPKKSTNLVKNKCVNFNFNGLTGTGVLTESNKKFLPFQQFGRDIADTTDAVRDPQTLEILDITPCSFGGVSVITPGTNTSNQVAVLYQGVNCTEVPVAIHADQLTPTWRVYSTGSNVFQTRAGCLIGAEHVNNSYECDIPIGAGICASYQTQTNSRGSASSVASQSIIAYTMSLGAENSVAYSNNSIAIPTNFTISVTTEILPVSMPKTSVDCTMYICGDSTECSNLLLQYGSFCTQLNRALTGIAVEQDKNTQEVFAQVKQIYKTPPIPDFGGFNFSQILPDPSKPSKRSPIEDLLFNKVTLADAGFIKQYGDCLGDIAARDLICAQKFNGLTVLPPLLTDEMIAQYTSALLAGTITSGWTFGAGPALQIPFPMQMAYRFNGIGVTQNVLYENQKLIANQFNSAIGKIQDSLSSTPSALGKLQNVVNQNAQALNTLVKCLSSNFGAISSVLNDILSRLDPPEAEVQIDRLITGRLQCLQTYVTQQLIRAAEIRASANLAATKMSECVLGQSKRVDFCGKGYHLMSFPQSAPHGVVFLHVTYVPAQEKNFTTAPAICHDGKAHFPREGVFVSNGTHWFVTQRNFYEPQIITTDNTFVSGNCDVVIGIVNNTVYDPLQPELDSFKEELDKYFKNHTSPDVDLGDISGILASVVNIQKEIDRLNEVAKNLNESLIDLQELGKYEQYIKWPGYIPEAPRDGQAYVRKDGEWVLLSTFLHHHHHH

SEQ ID NO: 93 - protein, 1242 aa, synthetic construct
MFVFLVLLPLVSSQCVNLITRTQSYTNSFTRGVYYPDKVFRSSVLHSTQDLFLPFFSNVTWFHAIHVSGTNGTKRFDNPALPFNDGVYFASTEKSNIIRGWIFGTTLDSKTQSLLIVNNATNVVIKVCEFQFCNDPFLDVYQKNNKSWMESEFRVYSSANNCTFEYVSQPFLMDLEGKEGNFKNLREFVFKNIDGYFKIYSKHTPINLERDLPQGFSALEPLVDLPIGINITRFQTLLALHRSYLTPVDSSSGWTAGAAAYYVGYLQPRTFLLKYNENGTITDAVDCALDPLSETKCTLKSFTVEKGIYQTSNFRVQPTESIVRFPQITNLCPFHEVFNATTFPSVYAWERKKISNCVADYSVLYNSTFFSTFKCYGVSATKLNDLCFSNVYADSFVVKGDDVRQIAPGQTGVIADYNYKLPDDFMGCVIAWNSNNLDSKVGGNYNYRYRLFRKSKLKPFERDISTEIYQAGSKPCNGVEGFNCYFPLQSYGFQPTYGVGYQPYRVVVLSFELLHAPATVCGPKKSTNLVKNKCVNFNFNGLTGTGVLTESNKKFLPFQQFGRDIADTTDAVRDPQTLEILDITPCSFGGVSVITPGTNTSNQVAVLYQGVNCTEVPVAIHADQLTPTWRVYSTGSNVFQTRAGCLIGAEHVNNSYECDIPIGAGICASYQTQTNSRGSASSVASQSIIAYTMSLGAENSVAYSNNSIAIPTNFTISVTTEILPVSMPKTSVDCTMYICGDSTECSNLLLQYGSFCTQLNRALTGIAVEQDKNTQEVFAQVKQIYKTPPIPDFGGFNFSQILPDPSKPSKRSPIEDLLFNKVTLADAGFIKQYGDCLGDIAARDLICAQKFNGLTVLPPLLTDEMIAQYTSALLAGTITSGWTFGAGPALQIPFPMQMAYRFNGIGVTQNVLYENQKLIANQFNSAIGKIQDSLSSTPSALGKLQNVVNQNAQALNTLVKCLSSNFGAISSVLNDILSRLDPPEAEVQIDRLITGRLQCLQTYVTQQLIRAAEIRASANLAATKMSECVLGQSKRVDFCGKGYHLMSFPQSAPHGVVFLHVTYVPAQEKNFTTAPAICHDGKAHFPREGVFVSNGTHWFVTQRNFYEPQIITTDNTFVSGNCDVVIGIVNNTVYDPLQPELDSFKEELDKYFKNHTSPDVDLGDISGILASVVNIQKEIDRLNEVAKNLNESLIDLQELGKYEQYIKWPGYIPEAPRDGQAYVRKDGEWVLLSTFLHHHHHH

SEQ ID NO: 94 - protein, 1242 aa, synthetic construct
MFVFLVLLPLVSSQCVNLITRTQSYTNSFTRGVYYPDKVFRSSVLHSTQDLFLPFFSNVTWFHAIHVSGTNGTKRFDNPALPFNDGVYFASTEKSNIIRGWIFGTTLDSKTQSLLIVNNATNVVIKVCEFQFCNDPFLDVYQKNNKSWMESEFRVYSSANNCTFEYVSQPFLMDLEGKEGNFKNLREFVFKNIDGYFKIYSKHTPINLERDLPQGFSALEPLVDLPIGINITRFQTLLALHRSYLTPVDSSSGWTAGAAAYYVGYLQPRTFLLKYNENGTITDAVDCALDPLSETKCTLKSFTVEKGIYQTSNFRVQPTESIVRFPQITNLCPFGEVFNATKFPSVYAWERKKISNCVADYSVLYNSTFFSTFKCYGVSATKLNDLCFSNVYADSFVVKGDDVRQIAPGQTGVIADYNYKLPDDFMGCVIAWNSNKLDSKVSGNYNYLYRLFRKSKLKPFERDISTEIYQAGSKPCNGVEGFNCYFPLQSYGFQPTYGVGYQPYRVVVLSFELLHAPATVCGPKKSTNLVKNKCVNFNFNGLTGTGVLTESNKKFLPFQQFGRDIADTTDAVRDPQTLEILDITPCSFGGVSVITPGTNTSNQVAVLYQGVNCTEVPVAIHADQLTPTWRVYSTGSNVFQTRAGCLIGAEHVNNSYECDIPIGAGICASYQTQTNSRGSASSVASQSIIAYTMSLGAENSVAYSNNSIAIPTNFTISVTTEILPVSMPKTSVDCTMYICGDSTECSNLLLQYGSFCTQLNRALTGIAVEQDKNTQEVFAQVKQIYKTPPIPDFGGFNFSQILPDPSKPSKRSPIEDLLFNKVTLADAGFIKQYGDCLGDIAARDLICAQKFNGLTVLPPLLTDEMIAQYTSALLAGTITSGWTFGAGPALQIPFPMQMAYRFNGIGVTQNVLYENQKLIANQFNSAIGKIQDSLSSTPSALGKLQNVVNQNAQALNTLVKCLSSNFGAISSVLNDILSRLDPPEAEVQIDRLITGRLQCLQTYVTQQLIRAAEIRASANLAATKMSECVLGQSKRVDFCGKGYHLMSFPQSAPHGVVFLHVTYVPAQEKNFTTAPAICHDGKAHFPREGVFVSNGTHWFVTQRNFYEPQIITTDNTFVSGNCDVVIGIVNNTVYDPLQPELDSFKEELDKYFKNHTSPDVDLGDISGILASVVNIQKEIDRLNEVAKNLNESLIDLQELGKYEQYIKWPGYIPEAPRDGQAYVRKDGEWVLLSTFLHHHHHH

SEQ ID NO: 95 - protein, 1242 aa, synthetic construct
MFVFLVLLPLVSSQCVNLITRTQSYTNSFTRGVYYPDKVFRSSVLHSTQDLFLPFFSNVTWFHAIHVSGTNGTKRFDNPALPFNDGVYFASTEKSNIIRGWIFGTTLDSKTQSLLIVNNATNVVIKVCEFQFCNDPFLDVYQKNNKSWMESEFRVYSSANNCTFEYVSQPFLMDLEGKEGNFKNLREFVFKNIDGYFKIYSKHTPINLGRDLPQGFSALEPLVDLPIGINITRFQTLLALHRSYLTPVDSSSGWTAGAAAYYVGYLQPRTFLLKYNENGTITDAVDCALDPLSETKCTLKSFTVEKGIYQTSNFRVQPTESIVRFPQITNLCPFGEVFNATKFPSVYAWERKKISNCVADYSVLYNSTFFSTFKCYGVSATKLNDLCFSNVYADSFVVKGDDVRQIAPGQTGVIADYNYKLPDDFMGCVIAWNSNNLDSKVGGNYNYRYRLFRKSKLKPFERDISTEIYQAGSKPCNGVEGFNCYFPLQSYGFQPTYGVGYQPYRVVVLSFELLHAPATVCGPKKSTNLVKNKCVNFNFNGLTGTGVLTESNKKFLPFQQFGRDIADTTDAVRDPQTLEILDITPCSFGGVSVITPGTNTSNQVAVLYQGVNCTEVPVAIHADQLTPTWRVYSTGSNVFQTRAGCLIGAEHVNNSYECDIPIGAGICASYQTQTNSRGSASSVASQSIIAYTMSLGAENSVAYSNNSIAIPTNFTISVTTEILPVSMPKTSVDCTMYICGDSTECSNLLLQYGSFCTQLNRALTGIAVEQDKNTQEVFAQVKQIYKTPPIPDFGGFNFSQILPDPSKPSKRSPIEDLLFNKVTLADAGFIKQYGDCLGDIAARDLICAQKFNGLTVLPPLLTDEMIAQYTSALLAGTITSGWTFGAGPALQIPFPMQMAYRFNGIGVTQNVLYENQKLIANQFNSAIGKIQDSLSSTPSALGKLQNVVNQNAQALNTLVKCLSSNFGAISSVLNDILSRLDPPEAEVQIDRLITGRLQCLQTYVTQQLIRAAEIRASANLAATKMSECVLGQSKRVDFCGKGYHLMSFPQSAPHGVVFLHVTYVPAQEKNFTTAPAICHDGKAHFPREGVFVSNGTHWFVTQRNFYEPQIITTDNTFVSGNCDVVIGIVNNTVYDPLQPELDSFKEELDKYFKNHTSPDVDLGDISGILASVVNIQKEIDRLNEVAKNLNESLIDLQELGKYEQYIKWPGYIPEAPRDGQAYVRKDGEWVLLSTFLHHHHHH

SEQ ID NO: 96 - protein, 1242 aa, synthetic construct
MFVFLVLLPLVSSQCVNLITRTQSYTNSFTRGVYYPDKVFRSSVLHSTQDLFLPFFSNVTWFHAIHVSGTNGTKRFDNPALPFNDGVYFASTEKSNIIRGWIFGTTLDSKTQSLLIVNNATNVVIKVCEFQFCNDPFLDVYQKNNKSWMESEFRVYSSANNCTFEYVSQPFLMDLEGKEGNFKNLREFVFKNIDGYFKIYSKHTPINLERDLPQGFSALEPLVDLPIGINITRFQTLLALHRSYLTPVDSSSGWTAGAAAYYVGYLQPRTFLLKYNENGTITDAVDCALDPLSETKCTLKSFTVEKGIYQTSNFRVQPTESIVRFPQITNLCPFGEVFNATKFPSVYAWERKKISNCVADYSVLYNSTFFSTFKCYGVSATKLNDLCFSNVYADSFVVKGDDVRQIAPGQTGVIADYNYKLPDDFMGCVIAWNSNNLDSKVGGNYNYRYRLFRKSKLKPFERDISTEIYQAGSKPCNGVEGFNCYFPLQSYGFQPTYGVGHQPYRVVVLSFELLHAPATVCGPKKSTNLVKNKCVNFNFNGLTGTGVLTESNKKFLPFQQFGRDIADTTDAVRDPQTLEILDITPCSFGGVSVITPGTNTSNQVAVLYQGVNCTEVPVAIHADQLTPTWRVYSTGSNVFQTRAGCLIGAEHVNNSYECDIPIGAGICASYQTQTNSRGSASSVASQSIIAYTMSLGAENSVAYSNNSIAIPTNFTISVTTEILPVSMPKTSVDCTMYICGDSTECSNLLLQYGSFCTQLNRALTGIAVEQDKNTQEVFAQVKQIYKTPPIPDFGGFNFSQILPDPSKPSKRSPIEDLLFNKVTLADAGFIKQYGDCLGDIAARDLICAQKFNGLTVLPPLLTDEMIAQYTSALLAGTITSGWTFGAGPALQIPFPMQMAYRFNGIGVTQNVLYENQKLIANQFNSAIGKIQDSLSSTPSALGKLQNVVNQNAQALNTLVKCLSSNFGAISSVLNDILSRLDPPEAEVQIDRLITGRLQCLQTYVTQQLIRAAEIRASANLAATKMSECVLGQSKRVDFCGKGYHLMSFPQSAPHGVVFLHVTYVPAQEKNFTTAPAICHDGKAHFPREGVFVSNGTHWFVTQRNFYEPQIITTDNTFVSGNCDVVIGIVNNTVYDPLQPELDSFKEELDKYFKNHTSPDVDLGDISGILASVVNIQKEIDRLNEVAKNLNESLIDLQELGKYEQYIKWPGYIPEAPRDGQAYVRKDGEWVLLSTFLHHHHHH

SEQ ID NO: 97 - protein, 1242 aa, synthetic construct
MFVFLVLLPLVSSQCVNLITRTQSYTNSFTRGVYYPDKVFRSSVLHSTQDLFLPFFSNVTWFHAIHVSGTNGTKRFDNPALPFNDGVYFASTEKSNIIRGWIFGTTLDSKTQSLLIVNNATNVVIKVCEFQFCNDPFLDVYQKNNKSWMESEFRVYSSANNCTFEYVSQPFLMDLEGKEGNFKNLREFVFKNIDGYFKIYSKHTPINLERDLPQGFSALEPLVDLPIGINITRFQTLLALHRSYLTPVDSSSGWTAGAAAYYVGYLQPRTFLLKYNENGTITDAVDCALDPLSETKCTLKSFTVEKGIYQTSNFRVQPTESIVRFPQITNLCPFGEVFNATKFPSVYAWERKNISNCVADYSVLYNSTFFSTFKCYGVSATKLNDLCFSNVYADSFVVKGDDVRQIAPGQTGVIADYNYKLPDDFMGCVIAWNSNNLDSKVGGNYNYRYRLFRKSKLKPFERDISTEIYQAGSKPCNGVEGFNCYFPLQSYGFQPTYGVGYQPYRVVVLSFELLHAPATVCGPKKSTNLVKNKCVNFNFNGLTGTGVLTESNKKFLPFQQFGRDIADTTDAVRDPQTLEILDITPCSFGGVSVITPGTNTSNQVAVLYQGVNCTEVPVAIHADQLTPTWRVYSTGSNVFQTRAGCLIGAEHVNNSYECDIPIGAGICASYQTQTNSRGSASSVASQSIIAYTMSLGAENSVAYSNNSIAIPTNFTISVTTEILPVSMPKTSVDCTMYICGDSTECSNLLLQYGSFCTQLNRALTGIAVEQDKNTQEVFAQVKQIYKTPPIPDFGGFNFSQILPDPSKPSKRSPIEDLLFNKVTLADAGFIKQYGDCLGDIAARDLICAQKFNGLTVLPPLLTDEMIAQYTSALLAGTITSGWTFGAGPALQIPFPMQMAYRFNGIGVTQNVLYENQKLIANQFNSAIGKIQDSLSSTPSALGKLQNVVNQNAQALNTLVKCLSSNFGAISSVLNDILSRLDPPEAEVQIDRLITGRLQCLQTYVTQQLIRAAEIRASANLAATKMSECVLGQSKRVDFCGKGYHLMSFPQSAPHGVVFLHVTYVPAQEKNFTTAPAICHDGKAHFPREGVFVSNGTHWFVTQRNFYEPQIITTDNTFVSGNCDVVIGIVNNTVYDPLQPELDSFKEELDKYFKNHTSPDVDLGDISGILASVVNIQKEIDRLNEVAKNLNESLIDLQELGKYEQYIKWPGYIPEAPRDGQAYVRKDGEWVLLSTFLHHHHHH

SEQ ID NO: 98 - protein, 1242 aa, synthetic construct
MFVFLVLLPLVSSQCVNLITRTQSYTNSFTRGVYYPDKVFRSSVLHSTQDLFLPFFSNVTWFHAIHNSTTQGTKRFDNPALPFNDGVYFASTEKSNIIRGWIFGTTLDSKTQSLLIVNNATNVVIKVCEFQFCNDPFLDVYQKNNKSWMESEFRVYSSANNCTFEYVSQPFLMDLEGKEGNFKNLREFVFKNIDGYFKIYSKHTPINLERDLPQGFSALEPLVDLPIGINITRFQTLLALHRSYLTPVDSSSGWTAGAAAYYVGYLQPRTFLLKYNENGTITDAVDCALDPLSETKCTLKSFTVEKGIYQTSNFRVQPTESIVRFPQITNLCPFGEVFNATKFPSVYAWERKKISNCVADYSVLYNSTFFSTFKCYGVSATKLNDLCFSNVYADSFVVKGDDVRQIAPGQTGVIADYNYKLPDDFMGCVIAWNSNNLDSKVGGNYNYRYRLFRKSKLKPFERDISTEIYQAGSKPCNGVEGFNCYFPLQSYGFQPTYGVGYQPYRVVVLSFELLHAPATVCGPKKSTNLVKNKCVNFNFNGLTGTGVLTESNKKFLPFQQFGRDIADTTDAVRDPQTLEILDITPCSFGGVSVITPGTNTSNQVAVLYQGVNCTEVPVAIHADQLTPTWRVYSTGSNVFQTRAGCLIGAEHVNNSYECDIPIGAGICASYQTQTNSRGSASSVASQSIIAYTMSLGAENSVAYSNNSIAIPTNFTISVTTEILPVSMPKTSVDCTMYICGDSTECSNLLLQYGSFCTQLNRALTGIAVEQDKNTQEVFAQVKQIYKTPPIPDFGGFNFSQILPDPSKPSKRSPIEDLLFNKVTLADAGFIKQYGDCLGDIAARDLICAQKFNGLTVLPPLLTDEMIAQYTSALLAGTITSGWTFGAGPALQIPFPMQMAYRFNGIGVTQNVLYENQKLIANQFNSAIGKIQDSLSSTPSALGKLQNVVNQNAQALNTLVKCLSSNFGAISSVLNDILSRLDPPEAEVQIDRLITGRLQCLQTYVTQQLIRAAEIRASANLAATKMSECVLGQSKRVDFCGKGYHLMSFPQSAPHGVVFLHVTYVPAQEKNFTTAPAICHDGKAHFPREGVFVSNGTHWFVTQRNFYEPQIITTDNTFVSGNCDVVIGIVNNTVYDPLQPELDSFKEELDKYFKNHTSPDVDLGDISGILASVVNIQKEIDRLNEVAKNLNESLIDLQELGKYEQYIKWPGYIPEAPRDGQAYVRKDGEWVLLSTFLHHHHHH

SEQ ID NO: 99 - protein, 1242 aa, synthetic construct
MFVFLVLLPLVSSQCVNLITRTQSYTNSFTRGVYYPDKVFRSSVLHSTQDLFLPFFSNVTWFHAIHVSGTNGTKRFDNPALPFNDGVYFASTEKSNIIRGWIFGTTLDSKTQSLLIVNNATNVVIKVCEFQFCNDPFLDVYQKNNKSWMESEFRVYSSANNCTFEYVSQPFLMDLEGKEGNFKNLREFVFKNIDGYFKIYSKHTPINLERDLPQGFSALEPLVDLPIGIVITRFQTLLALHRSYLTPVDSSSGWTAGAAAYYVGYLQPRTFLLKYNENGTITDAVDCALDPLSETKCTLKSFTVEKGIYQTSNFRVQPTESIVRFPQITNLCPFGEVFNATKFPSVYAWERKKISNCVADYSVLYNSTFFSTFKCYGVSATKLNDLCFSNVYADSFVVKGDDVRQIAPGQTGVIADYNYKLPDDFMGCVIAWNSNNLDSKVGGNYNYRYRLFRKSKLKPFERDISTEIYQAGSKPCNGVEGFNCYFPLQSYGFQPTYGVGYQPYRVVVLSFELLHAPATVCGPKKSTNLVKNKCVNFNFNGLTGTGVLTESNKKFLPFQQFGRDIADTTDAVRDPQTLEILDITPCSFGGVSVITPGTNTSNQVAVLYQGVNCTEVPVAIHADQLTPTWRVYSTGSNVFQTRAGCLIGAEHVNNSYECDIPIGAGICASYQTQTNSRGSASSVASQSIIAYTMSLGAENSVAYSNNSIAIPTNFTISVTTEILPVSMPKTSVDCTMYICGDSTECSNLLLQYGSFCTQLNRALTGIAVEQDKNTQEVFAQVKQIYKTPPIPDFGGFNFSQILPDPSKPSKRSPIEDLLFNKVTLADAGFIKQYGDCLGDIAARDLICAQKFNGLTVLPPLLTDEMIAQYTSALLAGTITSGWTFGAGPALQIPFPMQMAYRFNGIGVTQNVLYENQKLIANQFNSAIGKIQDSLSSTPSALGKLQNVVNQNAQALNTLVKCLSSNFGAISSVLNDILSRLDPPEAEVQIDRLITGRLQCLQTYVTQQLIRAAEIRASANLAATKMSECVLGQSKRVDFCGKGYHLMSFPQSAPHGVVFLHVTYVPAQEKNFTTAPAICHDGKAHFPREGVFVSNGTHWFVTQRNFYEPQIITTDNTFVSGNCDVVIGIVNNTVYDPLQPELDSFKEELDKYFKNHTSPDVDLGDISGILASVVNIQKEIDRLNEVAKNLNESLIDLQELGKYEQYIKWPGYIPEAPRDGQAYVRKDGEWVLLSTFLHHHHHH

SEQ ID NO: 100 - protein, 1242 aa, synthetic construct
MFVFLVLLPLVSSQCVNLITRTQSYTNSFTRGVYYPDKVFRSSVLHSTQDLFLPFFSNVTWFHAIHVSGTNGTKRFDNPALPFNDGVYFASTEKSNIIRGWIFGTTLDSKTQSLLIVNNATNVVIKVCEFQFCNDPFLDVYQKNNKSWMESEFRVYSSANNCTFEYVSQPFLMDLEGKEGNFKNLREFVFKNIDGYFKIYSKHTPINLERDLPQGFSALEPLVDLPIGINITRFQTLLALHRSYLTPVDSSSGWTAGAAAYYVGYLQPRTFLLKYNENGTITDAVDCALDPLSETKCTLKSFTVEKGIYQTSNFRVQPTESIVRFPQITNLCPFGEVFNATKFPSVYAWERKKISNCVADYSVLYNSTFFSTFKCYGVVATKLNDLCFSNVYADSFVVKGDDVRQIAPGQTGVIADYNYKLPDDFMGCVIAWNSNNLDSKVGGNYNYRYRLFRKSKLKPFERDISTEIYQAGSKPCNGVEGFNCYFPLQSYGFQPTYGVGYQPYRVVVLSFELLHAPATVCGPKKSTNLVKNKCVNFNFNGLTGTGVLTESNKKFLPFQQFGRDIADTTDAVRDPQTLEILDITPCSFGGVSVITPGTNTSNQVAVLYQGVNCTEVPVAIHADQLTPTWRVYSTGSNVFQTRAGCLIGAEHVNNSYECDIPIGAGICASYQTQTNSRGSASSVASQSIIAYTMSLGAENSVAYSNNSIAIPTNFTISVTTEILPVSMPKTSVDCTMYICGDSTECSNLLLQYGSFCTQLNRALTGIAVEQDKNTQEVFAQVKQIYKTPPIPDFGGFNFSQILPDPSKPSKRSPIEDLLFNKVTLADAGFIKQYGDCLGDIAARDLICAQKFNGLTVLPPLLTDEMIAQYTSALLAGTITSGWTFGAGPALQIPFPMQMAYRFNGIGVTQNVLYENQKLIANQFNSAIGKIQDSLSSTPSALGKLQNVVNQNAQALNTLVKCLSSNFGAISSVLNDILSRLDPPEAEVQIDRLITGRLQCLQTYVTQQLIRAAEIRASANLAATKMSECVLGQSKRVDFCGKGYHLMSFPQSAPHGVVFLHVTYVPAQEKNFTTAPAICHDGKAHFPREGVFVSNGTHWFVTQRNFYEPQIITTDNTFVSGNCDVVIGIVNNTVYDPLQPELDSFKEELDKYFKNHTSPDVDLGDISGILASVVNIQKEIDRLNEVAKNLNESLIDLQELGKYEQYIKWPGYIPEAPRDGQAYVRKDGEWVLLSTFLHHHHHH

SEQ ID NO: 101 - protein, 1242 aa, synthetic construct
MFVFLVLLPLVSSQCVNLITRTQSYTNSFTRGVYYPDKVFRSSVLHSTQDLFLPFFSNVTWFHAIHVSGTNGTKRFDNPALPFNDGVYFASTEKSNIIRGWIFGTTLDSKTQSLLIVNNATNVVIKVCEFQFCNDPFLDVYQKNNKSWMESEFRVYSSANNCTFEYVSQPFLMDLEGKNGTFKNLREFVFKNIDGYFKIYSKHTPINLERDLPQGFSALEPLVDLPIGINITRFQTLLALHRSYLTPVDNSTGWTAGAAAYYVGYLQPRTFLLKYNENGTITDAVDCALDPLSETKCTLKSFTVEKGIYQTSNFRVQPTESIVRFPQITNLCPFGEVFNATKFPSVYAWERKKISNCVADYSVLYNSTFFSTFKCYGVSATKLNDLCFSNVYADSFVVKGDDVRQIAPGQTGVIADYNYKLPDDFMGCVIAWNSNNLDSKVGGNYNYRYRLFRKSKLKPFERDISTEIYQAGSKPCNGVEGFNCYFPLQSYGFQPTYGVGYQPYRVVVLSFELLHAPATVCGPKKSTNLVKNKCVNFNFNGLTGTGVLTESNKKFLPFQQFGRDIADTTDAVRDPQTLEILDITPCSFGGVSVITPGTNTSNQVAVLYQGVNCTEVPVAIHADQLTPTWRVYSTGSNVFQTRAGCLIGAEHVNNSYECDIPIGAGICASYQTQTNSRGSASSVASQSIIAYTMSLGAENSVAYSNNSIAIPTNFTISVTTEILPVSMPKTSVDCTMYICGDSTECSNLLLQYGSFCTQLNRALTGIAVEQDKNTQEVFAQVKQIYKTPPIPDFGGFNFSQILPDPSKPSKRSPIEDLLFNKVTLADAGFIKQYGDCLGDIAARDLICAQKFNGLTVLPPLLTDEMIAQYTSALLAGTITSGWTFGAGPALQIPFPMQMAYRFNGIGVTQNVLYENQKLIANQFNSAIGKIQDSLSSTPSALGKLQNVVNQNAQALNTLVKCLSSNFGAISSVLNDILSRLDPPEAEVQIDRLITGRLQCLQTYVTQQLIRAAEIRASANLAATKMSECVLGQSKRVDFCGKGYHLMSFPQSAPHGVVFLHVTYVPAQEKNFTTAPAICHDGKAHFPREGVFVSNGTHWFVTQRNFYEPQIITTDNTFVSGNCDVVIGIVNNTVYDPLQPELDSFKEELDKYFKNHTSPDVDLGDISGILASVVNIQKEIDRLNEVAKNLNESLIDLQELGKYEQYIKWPGYIPEAPRDGQAYVRKDGEWVLLSTFLHHHHHH

SEQ ID NO: 102 - protein, 1242 aa, synthetic construct
MFVFLVLLPLVSSQCVNLITRTQSYTNSFTRGVYYPDKVFRSSVLHSTQDLFLPFFSNVTWFHAIHVSGTNGTKRFDNPALPFNDGVYFASTEKSNIIRGWIFGTTLDSKTQSLLIVNNATNVVIKVCEFQFCNDPFLDVYQKNNKSWMESEFRVYSSANNCTFEYVSQPFLMDLEGKEGNFKNLREFVFKNIDGYFKIYSKHTPINLERDLPQGFSALEPLVDLPIGINITRFQTLLALHRSYLTPVDSSSGWTAGAAAYYVGYLQPRTFLLKYNENGTITDAVDCALDPLSETKCTLKSFTVEKGIYQTSNFRVQPTESIVRFPQITNLCPFGEVFNATKFPSVYAWERKKISNCVADYSVLYNSTFFSTFKCYGVSATKLNDLCFSNVYADSFVVKGDDVRQIAPGQTGVIADYNYKLPDDFMGCVIAWNSNNLDSKVGGNYNYRYRLFRKSKLGPFERDISTEIYQAGSKPCNGVEGFNCYFPLQSYGFQPTYGVGYQPYRVVVLSFELLHAPATVCGPKKSTNLVKNKCVNFNFNGLTGTGVLTESNKKFLPFQQFGRDIADTTDAVRDPQTLEILDITPCSFGGVSVITPGTNTSNQVAVLYQGVNCTEVPVAIHADQLTPTWRVYSTGSNVFQTRAGCLIGAEHVNNSYECDIPIGAGICASYQTQTNSRGSASSVASQSIIAYTMSLGAENSVAYSNNSIAIPTNFTISVTTEILPVSMPKTSVDCTMYICGDSTECSNLLLQYGSFCTQLNRALTGIAVEQDKNTQEVFAQVKQIYKTPPIPDFGGFNFSQILPDPSKPSKRSPIEDLLFNKVTLADAGFIKQYGDCLGDIAARDLICAQKFNGLTVLPPLLTDEMIAQYTSALLAGTITSGWTFGAGPALQIPFPMQMAYRFNGIGVTQNVLYENQKLIANQFNSAIGKIQDSLSSTPSALGKLQNVVNQNAQALNTLVKCLSSNFGAISSVLNDILSRLDPPEAEVQIDRLITGRLQCLQTYVTQQLIRAAEIRASANLAATKMSECVLGQSKRVDFCGKGYHLMSFPQSAPHGVVFLHVTYVPAQEKNFTTAPAICHDGKAHFPREGVFVSNGTHWFVTQRNFYEPQIITTDNTFVSGNCDVVIGIVNNTVYDPLQPELDSFKEELDKYFKNHTSPDVDLGDISGILASVVNIQKEIDRLNEVAKNLNESLIDLQELGKYEQYIKWPGYIPEAPRDGQAYVRKDGEWVLLSTFLHHHHHH

SEQ ID NO: 103 - protein, 1242 aa, synthetic construct
MFVFLVLLPLVSSQCVNLITRTQSYTNSFTRGVYYPDKVFRSSVLHSTQDLFLPFFSNVTWFHAIHVSGTNGTKRFDNPALPFNDGVYFASTEKSNIIRGWIFGTTLDSKTQSLLIVNNATNVVIKVCEFQFCNDPFLDVYQKNNKSWMESEFRVYSSANNCTFEYVSQPFLMDLEGKEGNFKNLREFVFKNIDGYFKIYSKHTPINLERDLPQGFSALEPLVDLPIGINITRFQTLLALHRSYLTPVDSSSGWTAGAAAYYVGYLQPRTFLLKYNENGTITDAVDCALDPLSETKCTLKSFTVEKGIYQTSNFRVQPTESIVRFPQITNLCPFGEVFNATKFPSVYAWERKNISNCVADYSVLYNSTFFSTFKCYGVNATKLNDLCFSNVYADSFVVKGDDVRQIAPGQTGVIADYNYKLPDDFMGCVIAWNSNNLDSKVGGNYNYRYRLFRKSKLKPFERDNSTEIYQAGSKPCNGVEGFNCYFPLQSYGFQPTYGVGYQPYRVVVLSFELLHAPATVCGPKKSTNLVKNKCVNFNFNGLTGTGVLTESNKKFLPFQQFGRDIADTTDAVRDPQTLEILDITPCSFGGVSVITPGTNTSNQVAVLYQGVNCTEVPVAIHADQLTPTWRVYSTGSNVFQTRAGCLIGAEHVNNSYECDIPIGAGICASYQTQTNSRGSASSVASQSIIAYTMSLGAENSVAYSNNSIAIPTNFTISVTTEILPVSMPKTSVDCTMYICGDSTECSNLLLQYGSFCTQLNRALTGIAVEQDKNTQEVFAQVKQIYKTPPIPDFGGFNFSQILPDPSKPSKRSPIEDLLFNKVTLADAGFIKQYGDCLGDIAARDLICAQKFNGLTVLPPLLTDEMIAQYTSALLAGTITSGWTFGAGPALQIPFPMQMAYRFNGIGVTQNVLYENQKLIANQFNSAIGKIQDSLSSTPSALGKLQNVVNQNAQALNTLVKCLSSNFGAISSVLNDILSRLDPPEAEVQIDRLITGRLQCLQTYVTQQLIRAAEIRASANLAATKMSECVLGQSKRVDFCGKGYHLMSFPQSAPHGVVFLHVTYVPAQEKNFTTAPAICHDGKAHFPREGVFVSNGTHWFVTQRNFYEPQIITTDNTFVSGNCDVVIGIVNNTVYDPLQPELDSFKEELDKYFKNHTSPDVDLGDISGILASVVNIQKEIDRLNEVAKNLNESLIDLQELGKYEQYIKWPGYIPEAPRDGQAYVRKDGEWVLLSTFLHHHHHH

SEQ ID NO: 104 - protein, 1242 aa, synthetic construct
MFVFLVLLPLVSSQCVNLITRTQSYTNSFTRGVYYPDKVFRSSVLHSTQDLFLPFFSNVTWFHAIHVSGTNGTKRFDNPALPFNDGVYFASTEKSNIIRGWIFGTTLDSKTQSLLIVNNATNVVIKVCEFQFCNDPFLDVYQKNNKSWMESEFRVYSSANNCTFEYVSQPFLMDLEGKEGNFKNLREFVFKNIDGYFKIYSKHTPINLERDLPQGFSALEPLVDLPIGINITRFQTLLALHRSYLTPVDSSSGWTAGAAAYYVGYLQPRTFLLKYNENGTITDAVDCALDPLSETKCTLKSFTVEKGIYQTSNFRVQPTESIVRFPQITNLCPFGEVFNATKFPSVYAWERKKISNCVADYSVLYNSTFFSTFKCYGVSATKLNDLCFSNVYADSFVVKGDDVRQIAPGQTGVIADYNYKLPDDFMGCVIAWNSNNLDSKVGGNYNYRYRLFRKSKLKPFERDISTEIYQAGSKPCNGVEGFNCYFPLQNYTFQPTYGVGYQPYRVVVLSFELLHAPATVCGPKKSTNLVKNKCVNFNFNGLTGTGVLTESNKKFLPFQQFGRDIADTTDAVRDPQTLEILDITPCSFGGVSVITPGTNTSNQVAVLYQGVNCTEVPVAIHADQLTPTWRVYSTGSNVFQTRAGCLIGAEHVNNSYECDIPIGAGICASYQTQTNSRGSASSVASQSIIAYTMSLGAENSVAYSNNSIAIPTNFTISVTTEILPVSMPKTSVDCTMYICGDSTECSNLLLQYGSFCTQLNRALTGIAVEQDKNTQEVFAQVKQIYKTPPIPDFGGFNFSQILPDPSKPSKRSPIEDLLFNKVTLADAGFIKQYGDCLGDIAARDLICAQKFNGLTVLPPLLTDEMIAQYTSALLAGTITSGWTFGAGPALQIPFPMQMAYRFNGIGVTQNVLYENQKLIANQFNSAIGKIQDSLSSTPSALGKLQNVVNQNAQALNTLVKCLSSNFGAISSVLNDILSRLDPPEAEVQIDRLITGRLQCLQTYVTQQLIRAAEIRASANLAATKMSECVLGQSKRVDFCGKGYHLMSFPQSAPHGVVFLHVTYVPAQEKNFTTAPAICHDGKAHFPREGVFVSNGTHWFVTQRNFYEPQIITTDNTFVSGNCDVVIGIVNNTVYDPLQPELDSFKEELDKYFKNHTSPDVDLGDISGILASVVNIQKEIDRLNEVAKNLNESLIDLQELGKYEQYIKWPGYIPEAPRDGQAYVRKDGEWVLLSTFLHHHHHH

SEQ ID NO: 105 - protein, 1242 aa, synthetic construct
MFVFLVLLPLVSSQCVNLITRTQSYTNSFTRGVYYPDKVFRSSVLHSTQDLFLPFFSNVTWFHAIHVSGTNGTKRFDNPALPFNDGVYFASTEKSNIIRGWIFGTTLDSKTQSLLIVNNATNVVIKVCEFQFCNDPFLDVYQKNNKSWMESEFRVYSSANNCTFEYVSQPFLMDLEGKEGNFKNLREFVFKNIDGYFKIYSKHTPINLERDLPQGFSALEPLVDLPIGIWITRFQTLLALHRSYLTPVDSSSGWTAGAAAYYVGYLQPRTFLLKYNENGTITDAVDCALDPLSETKCTLKSFTVEKGIYQTSNFRVQPTESIVRFPQITNLCPFGEVFNATKFPSVYAWERKKISNCVADYSVLYNSTFFSTFKCYGVSATKLNDLCFSNVYADSFVVKGDDVRQIAPGQTGVIADYNYKLPDDFMGCVIAWNSNNLDSKVGGNYNYRYRLFRKSKLKPFERDISTEIYQAGSKPCNGVEGFNCYFPLQSYGFQPTYGVGYQPYRVVVLSFELLHAPATVCGPKKSTNLVKNKCVNFNFNGLTGTGVLTESNKKFLPFQQFGRDIADTTDAVRDPQTLEILDITPCSFGGVSVITPGTNTSNQVAVLYQGVNCTEVPVAIHADQLTPTWRVYSTGSNVFQTRAGCLIGAEHVNNSYECDIPIGAGICASYQTQTNSRGSASSVASQSIIAYTMSLGAENSVAYSNNSIAIPTNFTISVTTEILPVSMPKTSVDCTMYICGDSTECSNLLLQYGSFCTQLNRALTGIAVEQDKNTQEVFAQVKQIYKTPPIPDFGGFNFSQILPDPSKPSKRSPIEDLLFNKVTLADAGFIKQYGDCLGDIAARDLICAQKFNGLTVLPPLLTDEMIAQYTSALLAGTITSGWTFGAGPALQIPFPMQMAYRFNGIGVTQNVLYENQKLIANQFNSAIGKIQDSLSSTPSALGKLQNVVNQNAQALNTLVKCLSSNFGAISSVLNDILSRLDPPEAEVQIDRLITGRLQCLQTYVTQQLIRAAEIRASANLAATKMSECVLGQSKRVDFCGKGYHLMSFPQSAPHGVVFLHVTYVPAQEKNFTTAPAICHDGKAHFPREGVFVSNGTHWFVTQRNFYEPQIITTDNTFVSGNCDVVIGIVNNTVYDPLQPELDSFKEELDKYFKNHTSPDVDLGDISGILASVVNIQKEIDRLNEVAKNLNESLIDLQELGKYEQYIKWPGYIPEAPRDGQAYVRKDGEWVLLSTFLHHHHHH

SEQ ID NO: 106 - protein, 1242 aa, synthetic construct
MFVFLVLLPLVSSQCVNLITRTQSYTNSFTRGVYYPDKVFRSSVLHSTQDLFLPFFSNVTWFHAIHVSGTNGTKRFDNPALPFNDGVYFASTEKSNIIRGWIFGTTLDSKTQSLLIVNNATNVVIKVCEFQFCNDPFLDVYQKNNKSWMESEFRVYSSANNCTFEYVSQPFLMDLEGKEGNFKNLREFVFKNIDGYFKIYSKHTPINLERDLPQGFSALEPLVDLPIGINITRFQTLLALHRSYLTPVDSSSGWTAGAAAYYVGYLQPRTFLLKYNENGTITDAVDCALDPLSETKCTLKSFTVEKGIYQTSNFRVQPTESIVRFPQITNLCPFGEVFNATKFPSVYAWERKKISNCVADYSVLYNSTFFSTFKCYGVSATKLNDLCFSNVYADSFVVKGDDVRQIAPGQTGVIADYNYKLPDDFMGCVIAWNSNNLDSKVGGNYNYRYRLFRKKKLKPFERDISTEIYQAGSKPCNGVEGFNCYFPLQSYGFQPTYGVGYQPYRVVVLSFELLHAPATVCGPKKSTNLVKNKCVNFNFNGLTGTGVLTESNKKFLPFQQFGRDIADTTDAVRDPQTLEILDITPCSFGGVSVITPGTNTSNQVAVLYQGVNCTEVPVAIHADQLTPTWRVYSTGSNVFQTRAGCLIGAEHVNNSYECDIPIGAGICASYQTQTNSRGSASSVASQSIIAYTMSLGAENSVAYSNNSIAIPTNFTISVTTEILPVSMPKTSVDCTMYICGDSTECSNLLLQYGSFCTQLNRALTGIAVEQDKNTQEVFAQVKQIYKTPPIPDFGGFNFSQILPDPSKPSKRSPIEDLLFNKVTLADAGFIKQYGDCLGDIAARDLICAQKFNGLTVLPPLLTDEMIAQYTSALLAGTITSGWTFGAGPALQIPFPMQMAYRFNGIGVTQNVLYENQKLIANQFNSAIGKIQDSLSSTPSALGKLQNVVNQNAQALNTLVKCLSSNFGAISSVLNDILSRLDPPEAEVQIDRLITGRLQCLQTYVTQQLIRAAEIRASANLAATKMSECVLGQSKRVDFCGKGYHLMSFPQSAPHGVVFLHVTYVPAQEKNFTTAPAICHDGKAHFPREGVFVSNGTHWFVTQRNFYEPQIITTDNTFVSGNCDVVIGIVNNTVYDPLQPELDSFKEELDKYFKNHTSPDVDLGDISGILASVVNIQKEIDRLNEVAKNLNESLIDLQELGKYEQYIKWPGYIPEAPRDGQAYVRKDGEWVLLSTFLHHHHHH

SEQ ID NO: 107 - protein, 1242 aa, synthetic construct
MFVFLVLLPLVSSQCVNLITRTQSYTNSFTRGVYYPDKVFRSSVLHSTQDLFLPFFSNVTWFHAIHVSGTNGTKRFDNPALPFNDGVYFASTEKSNIIRGWIFGTTLDSKTQSLLIVNNATNVVIKVCEFQFCNDPFLDVYQKNNKSWMESEFRVYSSANNCTFEYVSQPFLMDLEGKEGNFKNLREFVFKNIDGYFKIYSKHTPINLERDLPQGFSALEPLVDLPIGINITRFQTLLALHRSYLTPVDSSSGWTAGAAAYYVGYLQPRTFLLKYNENGTITDAVDCALDPLSETKCTLKSFTVEKGIYQTSNFRVQPTESIVRFPQITNLCPFGEVFNATKFPSVYAWERKKISNCVADYSVLYNSTFFSTFKCYGVSATKLNDLCFSNVYADSFVVKGDDVRQIAPGQTGVIADYNYKLPDDFMGCVIAWNSNNLDSKVGGNYNYRYRLFRKSKLQPFERDISTEIYQAGSKPCNGVEGFNCYFPLQSYGFQPTYGVGYQPYRVVVLSFELLHAPATVCGPKKSTNLVKNKCVNFNFNGLTGTGVLTESNKKFLPFQQFGRDIADTTDAVRDPQTLEILDITPCSFGGVSVITPGTNTSNQVAVLYQGVNCTEVPVAIHADQLTPTWRVYSTGSNVFQTRAGCLIGAEHVNNSYECDIPIGAGICASYQTQTNSRGSASSVASQSIIAYTMSLGAENSVAYSNNSIAIPTNFTISVTTEILPVSMPKTSVDCTMYICGDSTECSNLLLQYGSFCTQLNRALTGIAVEQDKNTQEVFAQVKQIYKTPPIPDFGGFNFSQILPDPSKPSKRSPIEDLLFNKVTLADAGFIKQYGDCLGDIAARDLICAQKFNGLTVLPPLLTDEMIAQYTSALLAGTITSGWTFGAGPALQIPFPMQMAYRFNGIGVTQNVLYENQKLIANQFNSAIGKIQDSLSSTPSALGKLQNVVNQNAQALNTLVKCLSSNFGAISSVLNDILSRLDPPEAEVQIDRLITGRLQCLQTYVTQQLIRAAEIRASANLAATKMSECVLGQSKRVDFCGKGYHLMSFPQSAPHGVVFLHVTYVPAQEKNFTTAPAICHDGKAHFPREGVFVSNGTHWFVTQRNFYEPQIITTDNTFVSGNCDVVIGIVNNTVYDPLQPELDSFKEELDKYFKNHTSPDVDLGDISGILASVVNIQKEIDRLNEVAKNLNESLIDLQELGKYEQYIKWPGYIPEAPRDGQAYVRKDGEWVLLSTFLHHHHHH

SEQ ID NO: 108 - protein, 1242 aa, synthetic construct
MFVFLVLLPLVSSQCVNLITRTQSYTNSFTRGVYYPDKVFRSSVLHSTQDLFLPFFSNVTWFHAIHVSGTNGTKRFDNPALPFNDGVYFASTEKSNIIRGWIFGTTLDSKTQSLLIVNNATNVVIKVCEFQFCNDPFLDVYQKNNKSWMESEFRVYSSANNCTFEYVSQPFLMDLEGKEGNFKNLREFVFKNIDGYFKIYSKHTPINLERDLPQGFSALEPLVDLPIGINITRFQTLLALHRSYLTPVDSSSGWTAGAAAYYVGYLQPRTFLLKYNENGTITDAVDCALDPLSETKCTLKSFTVEKGIYQTSNFRVQPTESIVRFPQITNLCPFGEVFNATKFPSVYAWERKKISNCVADYSVLYNSTFFSTFKCYGVSATKLNDLCFSNVYADSFVVKGDDVRQIAPGQTGVIADYNYKLPDDFMGCVIAWNSNNLDSKVGGNYNYRYRLFRKSKLKPFERDISTEIYQAGSKPCNGVEGFNCYFPLQSYGFQPTYGVGYQPYRVVVLSFELNHTPATVCGPKKSTNLVKNKCVNFNFNGLTGTGVLTESNKKFLPFQQFGRDIADTTDAVRDPQTLEILDITPCSFGGVSVITPGTNTSNQVAVLYQGVNCTEVPVAIHADQLTPTWRVYSTGSNVFQTRAGCLIGAEHVNNSYECDIPIGAGICASYQTQTNSRGSASSVASQSIIAYTMSLGAENSVAYSNNSIAIPTNFTISVTTEILPVSMPKTSVDCTMYICGDSTECSNLLLQYGSFCTQLNRALTGIAVEQDKNTQEVFAQVKQIYKTPPIPDFGGFNFSQILPDPSKPSKRSPIEDLLFNKVTLADAGFIKQYGDCLGDIAARDLICAQKFNGLTVLPPLLTDEMIAQYTSALLAGTITSGWTFGAGPALQIPFPMQMAYRFNGIGVTQNVLYENQKLIANQFNSAIGKIQDSLSSTPSALGKLQNVVNQNAQALNTLVKCLSSNFGAISSVLNDILSRLDPPEAEVQIDRLITGRLQCLQTYVTQQLIRAAEIRASANLAATKMSECVLGQSKRVDFCGKGYHLMSFPQSAPHGVVFLHVTYVPAQEKNFTTAPAICHDGKAHFPREGVFVSNGTHWFVTQRNFYEPQIITTDNTFVSGNCDVVIGIVNNTVYDPLQPELDSFKEELDKYFKNHTSPDVDLGDISGILASVVNIQKEIDRLNEVAKNLNESLIDLQELGKYEQYIKWPGYIPEAPRDGQAYVRKDGEWVLLSTFLHHHHHH

SEQ ID NO: 109 - protein, 1242 aa, synthetic construct
MFVFLVLLPLVSSQCVNLITRTQSYTNSFTRGVYYPDKVFRSSVLHSTQDLFLPFFSNVTWFHAIHVSGTNGTKRFDNPALPFNDGVYFASTEKSNIIRGWIFGTTLDSKTQSLLIVNNATNVVIKVCEFQFCNDPFLDVYQKNNKSWMESEFRVYSSANNCTFEYVSQPFLMDLEGKEGNFKNLREFVFKNIDGYFKIYSKHTPINLERDLPQGFSALEPLVDLPIGINITRFQTLLALHRSYLTPVDSSSGWTAGAAAYYVGYLQPRTFLLKYNENGTITDAVDCALDPLSETKCTLKSFTVEKGIYQTSNFRVQPTESIVRFPQITNLCPFGEVFNATKFPSVYAWERKKISNCVADYSVLYNSTFFSTFKCYGVSATKLNDLCFSNVYADSFVVKGDDVRQIAPGQTGVIADYNYKLPDDFMGCVIAWNSNKLDSKVGGNYNYRYRLFRKSKLKPFERDISTEIYQAGNKPCNGVEGFNCYFPLQSYGFRPTYGVGYQPYRVVVLSFELLHAPATVCGPKKSTNLVKNKCVNFNFNGLTGTGVLTESNKKFLPFQQFGRDIADTTDAVRDPQTLEILDITPCSFGGVSVITPGTNTSNQVAVLYQGVNCTEVPVAIHADQLTPTWRVYSTGSNVFQTRAGCLIGAEHVNNSYECDIPIGAGICASYQTQTNSRGSASSVASQSIIAYTMSLGAENSVAYSNNSIAIPTNFTISVTTEILPVSMPKTSVDCTMYICGDSTECSNLLLQYGSFCTQLNRALTGIAVEQDKNTQEVFAQVKQIYKTPPIPDFGGFNFSQILPDPSKPSKRSPIEDLLFNKVTLADAGFIKQYGDCLGDIAARDLICAQKFNGLTVLPPLLTDEMIAQYTSALLAGTITSGWTFGAGPALQIPFPMQMAYRFNGIGVTQNVLYENQKLIANQFNSAIGKIQDSLSSTPSALGKLQNVVNQNAQALNTLVKCLSSNFGAISSVLNDILSRLDPPEAEVQIDRLITGRLQCLQTYVTQQLIRAAEIRASANLAATKMSECVLGQSKRVDFCGKGYHLMSFPQSAPHGVVFLHVTYVPAQEKNFTTAPAICHDGKAHFPREGVFVSNGTHWFVTQRNFYEPQIITTDNTFVSGNCDVVIGIVNNTVYDPLQPELDSFKEELDKYFKNHTSPDVDLGDISGILASVVNIQKEIDRLNEVAKNLNESLIDLQELGKYEQYIKWPGYIPEAPRDGQAYVRKDGEWVLLSTFLHHHHHH

SEQ ID NO: 110 - protein, 1242 aa, synthetic construct
MFVFLVLLPLVSSQCVNLITRTQSYTNSFTRGVYYPDKVFRSSVLHSTQDLFLPFFSNVTWFHAIHVSGTNGTKRFDNPALPFNDGVYFASTEKSNIIRGWIFGTTLDSKTQSLLIVNNATNVVIKVCEFQFCNDPFLDVYQKNNKSWMESEFRVYSSANNCTFEYVSQPFLMDLEGKEGNFKNLREFVFKNIDGYFKIYSKHTPINLERDLPQGFSALEPLVDLPIGINITRFQTLLALHRSYLTPVDSSSGWTAGAAAYYVGYLQPRTFLLKYNENGTITDAVDCALDPLSETKCTLKSFTVEKGIYQTSNFRVQPTESIVRFPQITNLCPFGEVFNATKFPSVYAWERKKISNCVADYSVLYNSTFFSTFKCYGVSATKLNDLCFSNVYADSFVVKGDDVRQIAPGQTGVIADYNYKLPDDFMGCVIAWNSNNLDSKVGGNYNYRYRLFRKDKLKPFERDISTEIYQAGSKPCNGVEGFNCYFPLQSYGFQPTYGVGYQPYRVVVLSFELLHAPATVCGPKKSTNLVKNKCVNFNFNGLTGTGVLTESNKKFLPFQQFGRDIADTTDAVRDPQTLEILDITPCSFGGVSVITPGTNTSNQVAVLYQGVNCTEVPVAIHADQLTPTWRVYSTGSNVFQTRAGCLIGAEHVNNSYECDIPIGAGICASYQTQTNSRGSASSVASQSIIAYTMSLGAENSVAYSNNSIAIPTNFTISVTTEILPVSMPKTSVDCTMYICGDSTECSNLLLQYGSFCTQLNRALTGIAVEQDKNTQEVFAQVKQIYKTPPIPDFGGFNFSQILPDPSKPSKRSPIEDLLFNKVTLADAGFIKQYGDCLGDIAARDLICAQKFNGLTVLPPLLTDEMIAQYTSALLAGTITSGWTFGAGPALQIPFPMQMAYRFNGIGVTQNVLYENQKLIANQFNSAIGKIQDSLSSTPSALGKLQNVVNQNAQALNTLVKCLSSNFGAISSVLNDILSRLDPPEAEVQIDRLITGRLQCLQTYVTQQLIRAAEIRASANLAATKMSECVLGQSKRVDFCGKGYHLMSFPQSAPHGVVFLHVTYVPAQEKNFTTAPAICHDGKAHFPREGVFVSNGTHWFVTQRNFYEPQIITTDNTFVSGNCDVVIGIVNNTVYDPLQPELDSFKEELDKYFKNHTSPDVDLGDISGILASVVNIQKEIDRLNEVAKNLNESLIDLQELGKYEQYIKWPGYIPEAPRDGQAYVRKDGEWVLLSTFLHHHHHH

SEQ ID NO: 111 - protein, 1242 aa, synthetic construct
MFVFLVLLPLVSSQCVNLITRTQSYTNSFTRGVYYPDKVFRSSVLHSTQDLFLPFFSNVTWFHAIHNSTTNGTKRFDNPALPFNDGVYFASTEKSNIIRGWIFGTTLDSKTQSLLIVNNATNVVIKVCEFQFCNDPFLDVYQKNNKSWMESEFRVYSSANNCTFEYVSQPFLMDLEGKEGNFKNLREFVFKNIDGYFKIYSKHTPINLNRTLPQGFSALEPLVDLPIGINITRFQTLLALHRSYLTPVDSSSGWTAGAAAYYVGYLQPRTFLLKYNENGTITDAVDCALDPLSETKCTLKSFTVEKGIYQTSNFRVQPTESIVRFPQITNLCPFGEVFNATKFPSVYAWERKKISNCVADYSVLYNSTFFSTFKCYGVSATKLNDLCFSNVYADSFVVKGDDVRQIAPGQTGVIADYNYKLPDDFMGCVIAWNSNNLDSKVGGNYNYRYRLFRKSKLKPFERDISTEIYQAGSKPCNGVEGFNCYFPLQSYGFQPTYGVGYQPYRVVVLSFELLHAPATVCGPKKSTNLVKNKCVNFNFNGLTGTGVLTESNKKFLPFQQFGRDIADTTDAVRDPQTLEILDITPCSFGGVSVITPGTNTSNQVAVLYQGVNCTEVPVAIHADQLTPTWRVYSTGSNVFQTRAGCLIGAEHVNNSYECDIPIGAGICASYQTQTNSRGSASSVASQSIIAYTMSLGAENSVAYSNNSIAIPTNFTISVTTEILPVSMPKTSVDCTMYICGDSTECSNLLLQYGSFCTQLNRALTGIAVEQDKNTQEVFAQVKQIYKTPPIPDFGGFNFSQILPDPSKPSKRSPIEDLLFNKVTLADAGFIKQYGDCLGDIAARDLICAQKFNGLTVLPPLLTDEMIAQYTSALLAGTITSGWTFGAGPALQIPFPMQMAYRFNGIGVTQNVLYENQKLIANQFNSAIGKIQDSLSSTPSALGKLQNVVNQNAQALNTLVKCLSSNFGAISSVLNDILSRLDPPEAEVQIDRLITGRLQCLQTYVTQQLIRAAEIRASANLAATKMSECVLGQSKRVDFCGKGYHLMSFPQSAPHGVVFLHVTYVPAQEKNFTTAPAICHDGKAHFPREGVFVSNGTHWFVTQRNFYEPQIITTDNTFVSGNCDVVIGIVNNTVYDPLQPELDSFKEELDKYFKNHTSPDVDLGDISGILASVVNIQKEIDRLNEVAKNLNESLIDLQELGKYEQYIKWPGYIPEAPRDGQAYVRKDGEWVLLSTFLHHHHHH

SEQ ID NO: 112 - protein, 1242 aa, synthetic construct
MFVFLVLLPLVSSQCVNLITRTQSYTNSFTRGVYYPDKVFRSSVLHSTQDLFLPFFSNVTWFHAIHVSGTNGTKRFDNPALPFNDGVYFASTEKSNIIRGWIFGTTLDSKTQSLLIVNNATNVVIKVCEFQFCNDPFLDVYQKNNKSWMESEFRVYSSANNCTFEYVSQPFLMDLEGKEGNFKNLREFVFKNIDGYFKIYSKHTPINLERDLPQGFSALEPLVDLPIGINITRFQTLLALHRSYLTPVDSSSGWTAGAAAYYVGYLQPRTFLLKYNENGTITDAVDCALDPLSETKCTLKSFTVEKGIYQTSNFRVQPTESIVRFPQITNLCPFGEVFNATKFPSVYAWERKKISNCVADYSVLYNSTFFSTFKCYGVSATKLNDLCFSNVYADSFVVKGDDVRQIAPGQTGVIADYNYKLPDDFMGCVIAWNSNNLDSKVGGNYNYRYRLFRKSKLKPFERDISTEIYQAGSKPCNGVEGFNCYFPLQSYGFQPTYGVGYQPYRVVVLSFELLHAPATVCGPKKSTNLVKNKCVNFNFNGLTGTGVLTESNKKFLPFQQFGRDIADTTDAVRDPQTLEILDITPCSFGGVSVITPGTNTSNQVAVLYQGVNCTEVPVAIHADQLTPNWTVYSTGSNVFQTRAGCLIGAEHVNNSYECDIPIGAGICASYQTQTNSRGSASSVASQSIIAYTMSLGAENSVAYSNNSIAIPTNFTISVTTEILPVSMPKTSVDCTMYICGDSTECSNLLLQYGSFCTQLNRALTGIAVEQDKNTQEVFAQVKQIYKTPPIPDFGGFNFSQILPDPSKPSKRSPIEDLLFNKVTLADAGFIKQYGDCLGDIAARDLICAQKFNGLTVLPPLLTDEMIAQYTSALLAGTITSGWTFGAGPALQIPFPMQMAYRFNGIGVTQNVLYENQKLIANQFNSAIGKIQDSLSSTPSALGKLQNVVNQNAQALNTLVKCLSSNFGAISSVLNDILSRLDPPEAEVQIDRLITGRLQCLQTYVTQQLIRAAEIRASANLAATKMSECVLGQSKRVDFCGKGYHLMSFPQSAPHGVVFLHVTYVPAQEKNFTTAPAICHDGKAHFPREGVFVSNGTHWFVTQRNFYEPQIITTDNTFVSGNCDVVIGIVNNTVYDPLQPELDSFKEELDKYFKNHTSPDVDLGDISGILASVVNIQKEIDRLNEVAKNLNESLIDLQELGKYEQYIKWPGYIPEAPRDGQAYVRKDGEWVLLSTFLHHHHHH

SEQ ID NO: 113 - protein, 1242 aa, synthetic construct
MFVFLVLLPLVSSQCVNLITRTQSYTNSFTRGVYYPDKVFRSSVLHSTQDLFLPFFSNVTWFHAIHVSGTNGTKRFDNPALPFNDGVYFASTEKSNIIRGWIFGTTLDSKTQSLLIVNNATNVVIKVCEFQFCNDPFLDVYQKNNKSWMESEFRVYSSANNCTFEYVSQPFLMDLEGKEGNFKNLREFVFKNIDGYFKIYSKHTPINLERDLPQGFSALEPLVDLPIGINITRFQTLLALHRSYLTPVDSSSGWTAGAAAYYVGYLQPRTFLLKYNENGTITDAVDCALDPLSETKCTLKSFTVEKGIYQTSNFRVQPTESIVRFPQITNLCPFGEVFNATKFPSVYAWERKKISNCVADYSVLYNSTFFSTFKCYGVSATKLNDLCFSNVYADSFVVKGDDVRQIAPGQTGVIADYNYKLPDDFMGCVIAWNSNNLDSKVGGNYNYRYRLFRKSKLKPFERDISTEIYQAGSKPCNGVEGFNCYFPLQSYGFQPTYGVGYQPYRVVVLSFELLHAPATVCGPKKSTNLVKNKCVNFNFNGLTGTGVLTESNKKFLPFQQFGRDIADTTDAVRDPQTLEILDITPCSFGGVSVITPGTNTSNQVAVLYQGVNCTEVPVAIHADQLTPTWRVYSTGSNVFQTRAGCLIGAEHVNNSYECDIPIGAGICASYQTQTNSRGSASSNATQSIIAYTMSLGAENSVAYSNNSIAIPTNFTISVTTEILPVSMPKTSVDCTMYICGDSTECSNLLLQYGSFCTQLNRALTGIAVEQDKNTQEVFAQVKQIYKTPPIPDFGGFNFSQILPDPSKPSKRSPIEDLLFNKVTLADAGFIKQYGDCLGDIAARDLICAQKFNGLTVLPPLLTDEMIAQYTSALLAGTITSGWTFGAGPALQIPFPMQMAYRFNGIGVTQNVLYENQKLIANQFNSAIGKIQDSLSSTPSALGKLQNVVNQNAQALNTLVKCLSSNFGAISSVLNDILSRLDPPEAEVQIDRLITGRLQCLQTYVTQQLIRAAEIRASANLAATKMSECVLGQSKRVDFCGKGYHLMSFPQSAPHGVVFLHVTYVPAQEKNFTTAPAICHDGKAHFPREGVFVSNGTHWFVTQRNFYEPQIITTDNTFVSGNCDVVIGIVNNTVYDPLQPELDSFKEELDKYFKNHTSPDVDLGDISGILASVVNIQKEIDRLNEVAKNLNESLIDLQELGKYEQYIKWPGYIPEAPRDGQAYVRKDGEWVLLSTFLHHHHHH

SEQ ID NO: 114 - protein, 1242 aa, synthetic construct
MFVFLVLLPLVSSQCVNLITRTQSYTNSFTRGVYYPDKVFRSSVLHSTQDLFLPFFSNVTWFHAIHVSGTNGTKRFDNPALPFNDGVYFASTEKSNIIRGWIFGTTLDSKTQSLLIVNNATNVVIKVCEFQFCNDPFLDVYQKNNKSWMESEFRVYSSANNCTFEYVSQPFLMDLEGKEGNFKNLREFVFKNIDGYFKIYSKHTPINLERDLPQGFSALEPLVDLPIGINITRFQTLLALHRSYLTPVDSSSGWTAGAAAYYVGYLQPRTFLLKYNENGTITDAVDCALDPLSETKCTLKSFTVEKGIYQTSNFRVQPTESIVRFPQITNLCPFGEVFNATKFPSVYAWERKKISNCVADYSVLYNSTFFSTFKCYGVSATKLNDLCFSNVYADSFVVKGDDVRQIAPGQTGVIADYNYKLPDDFMGCVIAWNSNNLDSKVGGNYNYRYRLFRKSKLKPFERDISTEIYQAGSKPCNGVEGFNCYFPLQSYGFQPTYGVGYQPYRVVVLSFELLHAPATVCGPKKSTNLVKNKCVNFNFNGLTGTGVLTESNKKFLPFQQFGRDIADTTDAVRDPQTLEILDITPCSFGGVSVITPGTNTSNQVAVLYQGVNCTEVPVAIHADQLTPTWRVYSTGSNVFQTRAGCLIGAEHVNNSYECDIPIGAGICASYQTQTNSRGSASSVASQSIIAYTMSLGAENSVAYSNNSIAIPTNFTISVTTEILPVSMPKTSVDCTMYICGDSTECSNLLLQYGSFCTQLNRALTGIAVEQDKNTQEVFAQVKQIYKTPPIPDFGGFNFSQILPDPSKPSKRSPIEDLLFNKVTLADAGFIKQYGDCNGTIAARDLICAQKFNGLTVLPPLLTDEMIAQYTSALLAGTITSGWTFGAGPALQIPFPMQMAYRFNGIGVTQNVLYENQKLIANQFNSAIGKIQDSLSSTPSALGKLQNVVNQNAQALNTLVKCLSSNFGAISSVLNDILSRLDPPEAEVQIDRLITGRLQCLQTYVTQQLIRAAEIRASANLAATKMSECVLGQSKRVDFCGKGYHLMSFPQSAPHGVVFLHVTYVPAQEKNFTTAPAICHDGKAHFPREGVFVSNGTHWFVTQRNFYEPQIITTDNTFVSGNCDVVIGIVNNTVYDPLQPELDSFKEELDKYFKNHTSPDVDLGDISGILASVVNIQKEIDRLNEVAKNLNESLIDLQELGKYEQYIKWPGYIPEAPRDGQAYVRKDGEWVLLSTFLHHHHHH

SEQ ID NO: 115 - protein, 1242 aa, synthetic construct
MFVFLVLLPLVSSQCVNLITRTQSYTNSFTRGVYYPDKVFRSSVLHSTQDLFLPFFSNVTWFHAIHVSGTNGTKRFDNPALPFNDGVYFASTEKSNIIRGWIFGTTLDSKTQSLLIVNNATNVVIKVCEFQFCNDPFLDVYQKNNKSWMESEFRVYSSANNCTFEYVSQPFLMDLEGKEGNFKNLREFVFKNIDGYFKIYSKHTPINLERDLPQGFSALEPLVDLPIGINITRFQTLLALHRSYLTPVDSSSGWTAGAAAYYVGYLQPRTFLLKYNENGTITDAVDCALDPLSETKCTLKSFTVEKGIYQTSNFRVQPTESIVRFPQITNLCPFGEVFNATKFPSVYAWERKKISNCVADYSVLYNSTFFSTFKCYGVSATKLNDLCFSNVYADSFVVKGDDVRQIAPGQTGVIADYNYKLPDDFMGCVIAWNSNNLDSKVGGNYNYRYRLFRKSKLKPFERDISTEIYQAGSKPCNGVEGFNCYFPLQSYGFQPTYGVGYQPYRVVVLSFELLHAPATVCGPKKSTNLVKNKCVNFNFNGLTGTGVLTESNKKFLPFQQFGRDIADTTDAVRDPQTLEILDITPCSFGGVSVITPGTNTSNQVAVLYQGVNCTEVPVAIHADQLTPTWRVYSTGSNVFQTRAGCLIGAEHVNNSYECDIPIGAGICASYQTQTNSRGSASSVASQSIIAYTMSLGAENSVAYSNNSIAIPTNFTISVTTEILPVSMPKTSVDCTMYICGDSTECSNLLLQYGSFCTQLNRALTGIAVEQDKNTQEVFAQVKQIYKTPPIPDFGGFNFSQILPDPSKPSKRSPIEDLLFNKVTLADAGFIKQYGDCLGDIAARDLICAQKFNGLTVLPPLLTDEMIAQYTSALLAGTITSGWTFGAGPALQIPFPMQMAYRFNGIGVTQNVLYENQKLIANQFNSAIGKIQDSLSSTPSALGKLQNVVNQNAQALNTLVKCLSSNFGAISSVLNDILSRLDPPEAEVQIDRLITGRLQCLQTYVTQQLIRAAEIRASANLAATKMSECVLGQSKRVDFCGKGYHLMSFPQSAPHGVVFLHVTYVPAQEKNFTTAPAICHDGKAHFPREGVFVSNGTHWFVTQRNFYEPQIITTDNTFVSGNCDVVIGIVNNTVYDPLQPELNSTKEELDKYFKNHTSPDVDLGDISGILASVVNIQKEIDRLNEVAKNLNESLIDLQELGKYEQYIKWPGYIPEAPRDGQAYVRKDGEWVLLSTFLHHHHHH

SEQ ID NO: 116 - protein, 1242 aa, synthetic construct
MFVFLVLLPLVSSQCVNLITRTQSYTNSFTRGVYYPDKVFRSSVLHSTQDLFLPFFSNVTWFHAIHVSGTNGTKRFDNPALPFNDGVYFASTEKSNIIRGWIFGTTLDSKTQSLLIVNNATNVVIKVCEFQFCNDPFLDVYQKNNKSWMESEFRVYSSANNCTFEYVSQPFLMDLEGKEGNFKNLREFVFKNIDGYFKIYSKHTPINLERDLPQGFSALEPLVDLPIGINITRFQTLLALHRSYLTPVDSSSGWTAGAAAYYVGYLQPRTFLLKYNENGTITDAVDCALDPLSETKCTLKSFTVEKGIYQTSNFRVQPTESIVRFPQITNLCPFGEVFNATKFPSVYAWERKKISNCVADYSVLYNSTFFSTFKCYGVSATKLNDLCFSNVYADSFVVKGDDVRQIAPGQTGVIADYNYKLPDDFMGCVIAWNSNNLDSKVGGNYNYRYRLFRKSKLKPFERDISTEIYQAGSKPCNGVEGFNCYFPLQSYGFQPTYGVGYQPYRVVVLSFELLHAPATVCGPKKSTNLVKNKCVNFNFNGLTGTGVLTESNKKFLPFQQFGRDIADTTDAVRDPQTLEILDITPCSFGGVSVITPGTNTSNQVAVLYQGVNCTEVPVAIHADQLTPNWTVYSTGSNVFQTRAGCLIGAEHVNNSYECDIPIGAGICASYQTQTNSRGSASSNATQSIIAYTMSLGAENSVAYSNNSIAIPTNFTISVTTEILPVSMPKTSVDCTMYICGDSTECSNLLLQYGSFCTQLNRALTGIAVEQDKNTQEVFAQVKQIYKTPPIPDFGGFNFSQILPDPSKPSKRSPIEDLLFNKVTLADAGFIKQYGDCLGDIAARDLICAQKFNGLTVLPPLLTDEMIAQYTSALLAGTITSGWTFGAGPALQIPFPMQMAYRFNGIGVTQNVLYENQKLIANQFNSAIGKIQDSLSSTPSALGKLQNVVNQNAQALNTLVKCLSSNFGAISSVLNDILSRLDPPEAEVQIDRLITGRLQCLQTYVTQQLIRAAEIRASANLAATKMSECVLGQSKRVDFCGKGYHLMSFPQSAPHGVVFLHVTYVPAQEKNFTTAPAICHDGKAHFPREGVFVSNGTHWFVTQRNFYEPQIITTDNTFVSGNCDVVIGIVNNTVYDPLQPELDSFKEELDKYFKNHTSPDVDLGDISGILASVVNIQKEIDRLNEVAKNLNESLIDLQELGKYEQYIKWPGYIPEAPRDGQAYVRKDGEWVLLSTFLHHHHHH

SEQ ID NO: 117 - protein, 1242 aa, synthetic construct
MFVFLVLLPLVSSQCVNLITRTQSYTNSFTRGVYYPDKVFRSSVLHSTQDLFLPFFSNVTWFHAIHVSGTNGTKRFDNPALPFNDGVYFASTEKSNIIRGWIFGTTLDSKTQSLLIVNNATNVVIKVCEFQFCNDPFLDVYQKNNKSWMESEFRVYSSANNCTFEYVSQPFLMDLEGKEGNFKNLREFVFKNIDGYFKIYSKHTPINLERDLPQGFSALEPLVDLPIGINITRFQTLLALHRSYLTPVDSSSGWTAGAAAYYVGYLQPRTFLLKYNENGTITDAVDCALDPLSETKCTLKSFTVEKGIYQTSNFRVQPTESIVRFPQITNLCPFGEVFNATKFPSVYAWERKKISNCVADYSVLYNSTFFSTFKCYGVSATKLNDLCFSNVYADSFVVKGDDVRQIAPGQTGVIADYNYKLPDDFMGCVIAWNSNNLDSKVGGNYNYRYRLFRKSKLKPFERDISTEIYQAGSKPCNGVEGFNCYFPLQSYGFQPTYGVGYQPYRVVVLSFELLHAPATVCGPKKSTNLVKNKCVNFNFNGLTGTGVLTESNKKFLPFQQFGRDIADTTDAVRDPQTLEILDITPCSFGGVSVITPGTNTSNQVAVLYQGVNCTEVPVAIHADQLTPTWRVYSTGSNVFQTRAGCLIGAEHVNNSYECDIPIGAGICASYQTQTNSRGSASSNATQSIIAYTMSLGAENSVAYSNNSIAIPTNFTISVTTEILPVSMPKTSVDCTMYICGDSTECSNLLLQYGSFCTQLNRALTGIAVEQDKNTQEVFAQVKQIYKTPPIPDFGGFNFSQILPDPSKPSKRSPIEDLLFNKVTLADAGFIKQYGDCNGTIAARDLICAQKFNGLTVLPPLLTDEMIAQYTSALLAGTITSGWTFGAGPALQIPFPMQMAYRFNGIGVTQNVLYENQKLIANQFNSAIGKIQDSLSSTPSALGKLQNVVNQNAQALNTLVKCLSSNFGAISSVLNDILSRLDPPEAEVQIDRLITGRLQCLQTYVTQQLIRAAEIRASANLAATKMSECVLGQSKRVDFCGKGYHLMSFPQSAPHGVVFLHVTYVPAQEKNFTTAPAICHDGKAHFPREGVFVSNGTHWFVTQRNFYEPQIITTDNTFVSGNCDVVIGIVNNTVYDPLQPELDSFKEELDKYFKNHTSPDVDLGDISGILASVVNIQKEIDRLNEVAKNLNESLIDLQELGKYEQYIKWPGYIPEAPRDGQAYVRKDGEWVLLSTFLHHHHHH

SEQ ID NO: 118 - protein, 1242 aa, synthetic construct
MFVFLVLLPLVSSQCVNLITRTQSYTNSFTRGVYYPDKVFRSSVLHSTQDLFLPFFSNVTWFHAIHVSGTNGTKRFDNPALPFNDGVYFASTEKSNIIRGWIFGTTLDSKTQSLLIVNNATNVVIKVCEFQFCNDPFLDVYQKNNKSWMESEFRVYSSANNCTFEYVSQPFLMDLEGKEGNFKNLREFVFKNIDGYFKIYSKHTPINLERDLPQGFSALEPLVDLPIGINITRFQTLLALHRSYLTPVDSSSGWTAGAAAYYVGYLQPRTFLLKYNENGTITDAVDCALDPLSETKCTLKSFTVEKGIYQTSNFRVQPTESIVRFPQITNLCPFGEVFNATKFPSVYAWERKKISNCVADYSVLYNSTFFSTFKCYGVSATKLNDLCFSNVYADSFVVKGDDVRQIAPGQTGVIADYNYKLPDDFMGCVIAWNSNNLDSKVGGNYNYRYRLFRKSKLKPFERDISTEIYQAGSKPCNGVEGFNCYFPLQSYGFQPTYGVGYQPYRVVVLSFELLHAPATVCGPKKSTNLVKNKCVNFNFNGLTGTGVLTESNKKFLPFQQFGRDIADTTDAVRDPQTLEILDITPCSFGGVSVITPGTNTSNQVAVLYQGVNCTEVPVAIHADQLTPTWRVYSTGSNVFQTRAGCLIGAEHVNNSYECDIPIGAGICASYQTQTNSRGSASSVASQSIIAYTMSLGAENSVAYSNNSIAIPTNFTISVTTEILPVSMPKTSVDCTMYICGDSTECSNLLLQYGSFCTQLNRALTGIAVEQDKNTQEVFAQVKQIYKTPPIPDFGGFNFSQILPDPSKPSNRTPIEDLLFNKVTLADAGFIKQYGDCNGTIAARDLICAQKFNGLTVLPPLLTDEMIAQYTSALLAGTITSGWTFGAGPALQIPFPMQMAYRFNGIGVTQNVLYENQKLIANQFNSAIGKIQDSLSSTPSALGKLQNVVNQNAQALNTLVKCLSSNFGAISSVLNDILSRLDPPEAEVQIDRLITGRLQCLQTYVTQQLIRAAEIRASANLAATKMSECVLGQSKRVDFCGKGYHLMSFPQSAPHGVVFLHVTYVPAQEKNFTTAPAICHDGKAHFPREGVFVSNGTHWFVTQRNFYEPQIITTDNTFVSGNCDVVIGIVNNTVYDPLQPELDSFKEELDKYFKNHTSPDVDLGDISGILASVVNIQKEIDRLNEVAKNLNESLIDLQELGKYEQYIKWPGYIPEAPRDGQAYVRKDGEWVLLSTFLHHHHHH

SEQ ID NO: 119 - protein, 1242 aa, synthetic construct
MFVFLVLLPLVSSQCVNLITRTQSYTNSFTRGVYYPDKVFRSSVLHSTQDLFLPFFSNVTWFHAIHVSGTNGTKRFDNPALPFNDGVYFASTEKSNIIRGWIFGTTLDSKTQSLLIVNNATNVVIKVCEFQFCNDPFLDVYQKNNKSWMESEFRVYSSANNCTFEYVSQPFLMDLEGKEGNFKNLREFVFKNIDGYFKIYSKHTPINLERDLPQGFSALEPLVDLPIGINITRFQTLLALHRSYLTPVDSSSGWTAGAAAYYVGYLQPRTFLLKYNENGTITDAVDCALDPLSETKCTLKSFTVEKGIYQTSNFRVQPTESIVRFPQITNLCPFGEVFNATKFPSVYAWERKKISNCVADYSVLYNSTFFSTFKCYGVSATKLNDLCFSNVYADSFVVKGDDVRQIAPGQTGVIADYNYKLPDDFMGCVIAWNSNNLDSKVGGNYNYRYRLFRKSKLKPFERDISTEIYQAGSKPCNGVEGFNCYFPLQSYGFQPTYGVGYQPYRVVVLSFELLHAPATVCGPKKSTNLVKNKCVNFNFNGLTGTGVLTESNKKFLPFQQFGRDIADTTDAVRDPQTLEILDITPCSFGGVSVITPGTNTSNQVAVLYQGVNCTEVPVAIHADQLTPTWRVYSTGSNVFQTRAGCLIGAEHVNNSYECDIPIGAGICASYQTQTNSRGSASSVASQSIIAYTMSLGAENSVAYSNNSIAIPTNFTISVTTEILPVSMPKTSVDCTMYICGDSTECSNLLLQYGSFCTQLNRALTGIAVEQDKNTQEVFAQVKQIYKTPPIPDFGGFNFSQILPDPSKPSNRTPIEDLLFNKVTLADAGFIKQYGDCLGDIAARDLICAQKFNGLTVLPPLLTDEMIAQYTSALLAGTITSGWTFGAGPALQIPFPMQMAYRFNGIGVTQNVLYENQKLIANQFNSAIGKIQDSLSSTPSALGKLQNVVNQNAQALNTLVKCLSSNFGAISSVLNDILSRLDPPEAEVQIDRLITGRLQCLQTYVTQQLIRAAEIRASANLAATKMSECVLGQSKRVDFCGKGYHLMSFPQSAPHGVVFLHVTYVPAQEKNFTTAPAICHDGKAHFPREGVFVSNGTHWFVTQRNFYEPQIITTDNTFVSGNCDVVIGIVNNTVYDPLQPELNSTKEELDKYFKNHTSPDVDLGDISGILASVVNIQKEIDRLNEVAKNLNESLIDLQELGKYEQYIKWPGYIPEAPRDGQAYVRKDGEWVLLSTFLHHHHHH

SEQ ID NO: 120 - protein, 1242 aa, synthetic construct
MFVFLVLLPLVSSQCVNLITRTQSYTNSFTRGVYYPDKVFRSSVLHSTQDLFLPFFSNVTWFHAIHVSGTNGTKRFDNPALPFNDGVYFASTEKSNIIRGWIFGTTLDSKTQSLLIVNNATNVVIKVCEFQFCNDPFLDVYQKNNKSWMESEFRVYSSANNCTFEYVSQPFLMDLEGKEGNFKNLREFVFKNIDGYFKIYSKHTPINLERDLPQGFSALEPLVDLPIGINITRFQTLLALHRSYLTPVDSSSGWTAGAAAYYVGYLQPRTFLLKYNENGTITDAVDCALDPLSETKCTLKSFTVEKGIYQTSNFRVQPTESIVRFPQITNLCPFGEVFNATKFPSVYAWERKKISNCVADYSVLYNSTFFSTFKCYGVSATKLNDLCFSNVYADSFVVKGDDVRQIAPGQTGVIADYNYKLPDDFMGCVIAWNSNNLDSKVGGNYNYRYRLFRKSKLKPFERDISTEIYQAGSKPCNGVEGFNCYFPLQSYGFQPTYGVGYQPYRVVVLSFELLHAPATVCGPKKSTNLVKNKCVNFNFNGLTGTGVLTESNKKFLPFQQFGRDIADTTDAVRDPQTLEILDITPCSFGGVSVITPGTNTSNQVAVLYQGVNCTEVPVAIHADQLTPTWRVYSTGSNVFQTRAGCLIGAEHVNNSYECDIPIGAGICASYQTQTNSRGSASSVASQSIIAYTMSLGAENSVAYSNNSIAIPTNFTISVTTEILPVSMPKTSVDCTMYICGDSTECSNLLLQYGSFCTQLNRALTGIAVEQDKNTQEVFAQVKQIYKTPPIPDFGGFNFSQILPDPSKPSKRSPIEDLLFNKVTLADAGFIKQYGDCNGTIAARDLICAQKFNGLTVLPPLLTDEMIAQYTSALLAGTITSGWTFGAGPALQIPFPMQMAYRFNGIGVTQNVLYENQKLIANQFNSAIGKIQDSLSSTPSALGKLQNVVNQNAQALNTLVKCLSSNFGAISSVLNDILSRLDPPEAEVQIDRLITGRLQCLQTYVTQQLIRAAEIRASANLAATKMSECVLGQSKRVDFCGKGYHLMSFPQSAPHGVVFLHVTYVPAQEKNFTTAPAICHDGKAHFPREGVFVSNGTHWFVTQRNFYEPQIITTDNTFVSGNCDVVIGIVNNTVYDPLQPELNSTKEELDKYFKNHTSPDVDLGDISGILASVVNIQKEIDRLNEVAKNLNESLIDLQELGKYEQYIKWPGYIPEAPRDGQAYVRKDGEWVLLSTFLHHHHHH

SEQ ID NO: 121 - protein, 1242 aa, synthetic construct
MFVFLVLLPLVSSQCVNLITRTQSYTNSFTRGVYYPDKVFRSSVLHSTQDLFLPFFSNVTWFHAIHVSGTNGTKRFDNPALPFNDGVYFASTEKSNIIRGWIFGTTLDSKTQSLLIVNNATNVVIKVCEFQFCNDPFLDVYQKNNKSWMESEFRVYSSANNCTFEYVSQPFLMDLEGKEGNFKNLREFVFKNIDGYFKIYSKHTPINLERDLPQGFSALEPLVDLPIGINITRFQTLLALHRSYLTPVDSSSGWTAGAAAYYVGYLQPRTFLLKYNENGTITDAVDCALDPLSETKCTLKSFTVEKGIYQTSNFRVQPTESIVRFPQITNLCPFGEVFNATKFPSVYAWERKKISNCVADYSVLYNSTFFSTFKCYGVSATKLNDLCFSNVYADSFVVKGDDVRQIAPGQTGVIADYNYKLPDDFMGCVIAWNSNNLDSKVGGNYNYRYRLFRKSKLKPFERDISTEIYQAGSKPCNGVEGFNCYFPLQSYGFQPTYGVGYQPYRVVVLSFELLHAPATVCGPKKSTNLVKNKCVNFNFNGLTGTGVLTESNKKFLPFQQFGRDIADTTDAVRDPQTLEILDITPCSFGGVSVITPGTNTSNQVAVLYQGVNCTEVPVAIHADQLTPNWTVYSTGSNVFQTRAGCLIGAEHVNNSYECDIPIGAGICASYQTQTNSRGSASSNATQSIIAYTMSLGAENSVAYSNNSIAIPTNFTISVTTEILPVSMPKTSVDCTMYICGDSTECSNLLLQYGSFCTQLNRALTGIAVEQDKNTQEVFAQVKQIYKTPPIPDFGGFNFSQILPDPSKPSKRSPIEDLLFNKVTLADAGFIKQYGDCNGTIAARDLICAQKFNGLTVLPPLLTDEMIAQYTSALLAGTITSGWTFGAGPALQIPFPMQMAYRFNGIGVTQNVLYENQKLIANQFNSAIGKIQDSLSSTPSALGKLQNVVNQNAQALNTLVKCLSSNFGAISSVLNDILSRLDPPEAEVQIDRLITGRLQCLQTYVTQQLIRAAEIRASANLAATKMSECVLGQSKRVDFCGKGYHLMSFPQSAPHGVVFLHVTYVPAQEKNFTTAPAICHDGKAHFPREGVFVSNGTHWFVTQRNFYEPQIITTDNTFVSGNCDVVIGIVNNTVYDPLQPELDSFKEELDKYFKNHTSPDVDLGDISGILASVVNIQKEIDRLNEVAKNLNESLIDLQELGKYEQYIKWPGYIPEAPRDGQAYVRKDGEWVLLSTFLHHHHHH

SEQ ID NO: 122 - protein, 1242 aa, synthetic construct
MFVFLVLLPLVSSQCVNLITRTQSYTNSFTRGVYYPDKVFRSSVLHSTQDLFLPFFSNVTWFHAIHVSGTNGTKRFDNPLLPFNDGVYFASTEKSNIIRGWIFGTTLDSKTQSLLIVNNATNVVIKVCEFQFCNDPFLDVYDKNNKSWMESEYRVYSSANNCTFEYVSQPFLMDLEGKNGNFKNLREFVFKNIDGYFKIYSKHTPINLDRDLPQGFSALEPLVDLPIGINITRFQTLLALHRSYLTPADSSSGWTAGAAAYYVGYLQPRTFLLKYNENGTITDAVDCALDPLSETKCTLKSFTVEKGIYQTSNFRVQPTESIVRFPQITNLCPFGEVFNATKFPSVYAWERKKISNCVADYSVLYNSTFFSTFKCYGVSATKLNDLCFSNVYADSFVVKGDDVRQIAPGQTGVIADYNYKLPDDFMGCVIAWNSNNLDSKVGGNYNYRYRLFRKSKLKPFERDISTEIYQAGSKPCNGVEGFNCYFPLQSYGFQPTYGVGYQPYRVVVLSFELLHAPATVCGPKKSTNLVKNKCVNFNFNGLTGTGVLTESNKKFLPFQQFGRDIADTTDAVRDPQTLEILDITPCSFGGVSVITPGTNTSNQVAVLYQGVNCTEVPVAIHADQLTPTWRVYSTGSNVFQTRAGCLIGAEHVNNSYECDIPIGAGICASYQTQTNSRGSASSVASQSIIAYTMSLGAENSVAYSNNSIAIPTNFTISVTTEILPVSMPKTSVDCTMYICGDSTECSNLLLQYGSFCTQLNRALTGIAVEQDKNTQEVFAQVKQIYKTPPIPDFGGFNFSQILPDPSKPSKRSPIEDLLFNKVTLADAGFIKQYGDCLGDIAARDLICAQKFNGLTVLPPLLTDEMIAQYTSALLAGTITSGWTFGAGPALQIPFPMQMAYRFNGIGVTQNVLYENQKLIANQFNSAIGKIQDSLSSTPSALGKLQNVVNQNAQALNTLVKCLSSNFGAISSVLNDILSRLDPPEAEVQIDRLITGRLQCLQTYVTQQLIRAAEIRASANLAATKMSECVLGQSKRVDFCGKGYHLMSFPQSAPHGVVFLHVTYVPAQEKNFTTAPAICHDGKAHFPREGVFVSNGTHWFVTQRNFYEPQIITTDNTFVSGNCDVVIGIVNNTVYDPLQPELDSFKEELDKYFKNHTSPDVDLGDISGILASVVNIQKEIDRLNEVAKNLNESLIDLQELGKYEQYIKWPGYIPEAPRDGQAYVRKDGEWVLLSTFLHHHHHH